European Patent Specification EP 3 942 028 B9, published August 23, 2023. Title: Methods of Producing Bioconjugates of E. coli O-Antigen Polysaccharides, Compositions Thereof, and Methods of Use Thereof. Applicant: Janssen Pharmaceuticals, Inc. GlaxoSmithKline Biologicals S.A. The sequence listing filed with the application follows.

SEQUENCE LISTING (19 sequences)

SEQ ID NO: 1 - protein, 3 aa, Artificial Sequence
  glycosylation consensus sequence
  VARIANT (2)..(2): any amino acid residue except Pro
  VARIANT (3)..(3): Ser orThr
NXX

SEQ ID NO: 2 - protein, 5 aa, Artificial Sequence
  optimized glycosylation consensus sequence
  VARIANT (1)..(1): Asp or Glu
  VARIANT (2)..(2): any amino acid residue except Pro
  VARIANT (4)..(4): any amino acid residue except Pro
  VARIANT (5)..(5): Ser or Thr
XXNXX

SEQ ID NO: 3 - protein, 652 aa, Artificial Sequence
  EPA carrier protein comprising 4 glycosylation consensus sequences (EPA-4)
GSGGGDQNATGSGGGKLAEEAFDLWNECAKACVLDLKDGVRSSRMSVDPAIADTNGQGVLHYSMVLEGGNDALKLAIDNALSITSDGLTIRLEGGVEPNKPVRYSYTRQARGSWSLNWLVPIGHEKPSNIKVFIHELNAGNQLSHMSPIYTIEMGDELLAKLARDATFFVRAHESNEMQPTLAISHAGVSVVMAQAQPRREKRWSEWASGKVLCLLDPLDGVYNYLAQQRCNLDDTWEGKIYRVLAGNPAKHDLDIKDNNNSTPTVISHRLHFPEGGSLAALTAHQACHLPLEAFTRHRQPRGWEQLEQCGYPVQRLVALYLAARLSWNQVDQVIRNALASPGSGGDLGEAIREQPEQARLALTLAAAESERFVRQGTGNDEAGAASADVVSLTCPVAKDQNRTKGECAGPADSGDALLERNYPTGAEFLGDGGDVSFSTRGTQNWTVERLLQAHRQLEERGYVFVGYHGTFLEAAQSIVFGGVRARSQDLDAIWRGFYIAGDPALAYGYAQDQEPDARGRIRNGALLRVYVPRWSLPGFYRTGLTLAAPEAAGEVERLIGHPLPLRLDAITGPEEEGGRVTILGWPLAERTVVIPSAIPTDPRNVGGDLDPSSIPDKEQAISALPDYASQPGKPPREDLKLGSGGGDQNAT

SEQ ID NO: 4 - protein, 421 aa, Artificial Sequence
  O4 GtrS amino acid sequence
MNNLIMNNWCKLSIFIIAFILLWLRRPDILTNAQFWAEDSVFWYKDAYENGFLSSLTTPRNGYFQTVSTFIVGLTALLNPDYAPFVSNFFGIMIRSVIIWFLFTERFNFLTLTTRIFLSIYFLCMPGLDEVHANITNAHWYLSLYVSMILIARNPSSKSWRFHDIFFILLSGLSGPFIIFILAASCFKFINNCKDHISVRSFINFYLRQPYALMIVCALIQGTSIILTFNGTRSSAPLGFSFDVISSIISSNIFLFTFVPWDIAKAGWDNLLLSYFLSVSILSCAAFVFVKGTWRMKVFATLPLLIIIFSMAKPQLTDSAPQLPTLINGQGSRYFVNIHIAIFSLLCVYLLECVRGKVATLFSKIYLTILLFVMGCLNFVITPLPNMNWREGATLINNAKTGDVISIQVLPPGLTLELRKK

SEQ ID NO: 5 - DNA, 1266 bp, Artificial Sequence
  Example O4 gtrS nucleic acid sequence
atgaataatttaattatgaataactggtgtaaattatctatatttattattgcatttattttgctatggcttagaaggccggatatactcacaaacgcacaattttgggcagaagattccgttttctggtataaggacgcctatgagaacggattcttaagttcactaacaacgcctaggaatgggtatttccagactgtttctacatttatagttggtctgactgctttattaaatccagattatgcaccttttgtttctaatttttttggcataatgattcgctcagtaattatatggtttttatttacagaaagattcaacttcctcacattgactactaggattttcttatctatttattttctatgcatgcctggattggatgaagttcatgcaaatataacaaatgcacattggtatttgtcattatatgtatcaatgatcctgatagctcgcaatccaagttcaaaatcatggaggtttcatgatatattctttatcttgctatccgggctcagtggcccatttataattttcattttagcagcttcatgctttaaatttataaataattgtaaagatcatattagtgtaagatctttcataaatttctacttgcgtcagccatacgcattaatgattgtttgcgctttaattcaaggaacttctataattctaactttcaatggcacacgttcctcagcaccgctaggattcagttttgatgtgatttcgtctattatatcatcgaatatttttttatttacatttgtcccatgggatattgcaaaggctgggtgggataatttactgttatcttattttttgtctgtttcgattttgtcgtgtgcggcctttgtttttgttaaaggtacgtggcgaatgaaagtatttgcaactttaccattgctaattataatattttcaatggcaaaaccacaattgacagactcggcacctcaattgccaacacttattaatgggcaaggttcaagatacttcgtaaatatacatattgcgatattctctttgctatgtgtttacttacttgagtgcgtcagggggaaagtggcaactttattttccaaaatatacttaacaattttgctattcgtgatgggatgtttgaattttgttatcaccccactcccaaacatgaactggagggaaggtgctactttgattaataatgcaaaaactggtgatgtcatttcgattcaagtgctaccacctggcctaacacttgaactaaggaaaaaataa

SEQ ID NO: 6 - protein, 713 aa, Artificial Sequence
  Example PglB sequence ('wild-type')
MLKKEYLKNPYLVLFAMIILAYVFSVFCRFYWVWWASEFNEYFFNNQLMIISNDGYAFAEGARDMIAGFHQPNDLSYYGSSLSALTYWLYKITPFSFESIILYMSTFLSSLVVIPTILLANEYKRPLMGFVAALLASIANSYYNRTMSGYYDTDMLVIVLPMFILFFMVRMILKKDFFSLIALPLFIGIYLWWYPSSYTLNVALIGLFLIYTLIFHRKEKIFYIAVILSSLTLSNIAWFYQSAIIVILFALFALEQKRLNFMIIGILGSATLIFLILSGGVDPILYQLKFYIFRSDESANLTQGFMYFNVNQTIQEVENVDLSEFMRRISGSEIVFLFSLFGFVWLLRKHKSMIMALPILVLGFLALKGGLRFTIYSVPVMALGFGFLLSEFKAIMVKKYSQLTSNVCIVFATILTLAPVFIHIYNYKAPTVFSQNEASLLNQLKNIANREDYVVTWWDYGYPVRYYSDVKTLVDGGKHLGKDNFFPSFALSKDEQAAANMARLSVEYTEKSFYAPQNDILKTDILQAMMKDYNQSNVDLFLASLSKPDFKIDTPKTRDIYLYMPARMSLIFSTVASFSFINLDTGVLDKPFTFSTAYPLDVKNGEIYLSNGVVLSDDFRSFKIGDNVVSVNSIVEINSIKQGEYKITPIDDKAQFYIFYLKDSAIPYAQFILMDKTMFNSAYVQMFFLGNYDKNLFDLVINSRDAKVFKLKI

SEQ ID NO: 7 - protein, 120 aa, Escherichia coli
MLKLFAKYTSIGVLNTLIHWVVFGVCIYVAHTNQALANFAGFVVAVSFSFFANAKFTFKASTTTMRYMLYVGFMGTLSATVGWAADRCALPPMITLVTFSAISLVCGFVYSKFIVFRDAK

SEQ ID NO: 8 - protein, 306 aa, Escherichia coli
MKISLVVPVFNEEEAIPIFYKTVREFEELKSYEVEIVFINDGSKDATESIINALAVSDPLVVPLSFTRNFGKEPALFAGLDHATGDAIIPIDVDLQDPIEVIPHLIEKWQAGADMVLAKRSDRSTDGRLKRKTAEWFYKLHNKISNPKIEENVGDFRLMSRDVVENIKLMPERNLFMKGILSWVGGKTDIVEYVRAERIAGDTKFNGWKLWNLALEGITSFSTFPLRIWTYIGLVVASVAFIYGAWMILDTIIFGNAVRGYPSLLVSILFLGGIQMIGIGVLGEYIGRTYIETKKRPKYIIKRVKK

SEQ ID NO: 9 - DNA, 14440 bp, Artificial Sequence
  example O4 rfb locus nucleotide sequence - O4-EPA production strain BVEC-L-00684f
atgacgaatttaaaagcagttattcctgtagcgggtctcgggatgcatatgttgcctgccactaaggcgatacccaaagagatgctaccaatcgtcgacaagccaatgattcagtacattgttgacgagattgtggctgcagggatcaaagaaatcctcctggtaactcacgcgtccaagaacgcggtcgaaaaccacttcgacacctcttatgagttagaatcactccttgagcagcgcgtgaagcgtcaactgctggcggaagtacagtccatctgtccgccgggcgtgaccattatgaacgtgcgtcagggcgaacctttaggtttaggccactccattttgtgtgcgcgacctgccattggtgacaacccatttgtcgtggtactgccagacgttgtgatcgacgatgccagcgccgacccgctacgttacaaccttgctgccatgattgcacgtttcaacgaaacgggccgcagccaggtgctggcaaaacgtatgccgggtgacctctctgaatactccgtcatccagactaaagagccgctggaccgtgagggtaaagtcagccgcattgttgaatttatcgaaaaaccggatcagccgcagacgctggactcagacatcatggccgtaggtcgctatgtgctttctgccgatatttggccggaactggaacgtactcagcctggtgcatggggacgtattcagctgactgatgctattgccgagctggcgaaaaaacaatccgttgatgcaatgctgatgaccggcgacagttacgactgcggcaaaaaaatgggctatatgcaggcgtttgtgaagtatggcctacgcaacctgaaagaaggggcgaagttccgtaaaggtattgagaagctgttaagcgaataatgaaaatctgaccggatgtaacggttgataagaaaattataacggcagtgaaaattcgcagcaaaagtaatttgttgcgaatcttcctgccgttgttttatataaaccatcagaataacaacgagttagcagtagggttttattcaaagttttccaggattttccttgtttccagagcggattggtaagacaattagcgtttgaatttttcgggtttagcgcgagtgggtaacgctcgtcacatcataggcatgcatgcagtgctctggtagctgtaaagccaggggcggtagcgtgcattaatacctctattaatcaaactgagagccgcttatttcacagcatgctctgaagtaatatggaataaattaagtgaaaatacttgttactggtggcgcaggatttattggttcagctgtagttcgtcacattataaataatacgcaggatagtgttgttaatgtcgataaattaacgtacgccggaaaccgggaatcacttgctgatgtttctgattctgaacgctatgtttttgaacatgcggatatttgcgatgcacctgcaatggcacggatttttgctcagcatcagccggatgcagtgatgcacctggctgctgaaagccatgttgaccgttcaattacaggccctgcggcatttattgaaaccaatattgttggtacttatgtccttttggaagccgctcgcaattactggtctgctcttgatagcgacaagaaaaatagcttccgttttcatcatatttctactgacgaagtatatggtgatttgcctcatcctgacgaggtaaataatacagaagaattacccttatttactgagacaacagcttacgcgccaagcagcccttattccgcatccaaagcatccagcgatcatttagtccgcgcgtggaaacgtacctatggtttaccgaccattgtgactaattgctctaacaattatggtccttatcatttcccggaaaaattgattccattggttattctcaatgctctggaaggtaaagcattacctatttatggtaaaggggatcaaattcgcgactggctgtatgttgaagatcatgcgcgtgcgttatataccgtcgtaaccgaaggtaaagcgggtgaaacttataacattggtgggcacaacgaaaagaaaaacatagatgtagtgctcactatttgtgatttgctggatgagattgtaccgaaagagaaatcttatcgtgagcaaatcacttatgttgccgatcgtccgggacacgatcgccgttatgcgattgatgctgagaatattggtcgcgaattgggatggaaaccacaggaaacgtttgagagcgggattcggaagacagtggaatggtatctgtccaatacaaaatgggttgataatgtgaaaagtggtgcctatcaatcgtggattgaagagaactatgagggccgccagtaatgaatatcctcctttttggcaaaacagggcaggtaggttgggaactacagcgtgctctggcacctctgggtaacttgattgctcttgatgttcattccactgattattgtggcgatttcagtaaccccgaaggtgtggctgaaaccgtcaaaaaaattcgcccagatgttattgttaatgctgctgctcataccgcggtagataaggctgagtcagaaccagaatttgcacaattactcaatgcgaccagcgttgaagcaattgcaaaagcggctaatgaagttggggcttgggtaattcattactcaactgactacgtcttccctggaaatggcgacatgccatggctcgagactgatgtaaccgctccgctcaatgtttatggcaaaaccaaattggctggagaaagagcattacaagaacattgcgcaaagcatcttattttccgtaccagctgggtatatgcaggtaaaggaaataactttgccaaaacaatgttacgtctggcaaaagagcgcgaagaactggctgtgataaacgatcagtttggcgcaccaacaggtgctgaattgctggctgattgcaccgctcatgccattcgcgtggcattaaaaaaaccagaagttgctggcttgtaccatctggtagcaaatggcacaacaacctggcacgattacgccgcgctagtattcgaagaagcccgtaaagcagggattgaccttgcacttaacaaactcaacgccgtaccaacaacggcttatcctactccagcccgccgtcctcataattctcgcctcaataccgaaaagtttcagcagaactttgcgcttgtcttgcctgactggcaggtgggcgtgaaacgtatgctcaacgaattatttacgactacggcaatttaacaaatttttgcatctcgctcatgatgccagagcgggatgaattaaaaggaatggtgaaatgaaaacgcgtaaaggtattattctggctggtggttccggcactcgtctttatcctgtgacgatggcagtgagtaaacaactgctgccgatttatgataagccgatgatttattatccgctttcaacgcttatgttagcgggtattcgcgatattcttattatcagtacgccacaggatacaccgcgtttccaacaattgttgggggacgggagtcagtgggggcttaatctacagtataaagtacaaccgagtccggatggcctggcgcaagcgtttattattggtgaagactttattggtggtgatgattgtgcactcgtacttggcgataatatcttctatggacacgacttgccgaaattaatggaagctgctgttaacaaagaaatcggtgcaacggtatttgcttatcacgtcaatgatcctgaacgttatggtgtcgtggagtttgataataacggtactgcaattagcctggaagaaaaaccgctggaaccaaaaagtaactatgcggttactgggctttatttctatgacaatgatgttgtagaaatggcgaaaaaccttaagccttctgcccgtggcgaactggaaattaccgatattaaccgtatttatatggagcagggacgtttgtctgtcgctatgatggggcgtggttatgcctggttggatactggtacacatcaaagtcttattgaagcaagtaacttcattgccaccattgaagagcgtcagggattaaaggtatcttgcccggaagagattgcttaccgtaaagggtttattgatgctgagcaggtgaaagtattagccgaaccgctgaagaaaaatgattatggtcagtatctgctaaaaatgattaaaggttattaataaaatgaacgtaattaaaactgaaattcctgatgtgctgatttttgaaccaaaagtttttggtgatgaacgtggcttcttttttgagagttttaaccagaaagtatttgaagaagctgtaggacggaaggttgaatttgttcaggataaccattctaagtctaaaataaatgtattgcgtgggatgcattatcaaacacaaaatactcaaggaaaactggttcgggtaatttctggttcagtatatgatgttgccgtagatttaagagaaaaatcaaagacatttggcaaatgggtgggtgtagaattatctgggaataataaaagacaattgtggatccccgaaggttttgcccatggtttttatgtgttggaggagaataccgaatttgtttataaatgtaccgatacttataaccctgctcatgaacacacattgctatggaatgatccaactatcaatataagttggccaatcatacaaaactgcaagccaattatttctgaaaaagatgctaatggacatcttttttcacataaaacctatttctgaaatgcaatattatgagtttaattagaaacagtttctataatattgctggttttgctgtgccgacattagttgcagtccctgctttggggattcttgccaggctgcttggaccggagaattttggacttttcacactagcattcgctttgataggatatgcaagtattttcgacgccgggattagtcgagctgtaatcagagaaatcgctctttatcgagaaagtgaaaaagagcaaatacaaattatttcgacagcaagtgtaatcgtactattcttaggggtggttgcagctttgttactttattttagtagtaataaagttgttgagttattgaatgttagttccgtttatattgaaacagcagtgcgtgcattctctgttatttcatttataatacctgtgtatctgattaaccagatttggcttggttatctggaagggctagaaaaatttgcaaatataaatgttcagagaatgatttctagcacaagcttggctatattaccagtgatattttgttattacaatccctcgttgctttatgctatgtatgggttggtggttgggcgtgtgatttcatttttgattagcgcaataatttgtcgagatattattcttaaaagtaaactttactttaatgtggcaacttgcaatcgtcttatctcttttggtggatggataacagttagtaatatcataagcccaatcatggcatatttcgaccgctttatcatctctcatattatgggggcttcgagaattgcattttatacagcgccctcagagggtgtatcaaggttaattaatatcccatatgctttggcaagagctctatttcctaaattggcatatagcaataatgatgatgaacgaaaaaaattacaactacagagctacgcaattataagcattgtatgtctacccatagttgttattggtgtcatttttgcctcattcataatgacaacatggatgggacctgattatgccttagaagcagcaactatcatgaaaatacttcttgctggttttttctttaactctttagcgcaaataccttatgcatacttgcaatctatcggaaagtcaaaaattaccgcatttgtgcatctcatagaacttgcgccatacttattattattgtattacttcacaatgcatttcggcataattggcacggcaatcgcttggtcacttagaacattttgtgattttgttatactactttcgatatcgagaagaaaatgattgcggttgatattgcgcttgcaacctacaatggtgctaattttattcggcaacagattgaatctatccagaaacaaacttatagaaattggcgtcttataataagtgatgataactcgagtgatgatactgttgatattattaaggatatgatgtctaacgacagtcgtatctatttggtaggaaataaaagacaaggaggggttattcagaactttaattatgctctttcacaaactacatctgaaattgtgttactatgtgaccaggatgacatttggccggaggagcgtctggaaattcttatagataaatttaaggccttgcagcgtaatgattttgttccggcaatgatgtttactgatttgaaattagtagacgaaaataattgtttgattgcagaaagtttttatcgaacgaataatattaatccacaagataatctgaaaaataataatcttctctggcgttcaacggtatatggctgtacttgcatcatgaataagaaacttgttgatattgcattgcctatacctacatatgcacatatgcatgatcaatggttggcattattagcgaagcaatatggtaacattttttatttcgactatgcgtctgttcgttataggcaacattctacaaatgttgttggtggtagaaataaaacgccatttcaaaaatttaattccatacaaaaaaacctaaaaaggattaatttgctagtggatagaactgttgctttaattaaatcaaataacgatttctatccagggaataaaatggaaaataaaattgattacttaaaatttggagtgaatgaagtattaccttatctttttaaaggaaacaagaaagttttttcactttgtgtattaattagtttggcattacaaaaatgatatatttattatttttttttgcactgtttatgatctgtacgtttttaacacacaggcgacaggcattatatgttgtatctgcgttagtatttctttttttggctttaacctatccatcaggaggggactggataggttattttctccattatgactgcatggttaatgagcagtgtaataatggttttataatgtttgaacctggatatgaattaattgtttccttatttggatatttgggatttcagacaattattatttttatagccgctgtaaatgtaattctaatattaaattttgcaaagcattttgaaaacggaagttttgttattgttgcgataatgtgcatgttcctttggagtgtttatgttgaggcgattagacaggctctggccttatctatagttatatttgggattcattctctttttttgggtagaaaaaggaaatttataacattagtattatttgcgtcaactttccatataactgctttgatttgttttcttctaatgactcctctattttcaaagaaattaagcaagataataagttatagcctattaattttcagtagcttctttttcgctttttctgaaaccatattaagtgcactccttgcaattttgccagaaggatccattgccagtgaaaaattaagtttttacttagcaaccgagcaatacaggccacagttatctattgggagtggcactattcttgacattatacttatttttctgatatgtgtaagttttaaacgaataaagaaatatatgctcgctaattataatgctgcaaatgagatattgcttattggttgctgtctttatatttctttcggtatttttatcgggaaaatgatgccagttatgactcgcattggttggtatggttttccatttgttatagtacttctttatattaacttgggttattcagaatattttaagaggtatataaataaaagagggtgtgggtatagcaaattattaattgctttttattttttgctacaaattttgcgaccattaacatatgattatagctattataatataatgcaccaggatactttgctgaataggtttgatgcattagatgatgcatcattaagacaatcagcgaagagaaaatgtttcgatttgggaaagataggatatggtttcttatgtagtatataatatcctgcattcattcggataatttcctatggaagtgtcctttgctctgtctgtcctcatttgttgaaattttatgttaataagaagctttagataaccacttaggaactgtatgtttgatctgtccaaaaattatattattgtaagtgcgacggcgctggcttccggaggtgcattaactatattaaagcaatttataaaacatgcatcacaaaattcaaatgactatattatgtttgtatctgcgggattggagttgccggtctgtgataacatcatttacatagaaaacacaccaaaaggatggttgaaaagaatatattgggattggttcggttgtcggaagtttatctcggaacataagattaacgttaagaaagtaatttctctacaaaattccagtttgaatgttccttacgaacagattatttacttgcaccagccaattccttttagtaaagttgattcttttttaaaaaatatcacatccgataacgtaaagctttttttatataaaaagttttattcctattttatatttaaatatgtgaatgccaatacaaccatcgtagtgcaaacgaattggatgaaaaaaggagtgctggagcaatgtgataaaattagtaccgaaagggtccttgttataaaacctgatatcaaagcatttaataatactaattttgatgtagatatggatgtatctgcaaaaacactcttatatccagcgacaccacttacctataaaaatcatttggtcattctgaaggcgttggttattttaaagaaaaagtattttatagatgatctgaaattccaagtgacttttgaaaagaataggtacaaaaattttgataagtttgtgcaattaaataacttaagcaaaaacgttgattatctcggcgttctttcatactcgaacttgcaaaaaaaatatatggcggcatctttaatcgtttttcctagctatatcgaatcatatgggttaccactcatcgaagctgctagtttaggaaaaaaaatcattagtagtgatcttccttatgcccgggatgttttaaaggattatagcggcgtagattttgtaatttacaataatgaagatggctgggctaaggcgttgtttaatgttttaaatggcaattcgaagctcaattttaggccttatgaaaaagatagtcgttcatcttggccacagttcttctctattttgaaataaggtgtattatgtttaatggtaaaatattgttaattactggtggtacggggtctttcggtaatgctgttctaagacgttttcttgacactgatatcaaagaaatacgtattttttcccgggatgaaaaaaaacaagatgacatgaggaaaaaatataataatccgaaacttaagttctatataggtgatgttcgcgactattcgagtatcctcaatgcttctcgaggtgttgattttatttatcatgctgcagctctgaagcaagtaccttcctgcgaattccacccaatggaagctgtaaaaacgaatgttttaggtacggaaaacgtactggaagcggcaatagctaatggagttaggcgaattgtatgtttgagtacagataaagctgtatatcctatcaatgcaatgggtatttccaaagcgatgatggaaaaagtaatggtagcaaaatcgcgcaatgttgactgctctaaaacggttatttgcggtacacgttatggcaatgtaatggcatctcgtggttcagttatcccattatttgtcgatctgattaaatcaggtagaccaatgacgataacagaccctaatatgactcgtttcatgatgactctcgaagacgctgttgatttggttctttacgcatttgaacatggcaataatggtgatatttttgtccaaaaggcacctgcggctaccatcgaaacgttggctattgcactcaaagaattacttaatgtaaaccaacaccctgtaaatataatcggcacccgacacggggaaaaactgtacgaagcgttattgagccgagaggaaatgattgcagcggaggatatgggtgattattatcgtgttccaccagatctccgcgatttgaactatggaaaatatgtggaacatggtgaccgtcgtatctcggaagtggaagattataactctcataatactgataggttagatgttgagggaatgaaaaaattactgctaaaacttccttttatccgggcacttcggtctggtgaagattatgagttggattcataatatgaaaattttagttactggcgctgcagggtttatcggtcgaaatttggtattccggcttaaggaagctggatataacgaactcattacgatagatcgtaactcttctttggcggatttagagcagggacttaagcaggcagattttatttttcaccttgctggggtaaatcgtcccgtgaaggagtgtgaatttgaagagggaaatagtaatctaactcaacagattgttgatatcctgaaaaaaaacaataaaaatactcctatcatgctgagttcttccatccaggctgaatgtgataacgcttatggaaagagtaaagcagctgcggaaaaaatcattcagcagtatggggaaacgacaaacgctaaatattatatttatcgcttgccgaatgtattcggtaagtggtgtcgaccaaattataactcctttatagcaactttctgccatcgcattgcaaatgatgaagctattacaattaatgatccttcagcagttgtaaatctggtgtatatagatgacttttgttctgacatattaaagctattagaaggagcgaacgaaactggttacaggacatttggtccaatttattctgttactgttggtgaagtggcacaattaatttaccggtttaaagaaagtcgccaaacattaatcaccgaagatgtaggtaatggatttacacgtgcattgtactcaacatggttaagttacctgtctcctgaacagtttgcgtatacggttccttcttatagtgatgacagaggggtattctgtgaagtattgaaaacgaaaaacgcgggccagttttcgttctttactgcgcatccaggaattactcggggtggtcattatcatcattccaaaaatgagaaatttattgtcatccgaggaagtgcttgtttcaaatttgaaaatattgtcacgagtgaacgatatgaacttaatgtttcctctgatgattttaaaattgttgaaacagttccgggatggacgcataacattactaataatggctcggatgagctagttgttatgctttgggcaaatgaaatatttaatcgttctgaaccagatactatagcgagagttttatcgtgaaaaaattgaaagtcatgtcggttgttgggactcgtccagaaattattcgactctcgcgtgtccttgcaaaattagatgaatattgtgaccaccttattgttcataccgggcaaaactacgattatgaactgaatgaagtttttttcaaagatttgggtgttcgcaaacctgattattttcttaatgccgcaggtaaaaatgcagcagagactattggacaagttatcattaaagttgatgaggtccttgaacaggaaaaaccagaagccatgttagtacttggcgatactaactcctgtatttcagcaataccagcaaagcgtcgaagaattccgatcttccatatggaggctgggaatcgttgttttgaccaacgcgtaccggaagaaactaacagaaaaatagttgatcataccgctgatatcaatatgacatatagtgatatcgcgcgtgaatatcttctggctgaaggtgtaccagccgatagaattattaaaaccggtagcccaatgtttgaagtactcactcattatatgccgcagattgatggttccgatgtactttctcgcctgaatttaacacctgggaatttctttgtggtaagtgcccacagagaagaaaatgttgatacccctaaacaacttgtgaaactggcgaatatacttaataccgtggctgaaaaatatgatgtcccggtagttgtttctactcatcctcgcactcgtaaccgcatcaacgaaaacggtattcaattccataaaaatatcttgcttcttaagccattaggatttcacgattacaaccatctgcaaaaaaatgcacgtgctgttttatcggatagtgggactattacagaagagtcctccattatgaacttccctgcactcaatatacgagaagcgcacgaacgcccggaaggcttcgaagaaggggcagtaatgatggtcggtcttgaatctgatcgcgttttacaggcattagaaattattgcaacacagcctcgtggagaagtacgcttacttcgtcaggttagtgactatagcatgccaaatgtttcagataaagttctgcgtattatccattcatatactgactacgttaaacgggttgtctggaagcaatactaatgaaacttgcattaatcattgatgattatttgccccatagcacacgcgttggggctaaaatgtttcatgagttaggccttgaattactgagcagaggccatgatgtaactgtaattacgcctgacatctcattacaagcaatttattctattagtatgattgatggtataaaggtttggcgtttcaaaagtggacctttaaaggatgtaggtaaggctaaacgtgccataaatgaaactcttttatcttttcgcgcatggcgcgcatttaagcacctcattcaacatgatacatttgatggtatcgtttattattccccctctattttttggggcgacttggttaaaaaaataaaacaacgatgccagtgcccaagctatctgatcctaagggatatgtttccacagtgggtcattgatgcaggtatgttgaaagccggttcaccaattgaaaaatattttaggtattttgaaaaaaagtcatatcagcaggctggccggataggggtaatgtctgataagaatcttgagatatttcgccagaccaataaaggttatccgtgtgaagttttacgtaattgggcctcaatgactcctgtgtctgccagcgatgattatcattcacttcgtcaaaaatacgatctaaaagataaagtcatttttttctatggcggtaatattgggcatgctcaggatatggcaaacttaatgcgccttgcgcgtaatatgatgcgttatcatgatgctcatttcctgtttatagggcagggtgatgaagttgagctgataaaatctcttgctgcagaatggaatttaactaatttcactcatctaccttcagtgaaccaggaagagtttaaattaattttatctgaagttgatgtcggcctgttctccctttcatctcgccattcttcacataatttccccggaaaattactagggtatatggttcaatcaatcccgatccttgggagtgtgaatggcggcaatgatttaatggatgtaattaataagcacagagccggtttcattcatgttaatggtgaagatgataaactgtttgaatctgcacaattgcttcttagtgattcagttttaagaaaacagctaggtcagaacgctaatgtgttgttaaagtctcaattttcggttgaatcggcggcacatactatcgaagtccgactggaggctggagaatgcgtttagttgatgacaatattctggatgaactttttcgcactgcagcaaattctgaacgtttgcgcgctcattatttattgcacgcatctcatcaggagaaggttcaacgtttacttattgcatttgtacgcgacagctatgttgaaccccattggcatgagttaccgcatcagtgggaaatgtttgtcgtcatgcaagggcaattagaagtttgtttgtatgagcaaaatggtgagatccaaaaacagtttgttgttggagacggtacgggaataagcgtcgtggaattttccccaggagatatacatagtgtcaaatgcctgtcaccaaaagcccttatgttggagataaaggaggggccatttgacccactcaaagctaaggctttttctaagtggttatagggcgatacaccaccgtttattcttctatcttattctatacatgctgggttaccatcttagcttcttcaagccgcgcaaccccgcggtgaccacccctgacaggagtagctagcatttgaccacccctgacaggattagctagcatatgagctcgaggatatctactgtgggtacccgggatccgtgtaggctggagctgcttcgaagttcctatactttctagagaataggaacttcggaataggaactaaggaggatattcatat

SEQ ID NO: 10 - protein, 19 aa, Artificial Sequence
  example signal sequence for EPA carrier protein
MKKIWLALAGLVLAFSASA

SEQ ID NO: 11 - DNA, 13043 bp, Artificial Sequence
  example O1A rfb locus nucleotide sequence - O1A-EPA production strain stGVXN4411 and stLMTB10217
atgacgaatttaaaagcagttattcctgtagcgggtctcgggatgcatatgttgcctgccactaaggcgatacccaaagagatgctaccaatcgtcgacaagccaatgattcagtacattgttgacgagattgtggctgcagggatcaaagaaatcctcctggtaactcacgcgtccaagaacgcggtcgaaaaccacttcgacacctcttatgagttagaatcactccttgagcagcgcgtgaagcgtcaactgctggcggaagtacagtccatctgtccgccgggcgtgaccattatgaacgtgcgtcagggcgaacctttaggtttaggccactccattttgtgtgcgcgacctgccattggtgacaacccatttgtcgtggtactgccagacgttgtgatcgacgatgccagcgccgacccgctacgttacaaccttgctgccatgattgcacgtttcaacgaaacgggccgcagccaggtgctggcaaaacgtatgccgggtgacctctctgaatactccgtcatccagactaaagagccgctggaccgtgagggtaaagtcagccgcattgttgaatttatcgaaaaaccggatcagccgcagacgctggactcagacatcatggccgtaggtcgctatgtgctttctgccgatatttggccggaactggaacgtactcagcctggtgcatggggacgtattcagctgactgatgctattgccgagctggcgaaaaaacaatccgttgatgcaatgctgatgaccggcgacagttacgactgcggcaaaaaaatgggctatatgcaggcgtttgtgaagtatggcctacgcaacctgaaagaaggggcgaagttccgtaaaggtattgagaagctgttaagcgaataatgaaaatctgaccggatgtaacggttgataagaaaattataacggcagtgaaaattcgcagcaaaagtaatttgttgcgaatcttcctgccgttgttttatataaaccatcagaataacaacgagttagcagtagggttttattcaaagttttccaggattttccttgtttccagagcggattggtaagacaattagcgtttgaatttttcgggtttagcgcgagtgggtaacgctcgtcacatcataggcatgcatgcagtgctctggtagctgtaaagccaggggcggtagcgtgcattaatacctctattaatcaaactgagagccgcttatttcacagcatgctctgaagtaatatggaataaattaagctagcgtgaagatacttgttactaggggcgcaggatttattggttctgctgtagttcgtcacattataaataatacgcaggatagtgttgttaatgtcgataaattaacgtacgccggaaacctggaatcacttgctgatgtttctgactctgaacgctatgtttttgaacatgcggatatttgcgatgctgctgcaatggcgcggatttttgctcagcatcagccggatgcagtgatgcacctggctgctgaaagccatgtggatcgttcaattacaggccctgcggcatttattgaaaccaatattgttggtacttatgtccttttggaagcggctcgcaattactggtctgctcttgatggcgacaagaaaaatagcttccgttttcatcatatttctactgacgaagtctatggtgatttgcctcatcctgacgaagtaaataataaagaacaattacccctctttactgagacgacagcttacgcgcctagtagtccttattccgcatcaaaagcatccagcgatcatttagtccgcgcgtggaaacgtacctatggtttaccgactattgtgactaactgttcgaataactacggtccttatcactttccggaaaaattgattccactagtaattcttaatgctctggaaggtaaggcattacctatttatggcaaaggggatcaaattcgtgactggctgtatgttgaagatcatgcgcgtgcgttatataccgtagttactgaaggtcaagcgggtgaaacctataacattggcggacacaacgaaaagaaaaacatcgatgttgtgctgactatttgtgatttgttggacgagatagtcccgaaagagaaatcttatcgtgagcaaattacttatgttgctgatcgcccagggcatgatcgccgttatgcgattgatgctgagaagattggtcgcgaattgggatggaaaccacaggaaacgtttgagagtgggattcgtaaaacggtggaatggtatttggctaatgcaaaatgggttgataatgtgaaaagtggtgcctatcaatcgtggattgaacagaactatgagggccgccagtaatgaatatcctcctttttggcaaaacagggcaggtaggttgggaactacagcgtgctctggcacctctgggtaatttgattgctcttgatgttcactccactgattactgtggtgattttagtaaccctgaaggtgtggctgaaacagtcaaaagaattcgacctgatgttattgttaatgctgcggctcacaccgcagtagataaggctgagtcagaacccgaatttgcacaattactcaatgcgactagcgttgaatcaattgcaaaagcggcaaatgaagttggggcttgggtaattcattactcaactgactacgtattccctggaaatggcgacacgccatggctggagatggatgcaaccgcaccgctaaatgtttacggtgaaaccaagttagctggagaaaaagcattacaagagcattgtgcgaagcacctaattttccgtaccagctgggtctatgcaggtaaaggaaataatttcgccaaaacgatgttgcgtctggcaaaagagcgtgaagaactagccgttattaatgatcagtttggtgcgccaacaggtgctgaactgctggctgattgtacggcacatgccattcgtgtcgcactgaataaaccggatgtcgcaggcttgtaccatttggtagccagtggtaccacaacctggtacgattatgctgcgctggtttttgaagaggcgcgcaatgcaggcattcctcttgcactcaacaagctcaacgcagtaccaacaactgcctatcctacaccagctcgtcgtccacataactctcgccttaatacagaaaaatttcagcagaattttgcgcttgtattgcctgactggcaggttggtgtgaaacgcatgctcaacgaattatttacgactacagcaatttaatagtttttgcatcttgttcgtgatggtggagcaagatgaattaaaaggaatgatgaaatgaaaacgcgtaaaggtattattttagcgggtggttctggtactcgtctttatcctgtgactatggtcgtcagtaaacagctattacctatatatgataaaccgatgatctattatccgctttctacactgatgttagcgggtattcgcgatattctgattattagtacgccacaggatactcctcgttttcaacaactgctgggtgacggtagccagtggggcctgaatcttcagtacaaagtgcaaccgagtccggatggtcttgcgcaggcatttattatcggtgaagagtttattggtggtgatgattgtgctttggtacttggtgataatatcttctacggtcacgacctgcctaagttaatggatgccgctgttaacaaagaaagtggtgcaacggtatttgcctatcacgttaatgatcctgaacgctatggtgtcgttgagtttgataaaaacggtacggcgatcagcctggaagaaaaaccgctacaaccaaaaagtaattatgcggtaaccgggctttatttttatgataacgacgttgtcgaaatggcgaaaaatcttaagccttctgcccgcggtgaactggaaattaccgatattaaccgtatctatatggaacaagggcgtttatctgttgccatgatggggcgtggttatgcgtggttagacacggggacacatcagagcctgattgaggcaagcaactttattgcaacaattgaagagcgtcaggggctgaaagtttcctgcccggaagaaattgcttaccgtaaagggtttgttgatgctgagcaggtgaaagtattagctgaacctctgaaaaaaaatgcttatggtcagtatctgctgaaaatgattaaaggttattaataaaatgaacgtaattaaaacagaaattcctgatgtactgatttttgaaccgaaagtttttggtgatgagcgtggtttcttttttgagagctttaaccagaaggtttttgaggaagctgtaggccgcaaagttgaatttgttcaggataaccattcgaagtctagtaaaggtgttttacgcgggctgcattatcagttggaaccttatgcacaaggaaaattggtgcgttgcgttgtcggtgaagtttttgacgtagctgttgatattcgtaaatcgtcatcgacttttggcaaatgggttggggtgaatttatctgctgagaataagcggcaattgtggattcctgagggatttgcacatggttttttagtgctgagtgagacggcggagtttttgtataagacgacaaattattatcatcctcagagtgatagaggaataaaatgggatgatccaagcatcaatatttcatggccagtcgattcacaagtgctgctatcagctaaagataataagcatcctccattaacaaagattgaaatgtatagttaagatcacgataaatcttggaagggttgcaaaattgaataaaatagtgagcaaaagtgaaataaggaacgtaatccacaatgctggctatatgatgattactcagatagctttatatgttgcaccattatttatactgagttatctgttaaaaacactgggggttgcacagtttggtaattatgccttaatactatcaatcgttgcatatttacagattataacggattatggtttttcttttagtgcaagtcgtgcgatctcacagaatagagaggacaaagaatatatatcaaaaatttatctgtcaactatgactatcaagttggcgatatgcgctttcttattcttattgctcatgctatttttaaatcttttgcctgtgcaagctgaattaaaacaaggaatattatatggatatcttcttgtaataggaaatactttccaaccacaatggtttttccaaggtatcgaaaaattaaaaatcatagccctttctaatgttatatcaagatgcgccgcgtgtttacttgtatttatctatgtgaggaatagcgaggatttacaaaaagcacttttagtacagtcacttccattagtaatttctgcgattggattaaatatatttatattgaaatatatcaatattatttttccggaaaaaaaattatttaaggtaattttaaaagaaggtaaggatttttttcttgcatcactttattctgttattctcaataatagtggcatttttctattagggatttttactaatcctgttattgttggtgtatatgccgccgctgaaaagatagtcaaggccgtattgtcgctatttacaccactgacgcaagctatatatccttataattgtcgtaagttttcactatccgtatttgacggcattgaggcagcaaaaaaaactggtataccaattataattttagcatttatagctgctgttatcgttgcaattaccttacctgttgcaatcgactatcttaattttccaaaagaaacaatttttgtaggtcaaatattaagtgcatggatcttttttggtgttcttaataatgtattcggcattcagatattgagtgcatcaggaagaagtaaaatatatagtaggatggtattcgtatcagcgcttataacattacttttgattactctattattgcagttttgtaacgccactggagtggcatgtgcaatattattgggtgaaatgttcttatcaatattgttacttaagcgatataaaaaaataatttaaggaatagttatgaagaagttattattagtgttcggtactaggcctgaagcaataaagatggcctctatcattgaattattaaaaaaagattgtagattcgaatataaaatatgtgtgacaggccaacataaagagatgcttgatcaagttatgcaagtatttgatgttaaacctgattataatttacggattatgcagcctgggcaaacattagtatctatagcaacaaatatactctcacggttaagtgaagttttaattatagaaaagccagatattatacttgtgcatggggatacaacgactacccttgctgctactttagctgggtattaccaccaaataaaagtttgtcatgtggaagcaggattaagaacaggggatatttactctccttggcctgaagagggcaatcgtaaagttacaggggcattagcatgtattcatttcgccccaacagagagatcaaaagataatctcctgagggagggggtcaaagtaaataatatatttgtaacgggtaataccgtcatcgactctttatttattgcaaaagatatcatagataatgaccctaatataaagaacgctttacataataaatttaattttcttgataaaagccgacgagtagtacttataacaggtcatcgaagagaaaatttcgggaaaggttttgaagatatatgctttgcaataaaggaattagctttcatttatcctaatgtagattttatttatccggtgcatcttaatcccaatgtaatggaaccagtacatcgtatattagataatatatgtaatatttaccttattgagcccttggattatttgccttttgtttatttaatgaatgagtcatatttaatattgactgattcaggggggatacaagaagaagcgccttcgttaggtaaaccggttttggttatgcgtgatactactgaacgccctgaggcggttgaggctggtactgttgtattagtggggacttctaagataaaaatagtaaataaagtaacggagctattaaacaatgctgatatctacaatgctatgtctctgttacataatccatatggcgatggaacagctgctcaaaaaattcttaatgtgctcgcccaagagctaatttaatttaagctaaaaatatgttattaattattgctgattatccaaacgaaatgaatatgcgcgagggagctatgcaacgaatagatgcgatagactctctcattcgagatcgcaagcgagtgtatttgaatatttcattcaaaaagcatctagttcgctcaaatagttcctttaataatgttatagttgaaaatctaaatgcaattattcacagaaacatcataaaacagtacatgcaaaaatcaacaactatatatgttcattctgtttataatttattaaaggttataacgctcattgatctaaaaaaaacaattcttgatatacatggtgttgtaccggaagaacttttggcagataataaaaaattacttagtaaagtatataacatggtggaaaaaaaaggtgtccttggatgcaaaaaattaatacacgtcagtacagaaatgcaaaaacactatgaagcaaaatatggagtaaacttggctgaaaggtcaatagtgctcccgatttttgaatataaaaatataacccaatcgcaaaacaaatggacagaaaataaaatacgaagtatctatcttggaggattacaaacatggcaaaatattgataaaatgattcaagtttgtgatgacacagtgataaacaatgaagcaggtaagtatgaattcaactttttcatcccacagagtaacttggaagggtttatagataaatattcgttaaaattacataatatcaatgctaatgcatctacgctatcacgtgatgaagtaattccctttctaaaagaatgtcatattggttttgtattgcgcgatgatataatagtaaacagagttgcgtgccctacaaaattggttgaatatttagagtgtggtgtcgttccagttgtgctctccccacttataggtgatttttattcgatgggatatcaatacattactacagaggaaatggctaacagaagtataagtttgttggatcttgaaaaaatggctgcacataatttacaaattttgacttcttatcagaagagaacctacaaggcacagaaagaacttattgctcaactgtgctgaattttttacatatataaaattatgtaagcatatcgcgggtcaggtaattgtatgcgtatcaaatataaagataacggttatatattatgttttctattatgtttcattttgagctacttagttttactcaaatctgactactttcctgctgattttctgccatatacagaaatatacgatgggacatacggagaaatcaataatattgagcctgcctttttatatttaacacggttgtttcattatttaaatttcccctatatattttttgcaatgttagtttgtgccttatgtttaagttggaaaataaaatatgcaagaaaaataattaaagatagttatatatatttgttcttgtatgtatatgtatcattttatgtgtttttgcatgaaatgactcaattgcgcatagcaattgcagtcactatgtgctatgtgtcggtttattattacttttataaaaattgtattaaacatgcactgccatggatggtgttggctattttgtttcattacagcgccttgcttttatttatgtcattatttatatacagttataggaggttattaatagtaattatagggtttgtaatatgtatgagctttttaaacgtgtatgcagatacaattgcactatatttgccaaatgaaaaaatagtaaattatttatatagtatttcatcatcattagacaatagaaatgatttggcaatattcaacctgaataatataatatttttatcaatatttattttgatcttttatcttagccgatatataaaattaaatgataatgaggcgaagtttattaagtatgtgcaatgttcaggaatattagccttttgtattttctttctggctagtggagtcccggtcattgcttatcgaactgcagagttgctgcgaatattttatccgatggctttagtattaatcctttcgcatataaaaaataataatatgcgttattttattgcagtcattatagttatcctttcaggcttaatgttgtttataacactaagggctgtatcaatagttggtcaaggattataaaatgaatgttgctattttgttgtctacgtataatggcgaaaaatatttagaggaacaactggattcattgctgcttcaaagttatcaggattttgtagtgtatatccgtgatgacggatcatctgatagaactgtaaatataataaaccaatacgtaatgaaagataacagatttattaacgtgggtaattcagaaaatcttggttgtgctgcttcgtttattaatttattaagaaatgcttcagccgatatttatatgttttgtgaccaagatgattattggcttccgaataaattacagcgtgctgtggattatttttcggctattgatcctttacaacctaccttgtatcattgcgatctaagcgttgttgatgaaaaacttaatattatacaaaattcatttttgcagcatcagaaaatgtcagcgtatgattcaatgagaaaaaataatcttttcatacaaaattttgttgttggttgttcatgtgctgttaatgcttcacttgcggaatttgttctttcgcgaattggagagcagcatgtaaaaatgatagctatgcatgactggtggttagccgtgactgcaaaactttttggtcgaatccattttgataatactcaaacgattctttatcgacaacatcagggcaatgtattaggtgcaaaatcatcaggtatgatgcgttttattcgattaggattaaatgggcaagggatttcgcgagtagtatcttttagaaaaaaagtttgtgcgcaaaataagcttcttttagatgtctatgataaagatttaaatcttgagcaaaaaaaatctatcaggcttgtaattgagggccttaaagagaactcttcaattgctgaccttttaaaatgtttctatcatggtagctatatgcaaggttttaaacgtaatcttgccttaatatattcagttctttacacaaaaaaaagaagatagtgtatccttatgaaaaaaattgctattatcggtactgttggcataccagcatcatatggcggatttgaaacattagttgaaaatttaacaagatacaattcctcgggagttgaatataatgttttttgttcatcgtttcactacaaatcccaccaaaaaaaacataatggggcccgtttaatttatattccgcttaaagccaatggatggcagagcattgcgtatgacataatttcgttagcatattctatttttttgaagcctgatgtgattctgattttaggggtttctggttgttcatttttgcctttcttcaaactcttaacacgcgctaagtttattactaatattgatggcctggaatggcgaagagataaatggaattcaaaagtgaaacgtttcttaaaattttcagaaaaaatcgcagttcaatattcggatgtcgttattacggataatgaggcaatttctgagtacgtttttaacgagtataataaagatagccgagttattgcctatggaggggatcatgcatggttaaatactgaggatgtatttacaacaagaaattataaaagcgattactacctttctgtatgtcgtatcgaacccgaaaacaatgtagaattaattttaaaaacattttcaaagctaaaatataaaataaaatttattggaaattggaatggcagcgagtttggaaagaaacttaggctgcattattctaactatccaaatattgaaatgattgatccgatttatgatcttcaacaattatttcacttacgaaataattgcataggatatatacatggtcattcggctggaggaacaaacccttctttagtcgaggcaatgcattttagtaaacctatatttgcatatgattgtaagtttaataggtacactactgaaaatgaagcatgttatttttctaatgaatctgacctcgcagagaaaatcataatgcattgtgagctatcattaggtgtctctggcacgaaaatgaaagaaattgctaaccagaaatacacttggagacgaatagcagaaatgtatgaggattgctattaactctgttaaacttcaaatcttttacaatatatggcatgactataagcgcattaattgtttttcaagccgctctcgcggtgaccaccccctgacaggggatccgtgtaggctggagctgcttcgaagttcctatactttctagagaataggaacttcggaataggaactaaggaggatattcatatggataaagccgtaagcatataagcatggataagctatttatactttaataagtactttgtatacttatttgcgaacattccaggccgcgagcattcagcgcggtgatcacacctgacaggagtatgtaatgtccaagcaacagatcggcgtagtcggtatggcagtgatgggacgcaaccttgcgctcaacatcgaaagccgtggttataccgtctctattttcaaccgttcccgtgagaagacggaagaagtgattgccgaaaatccaggcaagaaactggttccttactatacggtgaaagagtttgtcgaatctctggaaacgcctcgtcgcatcctgttaatggtgaaagcaggtgcaggcacggatgctgctattgattccctcaaaccatatctcgataaaggagacatcatcattgatggtggtaacaccttcttccaggacactattcgtcgtaatcgtgagctttcagcagagggctttaacttcatcggtaccggtgtttctggcggtgaagagggggcgctgaaaggtccttctattatgcctggtggccagaaagaagcctatgaattggtagcaccgatcctgaccaaaatcgccgccgtagctgaagacggtgaaccatgcgttacctatattggtgccgatggcgcaggtcactatgtgaagatggttcacaacggtattgaatacggcgatatgcagctgattgctgaagcctattctctgcttaaaggtggcctgaacctcaccaacgaagaactggcgcagacctttaccgagtggaataacggtgaactgagcagttacctgatcgacatcaccaaagatatcttcaccaaaaaagatgaagacggtaactacctggttgatgtgatcctggatgaagcggctaacaaaggtaccggtaaatggaccagccagagcgcgctggatctcggcgaaccgctgtcgctgattaccgagtctgtgtttgcacgttatatctcttctctgaaagatcagcgtgttgccgcatctaaagttctctctggtccgcaagcacagccagcaggcgacaaggctgagttcatcgaaaaagttcgtcgtgcgctgtatctgggcaaaatcgtttcttacgcccagggcttctctcagctgcgtgctgcgtctgaagagtacaactgggatctgaactacggcgaaatcgcgaagattttccgtgctggctgcatcatccgtgcgcagttcctgcagaaaatcaccgatgcttatgccgaaaatccacagatcgctaacctgttgctggctccgtacttcaagcaaattgccgatgactaccagcaggcgctgcgtgatgtcgttgcttatgcagtacagaacggtattccggttccgaccttctccgcagcggttgcctattacgacagctaccgtgctgctgttctgcctgcgaacctgatccaggcacagcgtgactattttggtgcgcatacttataagcgtatcgataaagaaggtgtgttccataccgaatggctggattaa

SEQ ID NO: 12 - DNA, 13790 bp, Artificial Sequence
  example O2 rfb locus nucleotide sequence - O2-EPA production strain stGVXN4906
atgacgaatttaaaagcagttattcctgtagcgggtctcgggatgcatatgttgcctgccactaaggcgatacccaaagagatgctaccaatcgtcgacaagccaatgattcagtacattgttgacgagattgtggctgcagggatcaaagaaatcctcctggtaactcacgcgtccaagaacgcggtcgaaaaccacttcgacacctcttatgagttagaatcactccttgagcagcgcgtgaagcgtcaactgctggcggaagtacagtccatctgtccgccgggcgtgaccattatgaacgtgcgtcagggcgaacctttaggtttaggccactccattttgtgtgcgcgacctgccattggtgacaacccatttgtcgtggtactgccagacgttgtgatcgacgatgccagcgccgacccgctacgttacaaccttgctgccatgattgcacgtttcaacgaaacgggccgcagccaggtgctggcaaaacgtatgccgggtgacctctctgaatactccgtcatccagactaaagagccgctggaccgtgagggtaaagtcagccgcattgttgaatttatcgaaaaaccggatcagccgcagacgctggactcagacatcatggccgtaggtcgctatgtgctttctgccgatatttggccggaactggaacgtactcagcctggtgcatggggacgtattcagctgactgatgctattgccgagctggcgaaaaaacaatccgttgatgcaatgctgatgaccggcgacagttacgactgcggcaaaaaaatgggctatatgcaggcgtttgtgaagtatggcctacgcaacctgaaagaaggggcgaagttccgtaaaggtattgagaagctgttaagcgaataatgaaaatctgaccggatgtaacggttgataagaaaattataacggcagtgaaaattcgcagcaaaagtaatttgttgcgaatcttcctgccgttgttttatataaaccatcagaataacaacgagttagcagtagggttttattcaaagttttccaggattttccttgtttccagagcggattggtaagacaattagcgtttgaatttttcgggtttagcgcgagtgggtaacgctcgtcacatcataggcatgcatgcagtgctctggtagctgtaaagccaggggcggtagcgtgcattaatacctctattaatcaaactgagagccgcttatttcacagcatgctctgaagtaatatggaataaattaagtgaaaatacttgttactggtggcgcaggatttattggttcagctgtagttcgtcacattataaataatacgcaggatagtgttgttaatgtcgataaattaacgtacgccggaaaccgggaatcacttgctgatgtttctgattctgaacgctatgtttttgaacatgcggatatttgcgatgcacctgcaatggcacggatttttgctcagcatcagccggatgcagtgatgcacctggctgctgaaagccatgttgaccgttcaattacaggccctgcggcatttattgaaaccaatattgttggtacttatgtccttttggaagccgctcgcaattactggtctgctcttgatagcgacaagaaaaatagcttccgttttcatcatatttctactgacgaagtctatggtgatttgcctcatccagatgaagtaaataatacagaagaattacccttatttactgagacgacagcttacgcgccaagcagcccttattccgcatccaaagcatccagcgatcatttagtccgcgcatggaaacgtacgtatggtttaccgaccattgtgactaattgctcgaacaactatggtccgtatcacttcccggaaaagcttattccattggttattcttaatgcactggaaggtaaggcattacctatttatggcaaaggggatcaaattcgcgactggttgtatgtagaggatcatgctcgtgcgttatataccgtcgtaaccgaaggtaaagcgggtgaaacttataacattggcggacacaacgaaaagaaaaacatcgatgttgtgctgactatttgtgatttgttggatgagattgtaccgaaagagaaatcttatcgtgagcaaattacttatgttgctgatcgcccagggcatgatcgccgttatgcaattgatgccgataaaattagccgcgaattgggctggaaaccacaggaaacgtttgagagcgggattcgcaaaacggtggaatggtatctggctaatacaaattgggttgagaatgtgaaaagcggtgcttatcagtcatggatcgaacaaaactatgagggccgtcagtaatgaatatcctgcttttcggcaaaacagggcaggtgggttgggaactgcagcgtgctctggcgccgctgggtaatctgatcgctcttgatgttcactccactaattattgtggagatttcagcaaccccgaaggtgtggcagaaaccgtcaaaaaaattcgtcctgacgttattgttaatgctgctgctcacactgcagtagataaagcagaatcagaaccggatttcgcacaattacttaacgcgacaagcgtcgaagcgattgcaaaagctgctaatgaagtcggggcctgggttatacactactctactgattatgttttcccaggcagtggtgacgcgccatggctggaaacggatgcaacagcaccgctaaatgtttacggtgaaacaaaattagctggggaaaaggcattacaagaacattgcgcaaagcatcttattttccgtaccagctgggtatacgctggtaaaggaaataactttgctaaaacgatgttgcgtttggcaaaagaacgcgaagaactggctgtgataaacgatcagtttggcgcaccaacaggtgctgaattgctggctgattgcaccgctcatgccattcgcgtggcattaaaaaaaccagaagtcgctggcttgtaccatctggtagcaagtggcacaacaacctggcacgattatgctgcgctggtttttgaagaggcgcgcaaagcagggattaatcttgcacttaacaaacttaacgccgtgccaacaacggcctatcccacaccagcccgtcgaccccataactctcgcctcaatacagaaaagtttcagcagaactttgcgcttgtcttgcctgactggcaggtgggcgtgaaacgtatgctcaacgaattatttacgactacggcaatttaacaaatttttgcatctcgctcatgatgccagagcgggatgaattaaaaggaatggtgaaatgaaaacgcgtaaaggtattattctggctggtggttccggcactcgtctttatcctgtgacgatggcagtgagtaaacaattgctgccgatttatgataagccgatgatttattatccgctttcaacgcttatgttagcgggtattcgcgatattcttattattagtacgccacaggatacaccgcgtttccaacaattattgggggacgggagccagtggggtcttaatctacagtataaagtacaaccgagtccggatggcctggcgcaagcgtttattattggcgaagactttattggtggtgatgattgtgcactcgtacttggcgataatatcttctatggacacgacttgccgaaattgatggaagctgctgttaacaaagaaagcggtgcaacggtatttgcttatcacgttaatgatcctgaacgctatggtgtcgtggagtttgataataacggtacggcaattagcctggaagaaaaaccgctggagccaaaaagcaactatgcggttactgggctttatttctatgacaatgacgttgtggaaatggctaaaaaccttaagccttctgcccgtggcgaactggaaattaccgatattaaccgtatttatatggaacaaggacgtttgtctgtagccatgatggggcgtggctatgcatggttggatacagggacgcatcaaagccttattgaagcaagtaacttcattgcaacaattgaagagcgtcagggattaaaggtatcttgcccggaagagattgcttaccgtaaagggtttattgatgccgagcaggtgaaagtattagccgaaccgcttatcaagaatcaatatggtcaatatttgctgaaaatgatcagcgaatagtatatgggaactcaatgatggatattaaattaatctctttgcaaaaacatggggatgagcgcggtgcattaattgctcttgaagagcaacgaaatatacctttcgaagtcaaaagaatatattacatacttgagactcttaatggagtaagacgcggatttcatgcgcacaaggttactcgtcagttagctattgtagtcaagggagcttgtaaatttcatctggataatggtaaagaaacaaagcaggtggaacttaatgatccaacaattgcgttgctgatagaaccctatatatggcatgaaatgtatgattttagtgatgattgtgtgctgcttgtaattgcggatgatttctataaagagtctgattatatccgcaattatgatgattttattagaagagtaaattcaattgagaattcataagctaagtgacgtccagacaacatcaattggtgatggaacaactatctggcagtttgttgtgatactaaaaggtgctgtaattggtaataattgcaacatctgtgcaaataccttaattgaaaataacgttgtaattggtaacaatgtcacagtcaaaagcggtgtgtatatttgggatggcgttaaaatagaggataatgtttttattggtccttgtgtagcatttacaaatgataagtatcctcgctctaaagtctatcctgatgaatttttgcaaacaataatacgcaaaggagcatcaataggtgctaacgcaaccatcctgccaggaattgaaattggtgaaaaagcaatcgttggtgcggggagtgttgtaaccaaaaatgtaccgccatgcgcaatagtagtaggtaatccagctcgatttattaaatgggtagaggataatgaataaaattgattttttagatctttttgcaattaaccagcgacagcacaaagaattagtctctgcgtttagtagggtgctagattctggttggtatatcatgggcgaagaacttgagcagttcgagaaagagttcgcagaatactgtggagttaagtattgcattggtgtagcaaatggccttgatgcgttgatactagtattgagggcatggaaagaacttggctatcttgaagacggtgacgaggtattagtaccggcaaatacatatattgcttctattcttgctataacagagaacaaacttgttcctgttcttgttgaaccagatatagaaacttataatattaatcctgctttaattgaaaattacattacggaaaaaactaaagcaatattaccggttcacttatatggtctattgtgcaatatgccagaaattagtgcaatcgccagaaaatataatctgttgattcttgaagattgtgcacaagcacatggtgcaatacgtgatggtcgcaaagctggagcttggggggatgctgcaggatttagtttttatccaggaaaaaaccttggagctttgggggatgcgggagctgttactacaaataatgcagaattatcctcaactataaaagctttgcgaaattatgggtcacataagaaatatgaaaatatttatcagggattgaatagtcgattggatgaactgcaagcagccttattgcgtgtaaaaatccatacattaccggaagatactgcgattcggcaaaggattgctgaaaaatatattcgtgaaataaaaaaccctgcgattacgttaccagtgtacgaaggccaaggtgcgcatgtttggcatttatttgtagtaagaatcgctaatcgtgaaaaattccagtcatacttattagagaagggtatcaaaaccttaattcactatccattaccaccccataagcagcaagcatatcaaaatatgtctagccttagccttccaattactgagcaaattcatgatgaagtcatttctttacctataagtccggtaatgagtgaagatgatgtcaattatgtaatcaaaatggtcaatgattacaagtaatgaaaaaatttcttcaggtaactatattatccgctatctatacattcattaaaatgattgcgggttttatcatcggtaaggtagtagcaatttatacagggccatcaggggtagcaatgcttggccaagtgcaaagtttaatcacaatagttgcaggtactacctctgcacctgtaagcacaggccttgttcgatatactgcggaaaattggcaagaaggacaagaagcatgcgcgccatggtggcgcgcatgcttaagggttactctgtttttattcttgcttattattcccgttgttattatattgtcgaaaaatattagtgagttactttttagcgatggacaatacacatggttaatcattttcgcatgttgtatattgccattctccattataaatacattgatcgcttcagttttaaatggtcaacaattttataagcaatatatattggttgggatgttttctgtattcatttctactatgtttatgattttgttgattgtagcttataatcttaaaggtgcattgattgccacagctataaatagtgctattgctggtcttgtattggttttattttgtctcaataaatcttggtttagatttaaatattggtggggtaaaacggataaagacaaaattataaaaattattcattatactctgatggctctggtttctgttatctccatgcctacagcattgatgtgtattagaaaaatattgattgctaaaactggttgggaggatgcagggcaatggcaggccgtatggaagatatctgaggtttatcttggtgttgtgacaattgctttgtcaacatatttcttaccaagattgacaattataaaaacaagtttccttataaaaaaagaagtaaatagtactatattatacataatatctattacttcattcatggcgttgagtatctatttattccgcgatttggtaataacagttttatttactgaacagtttcgctcagctcgtgaattatttttattacaacttataggggatgtaataaaaattgctgggtttctttatgcataccctcttcaaagtcaggggcatactaaactattcatcagttcagaagtgattttttctatgctctttatcattaccacctatatttttgttgtaaattatggagtacatggtgctaacataagttatgtcattacatatagtttatattttgtgtttgcatttgtgtttactaattttattaatgttagaagaaataattaaaaacagaggttgaattttgaaaataattatacctgtcttaggatttggcagggctggtggtgaaagagttctttctaagctggcaactgaattgatgaattatggacatgatgtaagttttgttgttccagataatagaactaatccatattatgctaccacagcaaaaattgtcacgagtaaatctagtcaaaaccgtgtaaaaatattgagaatcattaaaaattactataatctgtggcgtaaatgcatagagttaaatcctgatgctgtagttgctagttttcatttgactgcctatcttgtcgcattattaccaatcacccgtcgtaagaaatattattatattcaggcgtatgaagttaatttttttgataatataatatggaaattaatagcgggtttaacatattatttaccgcttaaaaaaatactaaatagtcctaatttgcttcctcataaacatgatgattttataggagtagttcctgcaggagtagatttaaacgttttctatccgaaaccatcaaataggttattaaatggtcacacatcaatagggattattggtagaaaagagaagcacaaaggaactagcgaaattatttcagtattgtgttcactggaaaataaagctggaattataatcaatattgcgatctatcttgaagaagttgataagcagcgtttaatcgctgccgggtttcaggttaatttttttccgattacttctgatttagaattggcatccttttatcgaagcaatgacatcatgattgctgttgggttaattgaagatggcgctttccattatccttgtgctgaatcaatggcttgtggttgtcttgttatttcaaattatgcgccacttactgaaactaacagtgtacttaaattagtcaagtttgatgcttgcaaacttggtgaagcaattaatctttgtctcaatcttgacctagaagaaaaaagcaaagaaatccaatctaatatttctgtgttgaataaatatgactggaaaattgttggtgaaactttcaatagtttattgttagatgcaaataaatagtatacgttgatggggaaaatatgaatattgttaaaactgatattccagatctgatcgttcttgaaccaaaagtgtttagtgatgaacgcggcttttttatggagagttataatcagattgaatttgagaaggcaataggaaggcacgtaaattttgttcaggataatcattcaaaatctagtaaaggcgtactacgtgggttgcattatcaattagcaccgtatgcacaggctaaattagttcgatgtgttgtaggtcaggtatttgatgttgctgttgatcttagaaaaaattcaccaacgttcaaaaaatggtttggaataaccctttccgcagaaaataaacgacaattatggatacccgaaggatttgctcatggtttcttggtgaccagtgatgaagctgagttcatttataagacaactaactactatgctcctggtcatcagcaagcaattatttacaatgatcctattttaaacatcgattggcctttctgcagtagtgctctgtcattatcacaaaaagatcaagaagcaaaattattttcagaattattggacagtgaactgttctaataaagtgtgccaccttatccgtctgaaggataggtggttgcttatatttttttgagtatgtttgtataatgacagaaaatagtccgaaatataaacacgataaaagcttaataagttttatctacttattttttatatttacacttattgtaggctttattatcgcaaatacccagtttttggggcgaagtagagactatgataattatatacagatcttttctggtaaagaaggggagggggttcttgaattattttatcgcggattgatgttaataacgaccagctatgaaactatcatttttataattttaacatgttctttttttataaaggcaaggtttctcgctaactattcgcgtaatttttcaggcttgaccttattctttatttattatgcaagcgttgcactttgggttttagattatactcaattcagaaatggtctatgtatttccattttaatgttttccgtatactatttatttataaataaaccgacttatttttatttctcggtattatgtgcaattgcaactcattggtctgctttgccttttttgcttttatatccttttgtctattcaacaaaaataagacgccttggttatttttgtttcagtattcttgttttgattgcgatctcaggagaaggaaaagagatcatatcttttataagaaattttggagtgggacaaaaaataggaaatgaagctggtgtaaatttaataaattcattatcccttaccgctatttcctggtttattattagttacatatcaagcattggaaatgaaaggagaaatttaaggcttttcttttgttatggtgtcatgcaatacgtgacttttagccttttctctctacctgttatggctttccgtattttggaaatgtattttttccttatgctaaccattggggtgtttattaagcaaaaaaagaattattattttattttttgcaaagtgttaattttattgtatctaacatactattatcatatggtctttggagtgattaatgtgtaaggctaaggtgttggctataattgttacttacaacccggaaattattcgattgacggaatgtattaactctttagccccacaagttgagagaataattcttgtagataatggctcaaataatagtgatttgataaaaaatatcagtattaataaccttgaaattattttactttcggaaaacaaaggcattgcatttgctcagaaccatggtgttaagaagggcctggaagcaaaagagtttgactatttatttttctcagatcaggatacttgctttcctagcgatgttattgaaaaacttaagagtacatttacgaaaaataataaaaaaggtaaaaatgttgcttgtgcttctcctttttttaaagaccatcgttcaaattatatgcatccgtcagtcagcctaaatatttttacgagtacaaaagttatatgtagtgaagtagacgatgatctttatccctcgcatgttattgcttctgggatgttaatgtctcgtgaagcatggcgcgtcgtcggaccattttgtgaaaaactctttatagactgggttgatacagaatggtgttggcgtgcattagctaataatatgattattgttcagacaccatcagtcatcatttctcatgaacttgggtatgggcagaaaatttttgctggtcgatctgttacaatacataattctttcagaaatttttataaaatacgcaatgcaatatacttaatgctgcattcaaattatagcttcaagtatcgttatcatgctttttttcatgcgacaaagaatgttgtatttgaaattttatattcgaaagaaaaattaaattcactgaaggtttgttttaaagctgtacgtgatggtatgttcaataatttttaatacgaaaatagttaggctcaaggtgtttaaatggaagaaaataatatgaagacggtcgctgtagttggcacagtgggtgttcctgcttgttatggtgggttcgaatcacttgttcagaatctaattgattatcaatctgatggtatacaatatcagatattttgctcttcaaaaaaatatgataaaaaatttaaaaattataaaaatgcagaattaatctatttgccgataaatgccaatggcgtctctagcataatttatgatattatgtgtttaattatttgtttattcaaaaggccagatgttgttttaatattgggggtgtctggttgtttatttctaccaatttataaactattttcaaaatcaaagattattgtcaatattgatgggcttgaatggcgtagaaataaatggggaacgtttgctaagaaatttcttaaaatatctgaggcgatatctattagaatagctgatattatcatttcagataatcaagcaatagctgattatgtggaaaataagtacaagaaaaaaagtgtagttatagcttatggcggagatcatgccactaatcttagtacaccgatagacaatgatcaaaaaaaagaaggttattatttggggctttgtaggatagagcctgagaataatatagaaatgattctgaatgccttcattaatacagataaaaaaattaaatttatgggtaattgggataacagcgagtatggacgccagctaaaaaaatattattcaaactatccaaatatcaccctactagaacctaactataatattgaagagctttataaactaagaaaaaattgtcttgcatacattcatggacactcggctggtggaacaaacccttctttagttgaagcgatgcattttaatattcctatttttgctttcgattgtgactttaatcgttacacaactaacaatttagctcattactttaatgattctgaacaacttagcttattagcagaaagtttgtcttttggaaatcttaaatgtcgagtattagatttaaaaaattatgctgaagatatgtataactggaggcatatagctgctatgtatgaatctatttattaaacgcattaacaataatataattgaccttatatagcagggaaagatcacgtaacgctgcggcgcgccgatccccatatgaatatcctccttagttcctattccgaagttcctattctttctagagaataggaacttcggaataggaactaaggaggatattcatatggataaagccgtaagcatataagcatggataagctatttatactttaataagtactttgtatacttatttgcgaacattccaggccgcgagcattcagcgcggtgatcacacctgacaggagtatgtaatgtccaagcaacagatcggcgtagtcggtatggcagtgatgggacgcaaccttgcgctcaacatcgaaagccgtggttataccgtctctattttcaaccgttcccgtgagaagacggaagaagtgattgccgaaaatccaggcaagaaactggttccttactatacggtgaaagagtttgtcgaatctctggaaacgcctcgtcgcatcctgttaatggtgaaagcaggtgcaggcacggatgctgctattgattccctcaaaccatatctcgataaaggagacatcatcattgatggtggtaacaccttcttccaggacactattcgtcgtaatcgtgagctttcagcagagggctttaacttcatcggtaccggtgtttctggcggtgaagagggggcgctgaaaggtccttctattatgcctggtggccagaaagaagcctatgaattggtagcaccgatcctgaccaaaatcgccgccgtagctgaagacggtgaaccatgcgttacctatattggtgccgatggcgcaggtcactatgtgaagatggttcacaacggtattgaatacggcgatatgcagctgattgctgaagcctattctctgcttaaaggtggcctgaacctcaccaacgaagaactggcgcagacctttaccgagtggaataacggtgaactgagcagttacctgatcgacatcaccaaagatatcttcaccaaaaaagatgaagacggtaactacctggttgatgtgatcctggatgaagcggctaacaaaggtaccggtaaatggaccagccagagcgcgctggatctcggcgaaccgctgtcgctgattaccgagtctgtgtttgcacgttatatctcttctctgaaagatcagcgtgttgccgcatctaaagttctctctggtccgcaagcacagccagcaggcgacaaggctgagttcatcgaaaaagttcgtcgtgcgctgtatctgggcaaaatcgtttcttacgcccagggcttctctcagctgcgtgctgcgtctgaagagtacaactgggatctgaactacggcgaaatcgcgaagattttccgtgctggctgcatcatccgtgcgcagttcctgcagaaaatcaccgatgcttatgccgaaaatccacagatcgctaacctgttgctggctccgtacttcaagcaaattgccgatgactaccagcaggcgctgcgtgatgtcgttgcttatgcagtacagaacggtattccggttccgaccttctccgcagcggttgcctattacgacagctaccgtgctgctgttctgcctgcgaacctgatccaggcacagcgtgactattttggtgcgcatacttataagcgtatcgataaagaaggtgtgttccataccgaatggctggattaa

SEQ ID NO: 13 - DNA, 13777 bp, Artificial Sequence
  example O6A rfb locus nucleotide sequence - O6A-EPA production strain stGVXN4112 and stLMTB10923
atgacgaatttaaaagcagttattcctgtagcgggtctcgggatgcatatgttgcctgccactaaggcgatacccaaagagatgctaccaatcgtcgacaagccaatgattcagtacattgttgacgagattgtggctgcagggatcaaagaaatcctcctggtaactcacgcgtccaagaacgcggtcgaaaaccacttcgacacctcttatgagttagaatcactccttgagcagcgcgtgaagcgtcaactgctggcggaagtacagtccatttgcccgccgggcgtgacaattatgaacgtgcgtcagggcgaacctttaggtttgggccactccattttatgtgcacgacctgccattggtgacaatccatttgtcgtggtgctgccagacgttgtgatcgacgacgccagcgccgacccgctgcgctacaaccttgctgccatgattgcgcgcttcaacgaaacgggccgcagccaggtgctggcaaaacgtatgccgggtgacctctctgaatactctgtcatccagaccaaagagccgctggaccgcgaaggtaaagtcagccgcattgttgaattcatcgaaaaaccggatcagccgcagacgctggactcagacatcatggccgttggtcgctatgtgctttctgccgatatttggccggaacttgaacgcactcagcctggtgcatgggggcgtattcagctgactgatgccattgccgaactggcgaaaaaacagtccgttgatgccatgctgatgaccggcgacagctacgactgcggtaaaaaaatgggttatatgcaagcgttcgtgaagtatggactacgcaacctcaaagaaggggcgaagttccgtaaagggattgagaagctgttaagcgaataatgaaaatctgaccggatgtaacggttgataagaaaattataacggcagtgaagattagcggcgaaagtaatttgttgcgaattttcctgccgttgttttatataaacaatcagaataacaacgacttagcaataggattttcgtcaaagttttccaggattttccttgtttccagagcggattggtaagacaattagcatttgaattttacgggtttagcgcgagtgggtaacgctcgtcacatcgtagacatgcatgcagtgctctggtagctgtaaagccaggggcggtagcgtgctgaaattataaagtcattcttatagaacatcgcatttcaataatataattacacctaaatgaataggatacaacgtgtgcacaattatttaaggcttaaagataaaataaaaaacgtatttttagggttgtatatattgcagttatttaattatatcgcgccattggtaattatccctatcctgataaaatatattgggttgggggaatatggggaattggtctatattacatctatttatcaaatagtggctttgattattgattttggctttacttacacaggacctgtggttgctgcgagacatagatgtgagacccaaaatttacagcgctattactcaatagttgttcttttaaaatcattgctttttataattgcattaacatgtgtatttttattgtgcagattaaatatagtccacttgtcattttttgggtttttgtcaatttttctatgcactattggtaatatattatcgcccaattggtttttgcaggggattggtgattttaaaaaactttcatactcacaagtaatagtgagaataacattgtttatcatacttcttgtttatgtctgtagtggcggagataatgtttttatcctaagttttttgcaaaatgcaacattactcatatgctgtatatacttatggccaaatattcatattagccatgttgttcatcttaaacctaatgaatgcattgtggaatttaagaaggcaggaaatgtttttattggcgtaataggtacgattggttacaatggtctaattcctgtgttaattggaaacctttgcggtaatacgagtcttggtgttttttcaatcgttcaaaaaatgacaacagcatgtcaaagtctaattaatccaatatcacagtatatgttatctcaagtttcagaaattaaacctcaagataaactgttttattatagaattaaaaaaagtttttttgtgcatttaacaattagcataattgcatgtttatgttatatggggttagggcaatatgtggcgacttttataggtaaagttgacgtttcatttgttattattttatttgcgtcaataattaccattttttcatctttaaataatgtccttggtatacagtttcttataccgacagataatgtaaaaatactacgaagtataaatgttatggcgggaattattgttgttagtttgtcctggctgttaatatcacgctttgacattctggggggggttttattaaacctaattggtgagtttcttgtattcagtatgctagcttttattgcccatcgaaagtggggagcgagagtataatgaaagtgaaggcggttcctgctattacattctatttaagtttaatgctgacaattttagtgttactgtttggtaatgaaccaaataaatcacaatatatccttgttatagcaacgataacagttttttatatcgcatatatcactaataaaataacttctccggccagccttctcgttatatcatcttttgtgtttttaggttgtcgccctttattatctttgtttgcaaactatgattataggattgccgattggtttattgaaggatatatggatgacgatgtgattttggctaactatgctataacactaatgtattatggttatacattgggactaattctatgcaaaaatactgaaaaattttatccgcatggtccttatcctgaaaaacaattgctaaaaataaagtttcttttgactttattttttctgggttcgataggtatggttgtaaaagggatattcttttttaactttatagaatctaatagttatgttgatatttatcaatcaaatataacaacgccaataggttatgattttctatcttatttattttattgttcttttttccttatatgtgcgtttcatatacagttcagaacaaataaaaaatttctttttattgcgatatgcattgctgcatttagcaccttgaagggtagtcgtagtgaagctataacgtttcttttaacggttacatgtatatattttaatgaagtaaagacaagaaacttacgtctgctgattacaatgatttttgtttttagcgtcatttttgtgattagtgaatttatctcaatgtggcgcactggagggagtttttttcaattaatgcagggtaataatcctgttataaactttgtatacggcatgggagtatcatatctttccatttatcaatcagtaaaactacaactattgtcagggggatataatgttacctatctattcagccagttaataataacttgctcgtcaatatttaatgtcaaattgagcttgccggaaataagctatagccatttggcctcatacacagcaaacccagaactatataatcttgggttcggacttggggggagttatttagcagaatcgtttttagcatttggtctgattggatgtttcattataccctttttacttttacttaatttaaatgtattggaaaaatatacaaaaaacaaaccaattatatattttgtttattatagtgtgttgccacctatattattcacaccaagagagactttgttctatttcttcccctatcttgtcaaaagtatatttgttgcttttttagttacattatacatccagtataaaaaggattgaccaaaatgtcagaaaaaaatgtcagcataataatcccaagttataacagggctcatattcttaaggaggtcataccaagttattttcaggatgagactttagaggttatagttatcaatgatggatcaacagataatacaaatagtgtattagctgaactgaaggaaaaatattctcagttagttattttagaaaatgaaacgaataaaaaacagatgtattctaaaaaccgagggattgaaatagccaaagggaaatatattttttttggtgatgatgactcttacctcttacccggtgttatatctcggttattggctacaaaatatgagacaggcgctgatgtaatcggcgcaagaatactttatatgaataataacgagaaaacaattgaagattgcataaatcgacataaaaaagaggggcgttttgttagtgatctaaatagattggattttagttatacatgtgatttggaccatccgattgaatgtttttatgcacagccttttgttctagctgaaagggaactaatatcgaaatatcgatttgatatatcttatacgggaaactgctatcgtgaggaaactgatttcatgctatctctatttattaaaaataaaaaatttatatatgattcaaaggctttgttaataaatttacctccaagaaaagcgacgggaggggcaagaacagctaatcgattaaaatatcattacgaaagttgcataaataattatagatttttaaaaaaatataatgataatttgaatcttctttcaggacaaaagcatgctatattttaccgacagtgtcaattcgttctgctaaaaatgaagtcgtttatcgggaagtttttaaaatgattatatatatcgccgcgtataatggttcaggagggcaaggtggggtggaaagggttgttgcccaacaatgtaacattcttaaaaatttgggggttaaagtcattatacttgataaaacatacttcaaaatttctaacaaaattcgtaacaaaaaaatacaagtagcactttatccaatattagtttctctttatttaaccttacaaaaattacgtggcgtgacgtttaaagttattgcacatggctattgttctcctttttataggaatgacatcttaatagctcatggcaatatgaaatgttattttcaaacagtcatgaataaaaaacctaatcggttgtctggcagtggtcttttatctttctatgagcgttgggctggagcattttcaaaaaatatctgggctgtttcaaataaggttaaaagtgaatggaatgagctttacaatattaattcacataaaatcaaagttgttcgaaattttataaatcttgcacaatttgattacactgatgttaatgaagcagaatatgtgacatttgtcgggcgattggaaaaaggaaaaggaatagatgatctgtattacatatgtaaaaatctgccagatacttccttccatttagtttcaagtattcccgccccacaaaattttgcttcgctaaataatgttctgaccagcattgctgtcccctatgcgaaaatgccagaaatatttaagaaatccagagtacttattttaccgtcctattatgaaggatatgagctggttactattgaagcgctatgctgtggttgccctgtgataggctataatgttggtgcaattagagagttgtatgcagaaagttttcctggcgtatttattgccaataataaagaagatttagcacaagtagcctacaaattaattagtcttgataatgaaaaatattatcatttgagacaaactatttatagcaagcgtgagcttttttctgaagagagatatgcggaaattttaacggcggcatttaatgaaaaaaaataagaaactctgtctcatttcaattaactcatataatgaacttaccggaggaggagtatatttacgtacgcttgttagttttctacaaaaacagaatgttaatttaacacttattgataaaaaatcctcaggtaaactattcgaagacaatacttttcaacatatatcatttattaaaggtaaacgtcaggatataatatccaggcttttttttataccatcattttatgtcccttatattttctcaataattaaaattttacggaagcaagatattcttgcttttcacaactctcggcttggattgttatgtctgctttttagaatactcatgccccacaaaaagatcatattgtttacggataacttcgaatatgacttaataagacaaaaagataaaaacataactacttttattgaaaaattaattgtttatctcaatgaatttatcgggcttaagaattcagatttagttagctatattacccggcaagataaaaatgcaatggataaattttatgggattaaaaaaagcagaaatttaattctccctgtgatatttagtagagaaaaaccaactgatgtattgtcagctcactttattaatgagtataatcgattgaataatgataataggaaaaaagtagtatttactgcatcttttgatttttttccaaatatagatgctgccaactatgttttaaatgcagcaaagtctaataatgattattgctatattttggcaggtaggaaaagtactactttgaatcttcctgatttggataatttattttttttcgataatctatctaatagtgaaatgtcatatttattatctgcttgtgatgttttttattctcctatagttttaggaagtggaatgaaaacaaaaattgcagaagcactatcatatggattatatatttatgcgacagagcattccttaatcggctatgatgaaattatacacaataaggagtgtgttaaaaaaatctcacatttggatgaggaatttcctaaagatttcaagatgaaaagtatcaataaacagctaataatgtcttatcagcaaaaatattattcacattatcggtttaatggccatgaacttgatataataaattttgacgattagttagtggagatataatatgaacatattagtaactggtggtgctggatatatcggatctcatacggctattgaattactgaatgcaggtcatgagattatcgttctggacaatttcagtaatgcttcatacaagtgtatcgaaaaaataaaagaaattactcgacgtgattttataacaattactggagatgctgggtgtaggaagacactctccgctattttcgagaaacacgccatagatatagttattcattttgctggctttaaatctgtttcagagtctaaaagtgaacccttaaagtattaccagaataatgttggagtgaccattactttattacaggtaatggaagagtacagaattaaaaaatttatctttagttcatctgcgacagtctatggtgaaccagagataattccaattccagaaacagctaaaattggaggaactacgaatccatatggcacatcgaagtattttgttgaaaaaattctagaggatgttagttccacgggaaaactggatataatttgcttgagatattttaatcctgtcggtgctcattctagtggtaaaataggtgaggctccatctggtatccctaataatcttgttccttatttattggatgttgcgagtggtaaacgtgataaattatttatttatggcaatgattaccctactaatgatggaacaggtgtaagggattttattcatgttgttgacttagcgaaaggtcatttggctgcaatgaattatttaagtatcaattcgggatataatatctttaatcttggtacaggaaaaggttattcggtacttgaattaatcactacatttgaaaaattaacaaacattaaggtcaataaatcttttatagagagaagggcaggggatgttgcgtcttgttgggctgatgcagataaagctaattctttattggactggcaagccgaacaaactctagaacagatgttattggactcgtggcgttggaaaaaaaattatccagacggattctgaatataaaaggtttcagttttatgaatcaatcagagcagagaaaaaaaatactggttcttacacctcgctttccctaccctgtcattggaggggatagattaagagtctatatgttatgtaaagaactttccaaaaaatatgatcttattcttctgagcttatgtgatcaaccactagaacttgaaataaatataaatgactcggtcttcaaagaaattcatcgtgtctatctaccaaaatataaatcatattataatgtattaaaagctttggttacgcaaaaaccgttgcaaattgcttattatcaatcggacacatttaagaataaatacaataaattaattaaacaatgcgatgcagtattttgtcatctgataagagttgctgattatgttaaggatacagacaagttcaaaattcttgatatgacagatgcaatatctttgaattacagtcgcgttaaaaaattagcaagtaaaaaaagtttgcgtgcaattatttattctctggaacaaaaaagattagaatcatatgaacgttctgtggcgaatctttttgatttgaccacttttatttcatccgtagaccgtgactatctctaccctaatctgggcagtaatatccatatagtcaataatggggttgatacatcagccttgagatatataaaaagagaaataaaaatcgataagcctgtggaacttatatttatcggaaatatgtattctttacaaaatatggatgctgcaaaacattttgctaagaatattttaccttgcttgtatgatgagtttaatattatttttaaagtgattggtaagatctcagaaactaataaaaatatattaaattcatttaaaaatacaattgctttaggtactgttgatgatatcaattcttccgcttctacagggcatataggtatatgtcctgttcgtcttggagcaggcgtacaaaataaaattcttgaatacatggctttaggtttaccatgtattacatctagcattggttatgaaggtattaatgcaaaatcaggtagcgaaatttttgttgcagatacagtagagcaatataaaaacgtactaagagaaataatttacgattataatcgttatactgaagtggctgaaaatgcccgtagttttgtagaaaataatttttcttgggaatcaaaagttgccaatttaatgaatacattagatgagaaattatatgaacaataataaaattattacacctatcattatggctggtggttcaggcagtcggttgtggccactatcaagaattctctatccgaaacaatttcttagcctaatcggtagtcataccatgcttcaaacaacggctaatcgtctggatggtttggattgtaccaacccttatgtcatttgtaatgaacaataccgctttatagttgctgaacagcttagaaaaatcgatagattgacttcaaagaatatcatccttgagcctgttgggcgtaacactgcccctgcaattgcattagcggcgttgctgatgtctaagtctgataaaagtgcagatgatcttatgctcgtactggctgcagatcacgttatacacgatgaagaaaaattttgtaacgctgttagatcggcaattccatacgctgctgatgggaaattggtaacatttggtataattccagacaaagcagaaactggttatggttatatacatcgaggacaatatattaatcaggaagattcggatgcatttatagtgtcatcatttgttgaaaagccaaatcatgagacagccactaaatatcttgcttccggtgagtattattggaatagcggtatgtttttgtttagtgcaaatcgttatatagaggaacttaaacaatttcggcctgatattttatccgcttgtgaaaaagcaattgcttcagcgaactttgaccttgattttgtgcgtttagatgaaagttctttctctaagtgccctgaagaatcaattgattacgctgtaatggaaaaaacaaaagacgcaattgttattccaatggatgctggctggagtgatgtcggttcatggtcttctctttgggaaattaatgataaagactcagacggcaacgtaatagttggggatattttctctcatgaaacaaagaattctttcatatatgccgaatcgggaattgttgctacagttggagtggaaaatttagttgttgtccaaacaaaggatgctgttcttgtctcagagagaaataaagttcaggatgtaaagaaaatagtagaacaaattaaaaattcaggtcgtagcgagcattatgttcatcgcgaagtatatcgtccttggggtaaatatgattccattgacacaggggagcgttatcaggtcaaacgtataacagtaaatcctggtgaaggactttctttacaaatgcaccatcatagggcagaacattggatcatagtttctggaactgcaagggtgactataggttctgaaactaagattcttagcgaaaatgaatctgtttacatacctcttggtgtaatacactgcttggaaaatccagggaaaattcctcttgatttaattgaagttcgttctggatcttatttagaagaagacgatgttatccgttttcaggaccgatatggtcgtagctaaatttttgataatgtaacgttagtagaagagcgctaatatttttagttaatctgtaataagtattatttgtttaaggtatatcatgtcgagtttaccctgctttaaagcctatgatattcgcgggaaattaggcgaagaactgaatgaagatattgcctggcgcattggtcgcgcttatggcgaatttctcaaaccgaaaaccattgtgttaggcggtgacgtccgactcaccagcgaaaccttaaaactggcgctggcgaaggggttacaggatgcgggcgtcgatgtgctggatattggcatgtccggcaccgaagagatctatttcgccacgttccatctcggcgtggatggcggcatcgaagttaccgccagccataacccgatggattacaacggcatgaaactggtgcgcgaaggggctcgcccgatcagcggtgataccggactgcgcgacatccagcgtctggcagaagccaacgactttcctcccgttgatgaaaccaaacgcggtcgctatcagcaaatcaatctgcgtgacgcttacgttgatcacctgttcggttatatcaacgtcaaaaacctcacgccgctcaagctggtgattaactccgggaacggcgcggcgggtccggtggtggacgccattgaagcccgctttaaagccctcggcgcacccgtggaattaatcaaagtgcacaacacgccggacggcaatttccccaacggtattcctaacccgctactgccggaatgtcgcgacgacacccgcaatgcggtcatcaaacacggcgcggatatgggcattgcctttgatggcgattttgaccgctgtttcctgtttgacgaaaaagggcagtttattgagggctactacattgtcggcctgctggcagaagcgttcctcgaaaaaaatcccggcgcgaagatcatccacgatccacgtctctcctggaacaccgttgatgtggtgactgccgcaggcggcaccccggtaatgtcgaaaaccggacacgcctttattaaagaacgtatgcgcaaggaagacgctatctacggtggcgaaatgagcgcccaccattacttccgtgatttcgcttactgcgacagcggcatgatcccgtggctgctggtcgccgaactggtgtgcctgaaaggaaaaacgctgggcgaactggtgcgcgaccggatggcagcgtttccggcaagcggtgagatcaacagcaaactggcacaccccgttgaggcgattaaccgcgtggaacagcactttagccgcgaggcgctggcggtggatcgcaccgatggcatcagcatgacctttgccgactggcgctttaacctgcgctcctctaacaccgaaccggtggtgcggttgaatgtggaatcgcgcggcgatgtaccgctgatggaagaaaagacaaaacttatccttgagttactgaacaagtaattcagtaatttcatataaatgggttttaaaaaacggaaaagatgagatatccggtgtggtatatccaaggtaatgctattcagtatctctatgagtgagttaacatctataccacatttaagccgcacacttcgggatccccatatgaatatcctccttagttcctattccgaagttcctattctttctagagaataggaacttcggaataggaactaaggaggatattcatatggataaagccgtaagcatataagcatggataagctatttatactttaataagtactttgtatacttatttgcgaacattccaggccgcgagcattcagcgcggtgatcacacctgacaggagtatgtaatgtccaagcaacagatcggcgtagtcggtatggcagtgatgggacgcaaccttgcgctcaacatcgaaagccgtggttataccgtctctattttcaaccgttcccgtgagaagacggaagaagtgattgccgaaaatccaggcaagaaactggttccttactatacggtgaaagagtttgtcgaatctctggaaacgcctcgtcgcatcctgttaatggtgaaagcaggtgcaggcacggatgctgctattgattccctcaaaccatatctcgataaaggagacatcatcattgatggtggtaacaccttcttccaggacactattcgtcgtaatcgtgagctttcagcagagggctttaacttcatcggtaccggtgtttctggcggtgaagagggggcgctgaaaggtccttctattatgcctggtggccagaaagaagcctatgaattggtagcaccgatcctgaccaaaatcgccgccgtagctgaagacggtgaaccatgcgttacctatattggtgccgatggcgcaggtcactatgtgaagatggttcacaacggtattgaatacggcgatatgcagctgattgctgaagcctattctctgcttaaaggtggcctgaacctcaccaacgaagaactggcgcagacctttaccgagtggaataacggtgaactgagcagttacctgatcgacatcaccaaagatatcttcaccaaaaaagatgaagacggtaactacctggttgatgtgatcctggatgaagcggctaacaaaggtaccggtaaatggaccagccagagcgcgctggatctcggcgaaccgctgtcgctgattaccgagtctgtgtttgcacgttatatctcttctctgaaagatcagcgtgttgccgcatctaaagttctctctggtccgcaagcacagccagcaggcgacaaggctgagttcatcgaaaaagttcgtcgtgcgctgtatctgggcaaaatcgtttcttacgcccagggcttctctcagctgcgtgctgcgtctgaagagtacaactgggatctgaactacggcgaaatcgcgaagattttccgtgctggctgcatcatccgtgcgcagttcctgcagaaaatcaccgatgcttatgccgaaaatccacagatcgctaacctgttgctggctccgtacttcaagcaaattgccgatgactaccagcaggcgctgcgtgatgtcgttgcttatgcagtacagaacggtattccggttccgaccttctccgcagcggttgcctattacgacagctaccgtgctgctgttctgcctgcgaacctgatccaggcacagcgtgactattttggtgcgcatacttataagcgtatcgataaagaaggtgtgttccataccgaatggctggattaa

SEQ ID NO: 14 - DNA, 15027 bp, Artificial Sequence
  example O8 rfb locus nucleotide sequence - O8-EPA production strain stLMTB11734
atgacgaatttaaaagcagttattcctgtagcgggtctcgggatgcatatgttgcctgccactaaggcgatacccaaagagatgctaccaatcgtcgacaagccaatgattcagtacattgttgacgagattgtggctgcagggatcaaagaaatcctcctggtaactcacgcgtccaagaacgcggtcgaaaaccacttcgacacctcttatgagttagaatcactccttgagcagcgcgtgaagcgtcaactgctggcggaagtacagtccatctgtccgccgggcgtgaccattatgaacgtgcgtcagggcgaacctttaggtttaggccactccattttgtgtgcgcgacctgccattggtgacaacccatttgtcgtggtactgccagacgttgtgatcgacgatgccagcgccgacccgctacgttacaaccttgctgccatgattgcacgtttcaacgaaacgggccgcagccaggtgctggcaaaacgtatgccgggtgacctctctgaatactccgtcatccagactaaagagccgctggaccgtgagggtaaagtcagccgcattgttgaatttatcgaaaaaccggatcagccgcagacgctggactcagacatcatggccgtaggtcgctatgtgctttctgccgatatttggccggaactggaacgtactcagcctggtgcatggggacgtattcagctgactgatgctattgccgagctggcgaaaaaacaatccgttgatgcaatgctgatgaccggcgacagttacgactgcggcaaaaaaatgggctatatgcaggcgtttgtgaagtatggcctacgcaacctgaaagaaggggcgaagttccgtaaaggtattgagaagctgttaagcgaataatgaaaatctgaccggatgtaacggttgataagaaaattataacggcagtgaaaattcgcagcaaaagtaatttgttgcgaatcttcctgccgttgttttatataaaccatcagaataacaacgagttagcagtagggttttattcaaagttttccaggattttccttgtttccagagcggattggtaagacaattagcgtttgaatttttcgggtttagcgcgagtgggtaacgctcgtcacatcataggcatgcatgcagtgctctggtagctgtaaagccaggggcggtagcgtgcattaatacctctattaatcaaactgagagccgcttatttcacagcatgctctgaagtaatatggaataaattaagctagcgatcgcttaagatctaggatttcattatgttacttcctgtaattatggctggtggtaccggcagtcgtctctggccgatgtcacgcgagctttatccgaaacagttcctccgcctgttcgggcagaactccatgctgcaggaaaccatcacccgactctcgggccttgaaatccatgaaccgatggtcatctgtaacgaagagcaccgcttcctggtggctgaacagctacgccagctcaataagctgtcgaataatattattcttgagccggtcgggcgcaacaccgccccggccatcgccctggcagcccttcaggccacccgcgacggcgacgacccgctgatgctggttctcgccgctgaccatatcatcaataaccagtcggccttccacgacgccatccgggtcgccgagcagtatgctgatgaaggtcatctggtcaccttcggtatcgtgccgaatgccccggaaactggctacggttacattcagcgcggcgtggcgctcaccgatagtgcccattccgcgtaccaggtggcccgctttgtggagaagccggatcgcgagcgcgccgaggcttacctcgcctccggggagtactactggaacagcggcatgtttatgttccgcgccaagaaatacctcatcgagctggccaaataccgtccggatatcctggaagcctgccaggctgcggtgaatgccgccgataatggcagcgatttcatcaatatcccgcatgatattttctgcgagtgcccggatgagtccgtggactatgccgttatggagaaaaccgccgatgcggtggtggtcggtctcgatgctgactggagcgacgtcggctcctggtccgcactatgggaggtcagcccgaaagacgagcagggcaatgtcctcagcggtgacgcgtgggtacacaacagcgaaaactgctacatcaacagcgacgagaagctagtggcggccattggcgtagagaatctggtgattgtcagcactaaggacgccgtgctggtgatgaatcgcgagcgttcccaggacgtgaagaaggcggtcgagttcctcaagcagaaccagcgcagcgagtacaagcgccaccgtgagatttaccgcccctggggccgttgcgacgtagtggtccagaccccgcgcttcaacgtcaaccgcatcacggtgaaaccaggcggtgccttctcgatgcagatgcaccaccatcgcgccgagcattgggttattctcgccggcaccggtcaggtgactgtcaacggtaagcagttcctgttgtccgagaaccagtccacctttattccgattggcgccgagcactgcctggaaaaccctggctgtattccgctggaagtgctggagatccagtcgggggcgtaccttggcgaggacgacattattcgtattaaagaccagtatggtcgttgctaattattttcgggacaagacgcagaatgacacagttaacttgttttaaagcttatgacatccgtggtgaactgggtgaggaactgaacgaggacatcgcctaccgtatcggtcgcgcctacggcgaatttctgaaacccgggaagatagtggtggggggcgatgtgcgcctcacaagcgagtcgctgaagctggcgctggcccgcgggttaatggacgccggtaccgacgtgctggacatcggcctgagcggtaccgaagagatttactttgccaccttccaccttggggtagatggtggcatcgaggtgaccgcgagccacaatcctatgaactacaacggcatgaagctggtgcgcgagaatgcgaagcccatcagcggcgacaccggcctgcgggatatccagcgcctggcggaggaaaaccagttcccgccagtggacccggcgcgtcgcgggaccctgagcaagatatcggtactgaaggagtatgttgaccatctgatgagctacgtggacttctcgaacttcacccgtccactgaagttggtggtgaactccggaaacggggctgcggggcacgtgattgatgaggtggagaaacgcttcgcggcggctggggtgccggtaacctttatcaaggtgcatcaccagccggatggccatttccctaacggtatcccgaatccgctgctgccggagtgccgccaggataccgccgacgcggtgcgcgagcatcaggccgacatggggattgcctttgacggcgacttcgatcgctgcttcctgttcgatgacgaagcttcgtttatcgaggggtattacattgtcggcctgctggctgaggcgttcctgcagaagcagccgggagcgaaaatcattcacgacccgcgcttgacgtggaacacggtagacatcgtgacccgcaacggcggccagccggtgatgtcgaagacggggcatgcgttcatcaaggagcggatgcgtcaggaagacgctatctacggcggggagatgagtgcgcaccattacttccgcgatttcgcctactgcgatagcgggatgatcccgtggctgctggtggcggagctgctgtgtctgaagaacagctcgctgaaatcgctggtggcggaccgccagaaggcgttccctgcgtcgggagagatcaaccgcaagctaagtaatgctgctgaggcgatcgcccgcatccgggcgcagtatgagccggcggctgcacacatcgacacaacggacgggatcagtattgaataccctgaatggcgctttaacctgcgcacgtctaacaccgagccggtggtgcgtctgaacgttgagtccagagctgatgtggcgcttatgaatgaaaaaacgaccgagctgttacacctgttaagcggggaataaggtgagagatttactaacgacgatttatcgttatcggggatttatctggagcagtgttaaacgtgattttcaggcacgctatcaaactagtatgctgggcgcactatggctcgttttacaaccgctctctatgattctggtctataccctggttttttccgaggtgatgaaggcaagaatgcccgataataccgggtcgtttgcctatagtatttatctctgttccggggtactgacctggggattatttactgagatgctggataaaggtcagagcgtatttattaacaatgctaatctgatcaagaaactcagttttccgaaaatctgtctgccgatcatcgtgacgttatcggcggtgctaaatttcgcgattattttcagtctgtttctaatttttatcattgtcaccggtaacttccccggctggctctttctctcggtgataccggtcctgcttttgcagatcctgtttgccggtgggctggggatgatccttggtgtcatgaacgtctttttcagggatgtggggcaactggttggcgttgcgctgcaattctggttttggttcacacccattgtttatgtactgaattcattacctgcatgggcaaaaaatctgatgatgtataacccgatgactcggatcatgcaatcttatcagtccatcttcgcctatcatctggcccccaactggtattcgctatggccagtattggctctcgccattattttctgcgtcatcggtttcaggatgttccgcaagcatgcggcggatatggtggatgaattataatgagttatatcagagtaaataatgtcggtaaggcgtatcgccagtatcactcaaagaccgggagactgatcgaatggttatcccctctgaataccaaacgccataatttgaaatggatcctccgcgatattaatttcgaagtcgctccgggcgaggctgtcggtattatcggtatcaacggtgcaggcaagagtaccctgcttaaactcataaccgggacgtccaggccgacgactggagaaattgaaatctccggacgtgtcgctgcattactcgaattggggatggggtttcattctgatttcactggtcggcagaatgtttatatgtctgggcaactgttggggttatcgtcagagaaaataactgaactgatgccgcaaattgaagagtttgctgagattggggactatatcgatcaacctgtgcgcgtctactccagtgggatgcaagttcgattagcttttagtgtagcgacggctatccgtcctgatgtgctaattatcgatgaggcattatctgttggggatgcatatttccagcataaaagctttgagcgtattcgaaaatttcgtcaggaagggaccacgctgttgctggtatcccatgataaacaagcgatccaaagcatttgcgaccgggccattttattgaataaaggccaaattgaaatggaaggtgaacctgaagcagtgatggattattacaatgctcttctggccgataaacaaaatcagtccattaaacaagttgagcataatggtaaaacgcaaactgtttcaggcactggtgaggtgactatctctgaggttcatcttctcgatgaacagggcaatgtgactgaatttgtttcggtagggcatcgtgtcagcttgcaggtcaacgttgaggtcaaggacgatattcctgagcttgttgtcggatatatgattaaggatcgacttgggcagccgattttcgggaccaatacgtaccatctcaatcagacactcacctccctgaaaaaaggagaaaagcgttcgttcttattttctttcgatgcgagattgggggttggctcctattctgtcgctgtcgcgttgcatacttccagtacgcacctcggcaaaaactatgaatggcgcgatctggccgtggtattcaacgtcgttaacacggaacaacaagagtttgtcggcgtgtcctggttgccgcctgaactggagatttcttaatgggttcgtcgttttatcgttcatttgaagaacgacacagaggttcggttgaagaaatcaagcgccgcttgagtttttatttaccttttcttgcaggtctgaaggacatttatcctgatggcgtgattgcggatattggttgcggacgtggcgaatggttggagatcctgactgaaaatggcattgcgaacatcggcgtcgatctcgatgatggcatgctggcgcgcgccagggaggccggactgaatgtgcagaaaatggattgtctgcagtttttgcaaagtcaggcggatcagagcctgatagcgttgaccggttttcatattgctgagcatttgccgtttgaggtcctgcagcaactcgccatgcataccctacgggtgctgaaaccaggtggtttgctgatcctcgaaacgccgaacccggagaatgtaagcgtcggcacctgttcattttatatggatccaacgcataatcatcctctgccaccgccactgcttgagtttttacctattcattatggttttacccgagcaattaccgttcgtctgcaggaaaaagaggttcttcaatctccggatgcagccgttaatttggtcgatgtactcaaaggggtgagccccgactacagcatcattgctcagaaagcagcgccaacagatattcttgaacgctttgacaccctgtttacccagcagtacggtctgacgctggatgctctgagcaaccgttacgatgcgattttgcgccaacagttttcgtccgttgtctcacggctggagacgttgaaccaaacctatatgcaacagataagccaaatgtcagagactattcagacgttgcaaggtgaggttgacgatctgagtcatgtcatcgatcagaaccatcagcttcatcagcaaatggcggatttacataacagtcgttcatggcgtattactcaaccactacgctggttgtctttgcaacgtcaattattacgtcaggaaggggctaaagtgcgagcccgtagggctgggaaaaaaatattgcgcaaagggatggcgctctcgctggtctttttccatcgttaccctaagtctaaggtttatctgtttaaggttctgagaaaaactggctgctatacattgctacaacgtttgttccaacgcgtaatgctggtgcaatctgacacgatgatgatgcagtccagaagatatgatgtgggtactgaagaaatgacaagtcgcgcgatgagtatttataacgaattaaaaaataaaaatacggagaaataacgatgcgtattgtcatagatttacaaggcgcacagacggaaagccgctttcgtggcatcggtcgttatagtatcgcaatcgccagaggcataatcagaaataacagccggcatgagattttcatcgcgctatccgccatgctggatgagtcgattgcaaatattaaggcgcaatttgccgatctcctgccggcagaaaatatagtcgtatggcatgccgtaggccctgttcgtgcgatggaccaaggtaatgaatggcgtcgggagagcgcagaactgattcgggaagcgtttcttgaatcattgtgtccagatgtcgttttcattacgagtttgtttgaaggtcatgtcgacgatgcggctacatcggtacacaaatttagtcgtcagtataaagtagccgtactgcaccacgatcttatccccctcgtgcaggcggaaacctatctgcaggacgatgtatacaaaccctactatttacagaaagttgagtggttaaaaaacgctgaccttttgttgactaactctgcttataccgcacaggaagcgatcgagcatctgcatttacagggcgatcatgtgcagaatattgcagccgcagtcgattctcagttttgtatggcggaggtggcagcgagcgaaaaagagaccgtccttggccattacggtattcagcgcgagttcatgttgtatgcgcccggaggatttgactcaaggaaaaactttaaacggttgattgaggcctatgccgggctcagtgatgccttacgtcgcagtcatcaactggtcatcgtcagtaagctttccatcggtgatcgtcagtatctggaatcccttgcgtcaggtaatggtttacagcagggcgaactggtactcactggttatgtgccggaagatgagctgatccagctctatcgcctatgtaagctgttcatctttgcttcactacatgaaggttttgggttgccggttctggaagcaatgtcgtgcggtgcgccggtgattggctcaaatgtcaccagtattcctgaagtcatcggtaatcctgaggcattattcgacccgtattctgtctcttccatgagggataagatcgcgcaatgtttgactgatgataccttcctcgcgcgtctgaaagaaatggcgcagcagcaagcgcgtaatttctcttgggataaagctgcggtgactgctctggaagctttcgaaaagatcgcggtagaagacaccggtactgcgcaggttttgcctgaagctttgattcagaagatccttgctatctcacaagggcagccagatgaccgcgatctgcgcttgtgcgcaacggccattgattacaatctgaaaacggcagaactttatcaaatcgacgataaatcgctgaactggcgtgtggaaggcccattcgatagctcatatagtctggcgttggtcaaccgcgaatttgcccgggcactctcagccgatggtgtagaggttttattgcattccactgaaggaccaggtgattttgccccagatgcctcgtttatggcacagtcggaaaatagtgatcttctggcattttataatcaatgtcagacccgcaagagtaacgaaaagatagatattattagcagaaatatctatccaccgcgggttaccaaaatggatgccaaagtaaaattccttcattgttatgcttgggaagaaacgggctttccgcaaccgtggatcaatgaatttaatcgggaacttgacggagtgctgtgtacttcggaacatgttcgtaaaatactgattgataacggactgaatgtgcccgcatttgttgttggcaatggctgtgaccattggctcaatatcccagccgagacgacaaaagatgtggatcacggaacattccgtttcctgcacgtctcttcttgtttcccacgcaaagggatacaggcaatgcttcaggcttgggggaaggcgttcactcgtcgtgacaatgttatcttaatcattaagacttttaacaatccgcacaatgaaattgacgcatggctggctcaggcccaggctcaattcatagactatcccaaagttgaagtgatcaaagaggatatgtcagccaccgagcttaaagggctttatgaaagctgtgatgttttggttgctccaggttgcgctgaaggctttggtttacctattgctgaagcaatgctgagtgggctaccggctatcgtcaccaattggagcgggcaacttgattttgttaattcacaaaattcatggctggttgactatcagttcactcgggtaaaaacgcactttggtctgttttcctcagcctgggccagtgtggatattgacaacttaacagatgcattaaaagcggcagcctcaaccgataaatcagtgctgcgtgacatggccaatgctggtcgcgagcttcttctgcagcagtttacctggaaagcggtggctgatcgttcttgccaggcggtcaagactctgcgtgcgcatattgatattgcacagcatcgggcgcgcattggctgggtgacgacctggaacacgaaatgtgggatcgcaacctattcccagcatctggtggaaagcgcacctcatggcgcggatgttgtttttgctccccaggtcagcgctggcgatcttgtgtgtgcagacgaagagtttgtacttcgcaactggattgtaggtaaagagagcaactatctggaaaacctccagccacacattgatgctctgagactcgatgtcattgtgatccaattcaactatggattctttaatcatcgagaactgtcggcgtttattcgtcgccagcatgacgccggtcgttcagttgttatgacgatgcactcaactgtggatccgctggaaaaagagccgagctggaatttccgtcttgctgaaatgaaagaggcgctggcactttgcgaccggttgttggtgcattcgattgccgatatgaaccgccttaaagatttaggcttaactgcgaatgttgctttattcccgcacggtgttatcaactactccgcagcgagcgtcacacgtcaacagcagtctttaccgctaattgcgagctatggcttctgcttaccgcataagggcctgatggaactagtagaatccgtccatagactcaagcaagccggtaaaccggttcgtttacgactggtgaacgcagagtatcctgttggggagtcacgcgatctggtggcagagcttaaagctgctgctcagcggttaggtgttaccgatctgattgagatgcataatgatttcctacctgatgcggagagtctgcggttgctttcagaagccgatcttctgatttttgcttatcagaatactggggagtctgctagcggggcggtacgttatggtatggcgactcaaaaacctgttgcggtaacgcccctggcgatatttgatgatttggacgatgccgtctttaaatttgatggatgcagcgtcgatgatatcagtcaggggattgaccggatcctgaattccatccgtgaacagaactcttgggcaaccaggactcaacaacgtgccgatgcatggcgggaacaacatgattatcaagctgtttcacgccgtctggttaatatgtgtcaaggcttagctaaagctaaatattttaaataaaaatatctctcttgtattttttgcctttgaatacaagaggggttagataatgtgtcatttattatgaaaattatttttgctactgagccaattaaatacccattaacgggcatcggtcggtattccctggagctggttaagcggctggcggtcgcccgcgaaattgaagaattaaagctatttcacggtgcgtcgtttatagaacagatccctttggtggagaataaaagcgataccaaagccagcaatcatggtcgtctgtcggcgtttctacgccgacagacgctgttgattgaggcttatcgcttgctgcatccgcggcgccaggcgtgggcattgcgcgactataaggattatatctaccatggccccaatttttatctgccgcataaactggaacgcgccgtgaccacgtttcatgacatatccatttttacctgcccggaatatcatccaaaagatcgggttcgctatatggagaagtccctgcatgagagtctggattcggcaaagctgatcctgaccgtttctgatttctcgcgcagtgaaattatccgcttgttcaactatccggcggagcggatcgtaaccaccaagctagcctgcagcagtgactatatcccacgcagcccggcagagtgtctgccggtactgcagaaatatcagctggcgtggcaggcctacgcgctatatatcggcactatggagccacgtaaaaatatccgaggcctgctgcatgcctatcagctgctaccgatggagatccgcatgcgctatccgctaatccttagcggctatcgcggctgggaagacgatgtgctgtggcagttagtcgagcgcggtactcgggaaggctggatccgttacctcggatatgttccggatgaagacctgccgtatctgtacgcagcggccagagtctttgtttatccctccttctacgagggattcggtttacctattcttgaagcgatgtcttgcggtgtgccggtagtatgctccaatgtcacctctttgcctgaggttgttggcgatgccggcctcgttgccgatcctaatgatatagacgcgattagcgcgcaaattttgcagagcctgcaagatgatagctggcgggaaatcgccaccgcgcgcggtcttgctcaggcgaaacagttttcgtgggagaactgtgcgacacagaccattaacgcctataaattactctaagggtgtcagttgagagttctacacgtctataagacttactatcccgatacctacggcggtattgagcaggtcatttatcagctaagtcagggctgcgcccgccggggaatcgcagccgatgttttcacttttagcccggacaaagatacaggtcctgtcgcttacgaagatcatcgggtcatttataataaacagctttttgaaattgcctccacgccgttttcgctgaaagcgttaaagcgttttaagctgattaaagatgactacgatatcatcaactaccattttccgtttccctttatggatatgctgcatctttcggcgcggcctgacgccaggactgtggtgacctatcactctgatatagtgaaacaaaaacggttaatgaagctgtaccagccgctgcaggagcgatttctcagcggcgtagattgcatcgttgcctcgtcgcccaattacgtggcttccagccagaccctgaaaaaatatctggataaaacggtggtgatcccgtttggtctggagcagcaggacgtgcagcacgatccgcagagggtcgcgcactggcgggaaactgtcggcgataagttctttctcttcgtcggcactttccgctactacaaagggctgcatattctgatggatgccgctgagcgtagccgactgccagtggtggttgtagggggcgggccgctggaatcggaagtgcggcgtgaagcgcagcagcgcgggctgagcaatgtgatgtttaccggcatgctcaacgacgaagataagtacattctcttccagctctgccggggcgtggtattcccctcgcatctgcgctctgaggcgtttggcattacgttattggaaggcgcacgctttgcaaggccgctgatctcttgcgagatcggtacaggtacctctttcattaaccaggacaaagtgagtggttgcgtgattccgccgaatgatagccaggcgctggtggaggcgatgaatgagctctggaataacgaggaaacctccaaccgctatggcgaaaactcgcgtcgtcgttttgaagagatgtttactgccgaccatatgattgacgcctatgtcaatctctacactacattgctggaaagcaaatcctgagcggccgcgagctcgtcgactcgaggatccgtgtaggctggagctgcttcgaagttcctatactttctagagaataggaacttcggaataggaactaaggaggatattcatatggataaagccgtaagcatataagcatggataagctatttatactttaataagtactttgtatacttatttgcgaacattccaggccgcgagcattcagcgcggtgatcacacctgacaggagtatgtaatgtccaagcaacagatcggcgtagtcggtatggcagtgatgggacgcaaccttgcgctcaacatcgaaagccgtggttataccgtctctattttcaaccgttcccgtgagaagacggaagaagtgattgccgaaaatccaggcaagaaactggttccttactatacggtgaaagagtttgtcgaatctctggaaacgcctcgtcgcatcctgttaatggtgaaagcaggtgcaggcacggatgctgctattgattccctcaaaccatatctcgataaaggagacatcatcattgatggtggtaacaccttcttccaggacactattcgtcgtaatcgtgagctttcagcagagggctttaacttcatcggtaccggtgtttctggcggtgaagagggggcgctgaaaggtccttctattatgcctggtggccagaaagaagcctatgaattggtagcaccgatcctgaccaaaatcgccgccgtagctgaagacggtgaaccatgcgttacctatattggtgccgatggcgcaggtcactatgtgaagatggttcacaacggtattgaatacggcgatatgcagctgattgctgaagcctattctctgcttaaaggtggcctgaacctcaccaacgaagaactggcgcagacctttaccgagtggaataacggtgaactgagcagttacctgatcgacatcaccaaagatatcttcaccaaaaaagatgaagacggtaactacctggttgatgtgatcctggatgaagcggctaacaaaggtaccggtaaatggaccagccagagcgcgctggatctcggcgaaccgctgtcgctgattaccgagtctgtgtttgcacgttatatctcttctctgaaagatcagcgtgttgccgcatctaaagttctctctggtccgcaagcacagccagcaggcgacaaggctgagttcatcgaaaaagttcgtcgtgcgctgtatctgggcaaaatcgtttcttacgcccagggcttctctcagctgcgtgctgcgtctgaagagtacaactgggatctgaactacggcgaaatcgcgaagattttccgtgctggctgcatcatccgtgcgcagttcctgcagaaaatcaccgatgcttatgccgaaaatccacagatcgctaacctgttgctggctccgtacttcaagcaaattgccgatgactaccagcaggcgctgcgtgatgtcgttgcttatgcagtacagaacggtattccggttccgaccttctccgcagcggttgcctattacgacagctaccgtgctgctgttctgcctgcgaacctgatccaggcacagcgtgactattttggtgcgcatacttataagcgtattgataaagaaggtgtgttccataccgaatggctggattaa

SEQ ID NO: 15 - DNA, 11283 bp, Artificial Sequence
  example O15 rfb locus nucleotide sequence - O15-EPA production strain stLMTB11738
atgacgaatttaaaagcagttattcctgtagcgggtctcgggatgcatatgttgcctgccactaaggcgatacccaaagagatgctaccaatcgtcgacaagccaatgattcagtacattgttgacgagattgtggctgcagggatcaaagaaatcctcctggtaactcacgcgtccaagaacgcggtcgaaaaccacttcgacacctcttatgagttagaatcactccttgagcagcgcgtgaagcgtcaactgctggcggaagtacagtccatctgtccgccgggcgtgaccattatgaacgtgcgtcagggcgaacctttaggtttaggccactccattttgtgtgcgcgacctgccattggtgacaacccatttgtcgtggtactgccagacgttgtgatcgacgatgccagcgccgacccgctacgttacaaccttgctgccatgattgcacgtttcaacgaaacgggccgcagccaggtgctggcaaaacgtatgccgggtgacctctctgaatactccgtcatccagactaaagagccgctggaccgtgagggtaaagtcagccgcattgttgaatttatcgaaaaaccggatcagccgcagacgctggactcagacatcatggccgtaggtcgctatgtgctttctgccgatatttggccggaactggaacgtactcagcctggtgcatggggacgtattcagctgactgatgctattgccgagctggcgaaaaaacaatccgttgatgcaatgctgatgaccggcgacagttacgactgcggcaaaaaaatgggctatatgcaggcgtttgtgaagtatggcctacgcaacctgaaagaaggggcgaagttccgtaaaggtattgagaagctgttaagcgaataatgaaaatctgaccggatgtaacggttgataagaaaattataacggcagtgaaaattcgcagcaaaagtaatttgttgcgaatcttcctgccgttgttttatataaaccatcagaataacaacgagttagcagtagggttttattcaaagttttccaggattttccttgtttccagagcggattggtaagacaattagcgtttgaatttttcgggtttagcgcgagtgggtaacgctcgtcacatcataggcatgcatgcagtgctctggtagctgtaaagccaggggcggtagcgtgcattaatacctctattaatcaaactgagagccgcttatttcacagcatgctctgaagtaatatggaataaattaagctagcatgagcaaaactaaactaaatgttctttaccttgcaataagtcagggtgccaattacctactgccattattaatttttccttatcttgttagagtcattggtgtatcgaattttggtgatctgagtttttcattgataactatacaagtgttgttaatggttgttgaatatggttttggatatagtgggacaagagaaatagcactaaataacgataaaaaataccattctgaatttttttgcggtgtggtgcttgctcgttttatattaatgctaattgcagctataatactcataatactctgttttttttatgtttttaacgacgttaagtctttgttatgtgttggttttctgtccgtaattgcaggtgttttcaatccaaattggtttttgcaaggtaaggaaatgatgagtgtgatggctgtgctgtcactattttcacgaggcatagcagtcgttgcagtttatctaattataaaacccgcaacgccgatgtacatcagtgccttattattgagcatgccatatattttgtattcattctgtggcgttgcctacttacttattatcaaggagatttttttatgtaggccaccgataaagaaaattcaagtaattttaaaaaatggatttcattttttttgttcaacacttgcgactagtgcatacacaatgttgacccctcttgtattgggtggcgtatctggaaagtttgatgtaggcatctttaactcagctaacatgatcaaacaaggtttggctggacttgcatcaccattagtccaagctttttatccaagaattaacattttgcaaagagagaatccatatattgcaaacttaaaatctagaatgattcttaaatacttgcttgttttttacatggctttagcaataccatttttactttttgccaaccaattatcattattaatattcggcatgaaaggtgaagtaattgcaggtgcaatgcaattaatgacattgcttcctatattcataggttttaatacagttgtcgggttacttgtattagtacctaatgggatgcaaaaacagtatttcaaatctattttcctaggaactattacttgtttaagcatagtttatccagcatgtaaatattatggagcaacgggtgcgattgtgagtcttattgtagctgaaattttcgttggcatgggaatgcttaaacaattcattaaagtaaataaaaccgtatgtaggcctcataaattatgaatatctcggtaataatatctgtttggaaacgcccagttcaattagaattgattctctctgagctcgattctcaggctaaagacaatagtctacacctagaagtaattgtttccgatagtcatagtggtaaagaaattgatgatgtagttgctgataatattcataaaaagaaaaatattaatattatccatcaacatactaaaaatatactctccgctaagcgcaatttcggagcatccctagcccatggggattatttaatatttcttgatgatgattgtatacccgcaagtggatatatatcatcgttgctgaactatttaaaaaaaatgaatagtaaaagcgttttatgtggggaagttagattcgaaaatgaactcattgagaccagcaattactatcgctacaggaactctttacaccctaagtttagtgatagtcctgatatctctatgaatgcctggacttttgtcgcaatgaattgtgttcttgatagaaaggcattttcatcaggtatagtttcatataatgaaaattttattggttatggttgtgaagatcatgagtttgggtggcaacttgaaaaaaatgacttcaaaattatttttgctgattttaaaatattacatcacgaatacagtggcgatatagaaggatatacaaaaaaaattcgtgctacagcacgtgatggtatgaatgtattaagcaaagtaaggcctgaaatgttttctactaataaaaaattattcctagttgagaaaatatttagtaaacacaaaacgtttagtaaaatatgccaatcaatatttttcaataaatttatttttaaaaaaataatacaatttttaaaaaaaacagatgcaaataaaaaactctatttcccaattctttacagatatgtgttgatttcggcatatatacatggtattggagagcgtggcacctcaaaaacagatgatttgcttaagaactggtatatatagatgatgctatcttcatttattaagacatttgtatggaaggtaaaaaacaatgaagtataatgcattgatggcttttttattattttttgttgttttttttagattgtcgctgataatacctttcttatatttggcatttattcctgcattttttggtattatgtatttagtgcgtaattttatgattactatgggcaatggattggtatctatagatcgtaaaaatttgttgctgttatctatattcataattatttttttattttgtttggttttcgatttgtttcaaaaaagccattcttttcaaagttattttaccgttagattatttatgttgtttttattttcatttgttcctgcgtattatttagtaaatagattcataaagggtgacttgaaattaatggagcgaatattagtgtattctctctgggttcaaatagttattttttttggtatgtatataagtccagagttaaaaagattgttatatactttctttggtatgtctgactctgttaatctttgggaacaaaatgctaaagtaagaggatttgggttgtcgggtgaaataaatttcatgacaccatttttgatgatctatatgtcattttttatgatgaaaaggcgttatgctttaattactttaatttgtctgactcaaatcgtaaattctaacatggctgtgattgcagccattattggtatcggttgctctagacttaatattaatataaaaattgcaacagtattgattttgggagttttagtttatagcttaggagcggtgttctttcctcgattttatgatgagttcgtttctggagatggcacaagaactctggatatcttattacagcaacatgtgtttgttgtaggtaatttagatttttttaatattatatttggattacagcaaaacatatcttcatcaatccccgatattaaacaaagttcggatatgggctgggttatactgtttaattacggtgggttaacatttattacactctttttatttttaatctttactatttctattgcgacatttggaatgacatatcaagcaattatatggatgttaattgggataattttcaataccaaaggtttagttttaggatctaacggctatttctttctatcttttatatatatgtttttgaatagagtaacacttagtggacagagttcaattactaataagttaggtcaagtaagtaaatagcttccagagtatatttgtcaatgatttgaggttcggttattatgttttcatctaaaacactgttaattactggtggtactggctctttcgggaatgctgtattaaatagatttcttgatacagatattgcagaaatccgtatatttagtcgtgatgaaaaaaaacaagatgatatgcggaaaaaatacaataatcaaaaattaaagttctatattggtgatgtcagagattaccgtagtattttgaatgcgactcgcggtgttgattttatatatcatgcagcggcacttaagcaagttccatcatgtgaatttcatcctatggaagccgttaaaactaatatccttggtacggaaaatgttcttgaagcagctatagcgaatgaagtgaagagggttgtatgcctaagtactgataaagctgtatacccgattaacgcaatgggtatttcaaaagctatgatggaaaaggtcatggtcgcgaaatcccgtaatgttgatcgcaataaaacagtaatatgtggtacccgttatgggaatgttatggcatctcgcggttcagttattccattatttgttgatcttattagagcgggcaagccactcacaataactgatcctaatatgacccgctttatgatgactcttgaggatgcggtagatttagttctttatgcgtttgaacatggtaataatggtgatatctttgtgcaaaaagcacctgcagcaactattgacacattagctattgctttaaaggaattactaaatgttcctgaccatccggtaaatgtcattggaacgcgtcatggcgagaaattatatgaagctctacttagtcgtgaggaaatgatcgctgctatagatatgggcgattattaccgtgtcccgccagatcttcgtgaccttaattatggcaaatatgttgagcaaggtgatagccgaatatctgaaatagaagattataactctcataatactcaacggttagatgttgaaggcatgaaagagctcttgctaaaattagcctttattcgagcaattcgtgctggtgaaaaatataatctggattcatgatatgaaaatattagttactggtgcaaatggttttattggtcgtaatttatgtttgaggcttgaggaacttggttataaagatcttattagaattgatcgagaatcaacgaagcaagatcttgaacaaggcttacaggatgccgattttatttatcacttagctggtatcaatagacctaagactgatgatgagtttatttctggaaacagtgatttaacaaagcatatagttgagtatctcctttctattggtaagaatacaccaattatgctaagttcttcgatacaagctgaacttaataatgcttatggggttagcaaagctgtagctgaaagctatgtcgaaaaatatgctgctgctagtggttcttcgtattatattttcagatatccaaacgtttttggtaaatggtgtaagccaaactataattcttttatagcaactttttgctacaatatttccaatgatattgagattactatcaatgatgcagcagcgccagtcaatctggtctatattgatgatgtttgtactgatgctatagctcttctctctgggacggttgaaagtggatataaagttgttgcaccaatttattcaacaacagttggtgaagttgcagaattaatttatagcttcaaaaatagccgttccaccctgatcacagaggctgtcggggcgggatttacccgtgcattgtattctacatggctgagttatttaccagcagagaagtttgcgtacaaggtacctttttatggggatgcccgcggagtcttttgtgagatgttgaaaacgccttcagcggggcagttttcattttttactgctcaccctggtattacgcgtggcggacattaccatcacagtaaaaatgagaagtttttggtcattcgaggtcaggcatgctttaaatttgaacatgtgattaccggtgagcgatatgaactgaaagtttcatcgggtgagtttaagattgttgaaacagttcctggttggacacatgacattacaaatattggaactgatgaattaatagtcatgctctgggcaaatgaaattttcaaccgtgatgagcccgatactattgcgagacctctataatgaaaaaattaaaagttatgtctgttgttggaacccgtcctgagattatccgtttgtcgagggttcttgctaagtttgatgaatactgcgagcatattattgtccatactggtcaaaattatgattacgaattaaatgaagtgttcttcaatgacttgggtgttcgaaaacctgattattttttaaatgcagcgggtaaaaatgcggcggaaaccattggtcaggttattattaaggtagatgaagtattagaaatcgaaaaacctgaagcaatactggtattgggcgatacgaattcatgtatttctgccattccggccaaacgccgtaaagtgcctatatttcatatggaagcaggtaaccgttgtttcgatcaacgcgtgcctgaagaaaccaacagacgtattgttgaccatacggctgatatcaatatgacctacagtgatattgctcgtgaatatctcttggctgaaggtatcccagctgatcggatcataaaaactggtagccctatgtttgaggttctttcatattatatgccccaaattgatggttcagatgtgctatcgcgtttgaatctacagtctggtgagttttttgtagtaagtgcgcatcgtgaagagaatgttgattctccaaaacagctcgtaaagcttgcgaacattctaaatactgttgctgaaaaatataatcttccagttattgtctccacacacccaaggacacgtaaccgaatccgtgagcaaggaattgaatttcattcaaatataaatctactgaaaccattgggtttccatgattataaccacttgcagaagaactcacgagctgtgctttcagatagcggtactatcactgaagagtcatccatcatgaatttcccagcggtaaacatccgggaagcgcatgagcgtccggaaggctttgaggaagcatccgtcatgatggtggggttagagtgtgaacgcgtattacaagcgctggatattctggcaacacaaccgcgaggtgaagtccgtcttttacgtcaggttagtgattacagcatgccaaatgtgtcggataaagttgtcagaattgttcactcttacacagattatgttaagagagtcgtctggaaagaatattgatgaaacttgctttaatcatagatgattacctgcccaacagtactcgtgttggtgcaaaaatgtttcatgaacttgctcaagaatttatccagcgtgggcacgatgttacggtaattactcctggtacgggcatgcaagaagagatttcttttgatacctttcagggggtaaaaacatggcgttttaaaagcgggccgctcaaggatgtaagtaaaattcagcgagcggtcaatgaaacgcttttgtcctatcgggcgtggaaagccatcaaaaaatgggtaaaaaaagagacctttgagggggtgatttattattcaccttccatattctgggggcctttagttaaaaaaattaaagctcgttgccaatgtcctgcttatcttattttaagagatatgtttccacaatgggtaattgatgcaggaatgcttaatgctggttccccaatagaacgctactttcgtctttttgaaaaaatatcttatcgtcaggcaaatcgtattggacttatgtctgataagaatcttgatgtttttcggaaagataataaaggctatccgtgcgaagttttgcgtaattgggcatccctaacaccaacgatcatacccaaggattatataccactacgtaagcgacttggcctagaggataaaaccattttcttctatggtggaaacataggtcatgcacaggacatgacaaacttgatgcgacttgtgagaaacatggcagcatatcctcaagctcatttcctatttattggccagggggatgaagttgaattaattaattcattagcatctgagtgggcattgacgaatttcacctatttgccctcggttaaccaagatgaatttaagttcattttgtcggaaatggatatcggcttgttttctctttccgctagacactcttcccataattttcctggtaagttattaggctatatggttcagtcgctacctattttaggtagcgtaaatgccggaaatgatttgctcgacattgtcaatcaaaataatgcgggattaatccatgtcaatggtgaggacgataaattatgtcaatctgcgctattaatgttgcatgatattgatgtgcgccggcaacttggttcgggggcgaatatattgttgaaagaacaattctccgttgagtctgcggcacagacgatagaaatgaggttggaggcatgcaatgcgattaattgataatgaccaactcgacgaattatatgatcaagccgggcaatcggaacgtttacgttcccaccttatgatgcacggctcgcatcaagaaaaggtacagcgtttacttattgcattagtaaagggcagctatgttgaaccgcattatcacgaacttcctcatcagtgggaaatgttcattgttatggaggggcaacttcaggtttgtttgtatggtagaaatggtgaggttataaagcaatttatagcaggagataatactggaatgagcattgtggagttttctccgggcgatatacacagtgtcgaatgcctatctccgcgtgctcttatggtggaagttaaggaggggccatttgacccttcttttgcaaaatcgttcgtgtgagcggccgcgagctcgtcgactcgaggatccgtgtaggctggagctgcttcgaagttcctatactttctagagaataggaacttcggaataggaactaaggaggatattcatatggataaagccgtaagcatataagcatggataagctatttatactttaataagtactttgtatacttatttgcgaacattccaggccgcgagcattcagcgcggtgatcacacctgacaggagtatgtaatgtccaagcaacagatcggcgtagtcggtatggcagtgatgggacgcaaccttgcgctcaacatcgaaagccgtggttataccgtctctattttcaaccgttcccgtgagaagacggaagaagtgattgccgaaaatccaggcaagaaactggttccttactatacggtgaaagagtttgtcgaatctctggaaacgcctcgtcgcatcctgttaatggtgaaagcaggtgcaggcacggatgctgctattgattccctcaaaccatatctcgataaaggagacatcatcattgatggtggtaacaccttcttccaggacactattcgtcgtaatcgtgagctttcagcagagggctttaacttcatcggtaccggtgtttctggcggtgaagagggggcgctgaaaggtccttctattatgcctggtggccagaaagaagcctatgaattggtagcaccgatcctgaccaaaatcgccgccgtagctgaagacggtgaaccatgcgttacctatattggtgccgatggcgcaggtcactatgtgaagatggttcacaacggtattgaatacggcgatatgcagctgattgctgaagcctattctctgcttaaaggtggcctgaacctcaccaacgaagaactggcgcagacctttaccgagtggaataacggtgaactgagcagttacctgatcgacatcaccaaagatatcttcaccaaaaaagatgaagacggtaactacctggttgatgtgatcctggatgaagcggctaacaaaggtaccggtaaatggaccagccagagcgcgctggatctcggcgaaccgctgtcgctgattaccgagtctgtgtttgcacgttatatctcttctctgaaagatcagcgtgttgccgcatctaaagttctctctggtccgcaagcacagccagcaggcgacaaggctgagttcatcgaaaaagttcgtcgtgcgctgtatctgggcaaaatcgtttcttacgcccagggcttctctcagctgcgtgctgcgtctgaagagtacaactgggatctgaactacggcgaaatcgcgaagattttccgtgctggctgcatcatccgtgcgcagttcctgcagaaaatcaccgatgcttatgccgaaaatccacagatcgctaacctgttgctggctccgtacttcaagcaaattgccgatgactaccagcaggcgctgcgtgatgtcgttgcttatgcagtacagaacggtattccggttccgaccttctccgcagcggttgcctattacgacagctaccgtgctgctgttctgcctgcgaacctgatccaggcacagcgtgactattttggtgcgcatacttataagcgtattgataaagaaggtgtgttccataccgaatggctggattaa

SEQ ID NO: 16 - DNA, 13435 bp, Artificial Sequence
  example O16 rfb locus nucleotide sequence - O16-EPA production strain stLMTB11739
atgacgaatttaaaagcagttattcctgtagcgggtctcgggatgcatatgttgcctgccactaaggcgatacccaaagagatgctaccaatcgtcgacaagccaatgattcagtacattgttgacgagattgtggctgcagggatcaaagaaatcctcctggtaactcacgcgtccaagaacgcggtcgaaaaccacttcgacacctcttatgagttagaatcactccttgagcagcgcgtgaagcgtcaactgctggcggaagtacagtccatctgtccgccgggcgtgaccattatgaacgtgcgtcagggcgaacctttaggtttaggccactccattttgtgtgcgcgacctgccattggtgacaacccatttgtcgtggtactgccagacgttgtgatcgacgatgccagcgccgacccgctacgttacaaccttgctgccatgattgcacgtttcaacgaaacgggccgcagccaggtgctggcaaaacgtatgccgggtgacctctctgaatactccgtcatccagactaaagagccgctggaccgtgagggtaaagtcagccgcattgttgaatttatcgaaaaaccggatcagccgcagacgctggactcagacatcatggccgtaggtcgctatgtgctttctgccgatatttggccggaactggaacgtactcagcctggtgcatggggacgtattcagctgactgatgctattgccgagctggcgaaaaaacaatccgttgatgcaatgctgatgaccggcgacagttacgactgcggcaaaaaaatgggctatatgcaggcgtttgtgaagtatggcctacgcaacctgaaagaaggggcgaagttccgtaaaggtattgagaagctgttaagcgaataatgaaaatctgaccggatgtaacggttgataagaaaattataacggcagtgaaaattcgcagcaaaagtaatttgttgcgaatcttcctgccgttgttttatataaaccatcagaataacaacgagttagcagtagggttttattcaaagttttccaggattttccttgtttccagagcggattggtaagacaattagcgtttgaatttttcgggtttagcgcgagtgggtaacgctcgtcacatcataggcatgcatgcagtgctctggtagctgtaaagccaggggcggtagcgtgcattaatacctctattaatcaaactgagagccgcttatttcacagcatgctctgaagtaatatggaataaattaagtgaaaatacttgttactggtggcgcaggatttattggttcagctgtagttcgtcacattataaataatacgcaggatagtgttgttaatgtcgataaattaacgtacgccggaaaccgggaatcacttgctgatgtttctgattctgaacgctatgtttttgaacatgcggatatttgcgatgcacctgcaatggcacggatttttgctcagcatcagccggatgcagtgatgcacctggctgctgaaagccatgttgaccgttcaattacaggccctgcggcatttattgaaaccaatattgttggtacttatgtccttttggaagccgctcgcaattactggtctgctcttgatagcgacaagaaaaatagcttccgttttcatcatatttctactgacgaagtctatggtgatttgcctcatccagatgaagtaaataatacagaagaattacccttatttactgagacgacagcttacgcgccaagcagcccttattccgcatccaaagcatccagcgatcatttagtccgcgcgtggaaacgtacatatggtttaccgacaattgtgactaattgctcgaacaactatggtccttatcatttcccggaaaagcttattccactggttattcttaatgcactggaaggtaaggcattacctatttatggcaaaggagatcagatccgcgactggttgtatgttgaagatcatgcgcgtgcgttatataccgtcgtaaccgaaggtaaagcgggtgaaacttataacattggtgggcacaacgaaaagaaaaacatcgatgtagtgctcactatttgtgatttgctggatgagattgtaccgaaagagaaatcttatcgtgagcaaatcacttatgttgctgatcgtccgggacacgatcgccgctatgctattgatgctgagaagattggtcgcgcattgggatggaaaccacaggaaacgtttgagagcgggattcgtaaaacggtggaatggtacctgtccaatacaaaatgggttgataatgtgaaaagtggtgcctatcaatcgtggattgaacagaactatgagggccgccagtaatgaatatcctcctttttggcaaaacagggcaggtaggttgggaactacagcgtgctctggcacctttgggtaatttgattgcttttgatgttcactctactgattattgcggtgattttagtaatcctgaaggtgtagctgaaaccgtaagaagcattcggccggatattattgtcaatgcagccgctcacaccgcagtagacaaagcagaatcagaaccggagtttgcacaattaattaacgcaacaagtgtcgaagcgattgcgaaagcagcaaatgaagttggagcctgggttatccattactcgactgattacgtcttccctggaaatggcgatatgccatggctggagacggatgcaaccgcaccactaaatgtttacggtgaaaccaagttagccggagaaaaagcgttacaggaatattgcgcgaagcatcttattttccggaccagctgggtctatgcaggaaaaggaaataacttcgccaaaacgatgttacgtctggcaaaagagcgtgaagaattagcggttattaacgatcagtttggtgcgccaacaggtgctgaactgctggctgattgtacagcacatgccattcgtgtcgcactgaataaaccggatgtcgcaggcttgtaccatttggtagccagtggtaccacaacctggtacgattatgctgcgctggtttttgaagaggcgcgcaaagcaggcattccccttgcactcaacaagctcaacgcagtaccaacaacagcctatcctacaccagctcgtcgtccacataactctcgccttaatacagaaaaatttcagcagaactttgcgcttgtcttgcctgactggcaggttggcgtgaaacgaatgctcaatgaattatttacgactacagcaatttaatagtttttgcatcttgttcgtgatggtggagcaagatgaattaaaaggaatgatgaaatgaaaatgcgtaaaggtattattttagcgggtggttctggtacacgtctttatcctgtgactatggctgtcagtaaacagctattacctatttatgataaaccgatgatctattacccgctctctacactgatgttggcgggtattcgcgatattttgattatcagtacacctcaggatactcctcgttttcaacaattgctgggtgacggtagccagtggggcctgaatcttcagtacaaagtgcaacctagcccagatggcctcgcgcaggcatttatcatcggtgaagagtttattggtggtgatgattgtgctttggttcttggtgataatatcttttacggtcacgatctgccgaagctaatggaggccgctgttaacaaagaaagtggtgcaacggtatttgcctatcacgttaatgatccagaacgctatggtgtcgttgagtttgataaaaacggtacggcaatcagtctggaagaaaaaccgttagaaccaaagagtaattacgccgttacaggtctgtacttttatgataacgacgtggttcagatggcgaaaaacttgaagccgtctgcacgtggtgagttagaaattacagatattaaccgtatttatcttgagcagggacgtctgtctgtcgcgatgatggggcgtggctacgcgtggctggacacggggactcatcagagtctgatagaagcaagtaattttattgcgacaattgaagagcgccagggattgaaggtttcctgtcctgaagagattgcatttcgtaaaggttttattgatgttgagcaagtaagaaaattagctgtaccactaataaagaataattatgggcagtatctttataaaatgacgaaggattcaaattaatgaatgtgattagaactgaaattgaagatgtgctaattctggagccaagagtatttggtgatgatagaggtttcttttatgagagctttaatcaatcagcatttgaacatattctaggctatccggtcagctttgttcaagacaatcactcacgttcatcaaaaaatgtactcagaggccttcactttcaacgcggcgagtacgcacaagataaacttgtacgctgcactcatggagcagtttttgatgttgctgttgatattcgacccaattcggtatcctttggtaaatgggttggtgttctgctttcagctgataataagcagcagttgtggataccaaaagggtttgctcatggctttttggttctgtctgatatcgctgaatttcaatataaaactacaaactattatcatcctgaaagcgattgtggaatatgttggaatgatgaacgcattgcaattgattggccccaaacatcagggttaatcctttcgccaaaagatgaaaggctctttacgttagatgagcttatcagattaaaattaattgcatgaatacgaataaattatctttaagaagaaacgttatatatctggctgtcgttcaaggtagcaattatcttttaccattgcttacatttccatatcttgtaagaacacttggtcctgaaaatttcggtatattcggtttttgccaagcgactatgctatatatgataatgtttgttgaatatggtttcaatctcacagcaactcagagtattgccaaagcagcagatagtaaagataaagtaacgtctattttttgggcggtgatattttcaaaaatagttcttatcgtcattacattgattttcttaacgtcgatgaccttgcttgttcctgaatataacaagcatgccgtaattatatggtcgtttgttcctgcattagtcgggaatttaatctaccctatctggctgtttcagggaaaagaaaaaatgaaatggctgactttaagtagtattttatcccgcttggctattatccctctaacatttatttttgtgaacacaaagtcagatatagcaattgccggttttattcagtcaagtgcaaatctggttgctggaattattgcactagctatcgttgttcatgaaggttggattggtaaagttacgctatcattacataatgtgcgtcgatctttagcagacggttttcatgtttttatttccacatctgctattagtttatattctacgggaatagttattatcctgggatttatatctggaccaacgtccgtagggaattttaatgcggccaatactataagaaacgcgcttcaagggctattaaatcctatcacccaagcaatatacccaagaatatcaagtacgcttgttcttaatcgtgtgaagggtgtgattttaattaaaaaatcattgacctgcttgagtttgattggtggtgctttttcattaattctgctcttgggtgcatctatactagtaaaaataagtatagggccgggatatgataatgcagtgattgtgctaatgattatatcgcctctgccttttcttatttcattaagtaatgtctatggcattcaagttatgctgacccataattataagaaagaattcagtaagattttaatcgctgcgggtttgttgagtttgttgttgatttttccgctaacaactctttttaaagagattggtgcagcaataacattgcttgcaacagagtgcttagttacgtcactcatgctgatgttcgtaagaaataataaattactggtttgctgaggattttatgtacgattatatcattgttggttctggtttgtttggtgccgtttgtgcgaatgagttaaaaaagctaaacaaaaaagttttagtgattgagaaaagaaatcatatcggtggaaatgcgtacacagaggactgtgagggtatccagattcataaatatggtgcacatatttttcataccaatgataaatatatatgggattacgttaatgatttagtagaatttaatcgttttactaattctccactggcgatttataaagacaaattattcaaccttccttttaatatgaatactttccaccaaatgtggggagttaaagatcctcaagaagctcaaaatatcattaatgctcagaaaaaaaagtatggtgacaaggtacctgaaaatttggaggagcaggcgatttcattagttggggaggacttataccaagcattgataaagggttatacggagaagcagtggggaagaagtgcaaaagaattgcctgcatttattattaagcgaatcccagtgagatttacgtttgataacaattatttttccgatcgctatcaaggtattccggtgggaggctacactaagcttattgaaaaaatgcttgaaggtgtggacgtaaaattaggcattgattttttgaaagacaaagattctctagcgagtaaagcccatagaatcatctacactggacccattgatcagtacttcgactataggtttggagcgttagaatatcgctctttaaaatttgagacggaacgccatgaatttccaaacttccaagggaatgcagtaataaatttcactgatgctaatgtaccatataccagaataattgagcataaacattttgactatgttgagacaaagcatacggttgttacaaaagaatatccattagagtggaaagttggcgacgaaccctactatccagttaatgataataaaaacatggagctttttaagaaatatagagagttagctagcagagaagacaaggttatatttggcgggcgtttggccgagtataaatattatgatatgcatcaagtgatatctgccgctctttatcaagtgaaaaatataatgagtacggattaatgatctatcttgtaattagtgtctttctcattacagcatttatctgtttatatcttaagaaggatatattttatccagccgtatgcgttaatatcatcttcgcactggtcttattgggatatgaaataacgtcagatatatatgcttttcagttaaatgacgctacgttgatttttctactttgcaatgttttgacatttaccctgtcatgtttattgacggaaagtgtattagatctaaatatcagaaaagtcaataatgctatttatagcataccatcgaagaaagtgcataatgtaggcttgttagttatttctttttcgatgatatatatatgcatgaggttaagtaactaccagttcgggactagcttacttagctatatgaatttgataagagatgctgatgttgaagacacatcaagaaatttctcagcatacatgcagccaatcattctaactacttttgctttatttatttggtctaaaaaatttactaatacaaaggtaagtaaaacatttactttacttgtttttattgtattcatctttgcaattatactgaatactggtaagcaaattgtctttatggttatcatctcttatgcattcatcgtaggtgttaatagagtaaaacattatgtttatcttattacagctgtaggtgttctattctccttgtatatgctctttttacgtggactgcctggggggatggcatattatctatccatgtatttggtcagccctataatcgcgtttcaggagttttattttcagcaagtatctaactctgccagttctcatgtcttttggttttttgaaaggctgatggggctattaacaggtggagtctctatgtcgttgcataaagaatttgtgtgggtgggtttgccaacaaatgtttatactgctttttcggattatgtttatatttccgcggagctaagctatttgatgatggttattcatggctgtatttcaggtgttttatggagattgtctcgaaattacatatctgtgaaaatattttattcatattttatttataccttttctttcattttttatcatgaaagcttcatgactaatattagcagttggatacaaataactctttgtatcatagtattctctcaatttcttaaggcccagaaaataaagtgaaaatgtattttttgaatgatttaaatttctctagacgcgatgctggatttaaagcaagaaaagatgcactggacattgcttcagattatgaaaacatttctgttgttaacattcctctatggggtggagtagtccagagaattattagttctgttaagcttagtacatttctctgcggtcttgaaaataaagatgttttaattttcaatttcccgatggccaaaccattttggcatatattgtcattctttcaccgccttctaaaatttagaatagtacctctgattcatgatattgatgaattaagaggaggagggggtagtgattctgtgcggcttgctacctgtgatatggtcataagtcacaatccacaaatgacaaagtaccttagtaaatatatgtctcaggataaaatcaaagacataaaaatatttgattacctcgtctcatctgatgtggagcatcgagatgttacggataagcaacgaggggtcatatatgctggcaacctttctaggcataaatgttctttcatatatactgaaggatgcgattttactctctttggtgtcaactatgaaaataaagataatcctaaatatcttggaagttttgatgctcaatctccggaaaagattaacctcccaggcatgcaatttggactcatttgggatggagattctgtcgaaacctgtagtggtgcctttggcgactatttaaagtttaataaccctcataagacatctctttatctttcaatggaacttccagtatttatatgggataaagccgcccttgcggatttcattgtagataatagaataggatatgcagtgggatcaatcaaagaaatgcaagagattgttgactccatgacaatagaaacttataagcaaattagtgagaatacaaaaattatttctcagaaaattcgaacaggaagttacttcagggatgttcttgaagaggtgatcgatgatcttaaaactcgctaaacgatatggtctctgtggttttattcggcttgttagagatgtcttattgactcgtgtattttaccggaactgtagaattattcgatttccctgctatattcgcaatgatggtagcattaattttggtgaaaatttcacaagtggagtcggtctcaggctggatgcatttggacgtggcgtgatttttttttccgataatgtgcaagttaacgactatgttcatatcgcctcaattgagagcgttacgataggtcgggatacgcttattgcaagtaaagtatttattaccgatcataatcacggttcctttaagcactctgatccaatgagttcgccaaatatacctccagacatgcgcacgttggaatcttcagctgttgtaattggccagagggtttggttgggtgagaatgtgacggttttgcctggaacaattattggtaatggagtcgtagtcggcgccaattctgttgttagaggttctattcccgaaaatactgtcattgcgggagtaccagcaaaaatcataaagaaatacaatcatgagaccaaattatgggaaaaagcatagtcgttgtttctgcggtcaattttaccactggcggtccatttaccattttgaaaaaatttttggcagcaactaataataaagaaaatgtcagttttatcgcattagtccattctgctaaagagttaaaagaaagttatccatgggttaaattcattgagtttcctgaggttaaagggtcgtggctaaaacgtttgcactttgaatatgtagtttgtaaaaaactttcaaaagagctgaatgctacgcattggatttgtctgcatgatattacggccaatgtcgtcactaaaaaaagatatgtgtattgtcataaccctgcccctttttataaaggaattttattccgtgaaattcttatggagcctagctttttcttatttaaaatgctatacgggctgatatataaaataaacattaaaaaaaatactgcagtgtttgttcaacaattctggatgaaagaaaaatttatcaagaaatattctataaataacatcattgtcagtcggccagaaattaaattatctgataaaagccaacttactgatgatgattctcaatttaagaataacccttctgagttgacaatattttaccctgctgttccacgagtatttaaaaattacgagcttattattagtgcagcaaggaaattgaaagaacaatccaatattaaatttctgcttactatcagtggtacagaaaatgcgtatgcaaaatatattatcagtcttgcagaaggactggataatgttcatttcctcgggtacttggataaagaaaaaatcgatcattgttataatatttcagatatagtttgttttccctctaggttagaaacatggggattgccgttgtctgaggctaaagagcgaggtaagtgggtattagcatcagatttcccatttactagagaaactcttggtagttatgaaaagaaagctttttttgattctaataacgatgacatgttagttaaacttattattgacttcaaaaaaggtaacctcaaaaaagatatctctgatgcaaatttcatttatcgtaatgaaaatgtattagttgggtttgatgaactagttaattttattactgaagaacattgaaatggtatatataataatcgtttcccacggacatgaagactacatcaaaaaattactcgaaaatcttaatgctgacgatgagcactacaagattatcgtacgcgacaacaaagactctctattattgaaacaaatatgccagcattatgcaggcctggactatattagtggaggtgtatacggctttggtcataataataatattgcggtggcgtatgtaaaggaaaaatatagacccgcagatgatgattacattttgtttttgaatcccgatatcatcatgaagcatgatgatttgctgacatatattaaatatgtcgaaagtaagcgttatgcttttagtacattatgcctgttccgagatgaagcgaaatctttacatgattattccgtaagaaaatttcctgtgctttctgattttattgtgtcatttatgttagggattaataaaacaaaaattcctaaagaaagtatctattctgatacggttgttgattggtgcgcaggatcatttatgctggtacgtttttcagattttgtgcgtgtaaatggcttcgatcaaggttactttatgtactgtgaagatattgacctgtgcttgaggcttagcctggctggtgtcagacttcattatgttcccgcttttcatgcgatacattatgctcatcatgacaatcgaagttttttttcaaaagccttcagatggcacttaaaaagtacttttagatatttagccagaaaacgtattttatcaaatcgcaactttgatcgaatttcatcagtttttcacccgtaagagctcggtacccgggcctagggtgtaggctggagctgcttcgaagttcctatactttctagagaataggaacttcggaataggaactaaggaggatattcatatccgtcgacggcggccgccctgcaggcatgcaagcttgatccatatggatcgctagcttaattaaataaagccgtaagcatataagcatggataagctatttatactttaataagtactttgtatacttatttgcgaacattccaggccgcgagcattcagcgcggtgatcacacctgacaggagtatgtaatgtccaagcaacagatcggcgtagtcggtatggcagtgatgggacgcaaccttgcgctcaacatcgaaagccgtggttataccgtctctattttcaaccgttcccgtgagaagacggaagaagtgattgccgaaaatccaggcaagaaactggttccttactatacggtgaaagagtttgtcgaatctctggaaacgcctcgtcgcatcctgttaatggtgaaagcaggtgcaggcacggatgctgctattgattccctcaaaccatatctcgataaaggagacatcatcattgatggtggtaacaccttcttccaggacactattcgtcgtaatcgtgagctttcagcagagggctttaacttcatcggtacgggtgtttctggcggtgaagagggggcgctgaaaggtccttctattatgcctggtggccagaaagaagcctatgaattggtagcaccgatcctgaccaaaatcgccgccgtagctgaagacggtgaaccatgcgttacctatattggtgccgatggcgcaggtcactatgtgaagatggttcacaacggtattgaatacggcgatatgcagctgattgctgaagcctattctctgcttaaaggtggcctgaacctcaccaacgaagaactggcgcagacctttaccgagtggaataacggtgaactgagcagttacctgatcgacatcaccaaagatatcttcaccaaaaaagatgaagacggtaactacctggttgatgtgatcctggatgaagcggctaacaaaggtacgggtaaatggaccagccagagcgcgctggatctcggcgaaccgctgtcgctgattaccgagtctgtgtttgcacgttatatctcttctctgaaagatcagcgtgttgccgcatctaaagttctctctggtccgcaagcacagccagcaggcgacaaggctgagttcatcgaaaaagttcgtcgtgcgctgtatctgggcaaaatcgtttcttacgcccagggcttctctcagctgcgtgctgcgtctgaagagtacaactgggatctgaactacggcgaaatcgcgaagattttccgtgctggctgcatcatccgtgcgcagttcctgcaaaaaatcaccgatgcttatgccgaaaatccacagatcgctaacctgttgctggctccgtacttcaagcaaattgccgatgactaccagcaggcgctgcgtgatgtcgttgcttatgcagtacagaacggtattccggttccgaccttctccgcagcggttgcctattacgacagctaccgtgctgctgttctgcctgcgaacctgatccaggcacagcgtgactattttggtgcgcatacttataagcgtattgataaagaaggtgtgttccataccgaatggctggattaa

SEQ ID NO: 17 - DNA, 13228 bp, Artificial Sequence
  example O18A rfb locus nucleotide sequence - O18A-EPA production strain BVEC-L-00559
atgacgaatttaaaagcagttattcctgtagcgggtctcgggatgcatatgttgcctgccactaaggcgatacccaaagagatgctaccaatcgtcgacaagccaatgattcagtacattgttgacgagattgtggctgcagggatcaaagaaatcctcctggtaactcacgcgtccaagaacgcggtcgaaaaccacttcgacacctcttatgagttagaatcactccttgagcagcgcgtgaagcgtcaactgctggcggaagtacagtccatctgtccgccgggcgtgaccattatgaacgtgcgtcagggcgaacctttaggtttaggccactccattttgtgtgcgcgacctgccattggtgacaacccatttgtcgtggtactgccagacgttgtgatcgacgatgccagcgccgacccgctacgttacaaccttgctgccatgattgcacgtttcaacgaaacgggccgcagccaggtgctggcaaaacgtatgccgggtgacctctctgaatactccgtcatccagactaaagagccgctggaccgtgagggtaaagtcagccgcattgttgaatttatcgaaaaaccggatcagccgcagacgctggactcagacatcatggccgtaggtcgctatgtgctttctgccgatatttggccggaactggaacgtactcagcctggtgcatggggacgtattcagctgactgatgctattgccgagctggcgaaaaaacaatccgttgatgcaatgctgatgaccggcgacagttacgactgcggcaaaaaaatgggctatatgcaggcgtttgtgaagtatggcctacgcaacctgaaagaaggggcgaagttccgtaaaggtattgagaagctgttaagcgaataatgaaaatctgaccggatgtaacggttgataagaaaattataacggcagtgaaaattcgcagcaaaagtaatttgttgcgaatcttcctgccgttgttttatataaaccatcagaataacaacgagttagcagtagggttttattcaaagttttccaggattttccttgtttccagagcggattggtaagacaattagcgtttgaatttttcgggtttagcgcgagtgggtaacgctcgtcacatcataggcatgcatgcagtgctctggtagctgtaaagccaggggcggtagcgtgcattaatacctctattaatcaaactgagagccgcttatttcacagcatgctctgaagtaatatggaataaattaagtgaaaatacttgttactggtggcgcaggatttattggttcagctgtagttcgtcacattataaataatacgcaggatagtgttgttaatgtcgataaattaacgtacgccggaaaccgggaatcacttgctgatgtttctgattctgaacgctatgtttttgaacatgcggatatttgcgatgcacctgcaatggcacggatttttgctcagcatcagccggatgcagtgatgcacctggctgctgaaagccatgttgaccgttcaattacaggccctgcggcatttattgaaaccaatattgttggtacttatgtccttttggaagccgctcgcaattactggtctgctcttgatagcgacaagaaaaatagcttccgttttcatcatatttctactgacgaagtctatggtgatttgcctcatccagatgaagtaaataatacagaagaattacccttatttactgagacgacagcttacgcgccaagcagcccttattccgcatccaaagcatccagcgatcatttagtccgcgcgtggaaacgtacatatggtttaccgacaattgtgactaattgctcgaacaactatggtccttatcatttcccggaaaagcttattccactggttattcttaatgcactggaaggtaaggcattacctatttatggcaaaggagatcagatccgcgactggttgtatgttgaagatcatgcgcgtgcgttatataccgtcgtaaccgaaggtaaagcgggtgaaacttataacattggtgggcacaacgaaaagaaaaacatcgatgtagtgctcactatttgtgatttgctggatgagattgtaccgaaagagaaatcttatcgtgagcaaatcacttatgttgctgatcgtccgggacacgatcgccgctatgctattgatgctgagaagattggtcgcgcattgggatggaaaccacaggaaacgtttgagagcgggattcgtaaaacggtggaatggtacctgtccaatacaaaatgggttgataatgtgaaaagtggtgcctatcaatcgtggattgaacagaactatgagggccgccagtaatgaatatcctcctttttggcaaaacagggcaggtaggttgggaactacagcgtgctctggcacctttgggtaatttgattgcttttgatgttcactctactgattattgcggtgattttagtaatcctgaaggtgtagctgaaaccgtaagaagcattcggccggatattattgtcaatgcagccgctcacaccgcagtagacaaagcagaatcagaaccggagtttgcacaattaattaacgcaacaagtgtcgaagcgattgcgaaagcagcaaatgaagttggagcctgggttatccattactcgactgattacgtcttccctggaaatggcgatatgccatggctggagacggatgcaaccgcaccactaaatgtttacggtgaaaccaagttagccggagaaaaagcgttacaggaatattgcgcgaagcatcttattttccggaccagctgggtctatgcaggaaaaggaaataacttcgccaaaacgatgttacgtctggcaaaagagcgtgaagaattagcggttattaacgatcagtttggtgcgccaacaggtgctgaactgctggctgattgtacagcacatgccattcgtgtcgcactgaataaaccggatgtcgcaggcttgtaccatttggtagccagtggtaccacaacctggtacgattatgctgcgctggtttttgaagaggcgcgcaaagcaggcattccccttgcactcaacaagctcaacgcagtaccaacaacagcctatcctacaccagctcgtcgtccacataactctcgccttaatacagaaaaatttcagcagaactttgcgcttgtcttgcctgactggcaggttggcgtgaaacgaatgctcaatgaattatttacgactacagcaatttaatagtttttgcatcttgttcgtgatggtggagcaagatgaattaaaaggaatgatgaaatgaaaatgcgtaaaggtattattttagcgggtggttctggtacacgtctttatcctgtgactatggctgtcagtaaacagctattacctatttatgataaaccgatgatctattacccgctctctacactgatgttggcgggtattcgcgatattttgattatcagtacacctcaggatactcctcgttttcaacaattgctgggtgacggtagccagtggggcctgaatcttcagtacaaagtgcaacctagcccagatggcctcgcgcaggcatttatcatcggtgaagagtttattggtggtgatgattgtgctttggttcttggtgataatatcttttacggtcacgatctgccgaagctaatggaggccgctgttaacaaagaaagtggtgcaacggtatttgcctatcacgttaatgatccagaacgctatggtgtcgttgagtttgataaaaacggtacggcaatcagtctggaagaaaaaccgttagaaccaaagagtaattacgccgttacaggtctgtacttttatgataacgacgtggttcagatggcgaaaaacttgaagccgtctgcacgtggtgagttagaaattacagatattaaccgtatttatcttgagcagggacgtctgtctgtcgcgatgatggggcgtggctacgcgtggctggacacggggactcatcagagtctgatagaagcaagtaattttattgcgacaattgaagagcgccagggattgaaggtttcctgtcctgaagagattgcatttcgtaaaggttttattgatgttgagcaagtaagaaaattagctgtaccactaataaagaataattatgggcagtatctttataaaatgacgaaggattcaaattaatgaatgtgattagaactgaaattgaagatgtgctaattctggagccaagagtatttggtgatgatagaggtttcttttatgagagctttaatcaatcagcatttgaacatattctaggctatccggtcagctttgttcaagacaatcactcacgttcatcaaaaaatgtactcagaggccttcactttcaacgcggcgagtacgcacaagataaacttgtacgctgcactcatggagcagtttttgatgttgctgttgatattcgacccaattcggtatcctttggtaaatgggttggtgttctgctttcagctgataataagcagcagttgtggataccaaaagggtttgctcatggctttttggttctgtctgatatcgctgaatttcaatataaaactacaaactattatcatcctgaaagcgattgtggaatatgttggaatgatgaacgcattgcaattgattggccccaaacatcagggttaatcctttcgccaaaagatgaaaggctctttacgttagatgagcttatcagattaaaattaattgcatgaggccggccttaaggaggactagtcccggcgcgccatgagtttaatcaaaaacagtttttggaacctttgcgggtatgtacttccagctattgtgacactaccagctttgggtattatggggcgaaaattaggcccagaattatttggtgtattcactttggcattagctgttgtgggttatgcaagcatttttgatgcaggccttactcgcgcagtgatacgagaagtcgcaattgaaaaagataatgaagaaaataagttgaaaattatttcttcagcgacagttgtaattatttatttgagtttggccgcctcactcttattatttttttttagtggtcatatcgcattgctactgaacattagtgagactttttttcataatgtaagtgtctcgcttaaaattctcgcagcatccataccattatttttgattactcaaatatggttgtcaattttagaaggtgaagaaagatttggtttacttaatatctacaaatcaattacgggagtgatattagcaatctcaccggcattatttatacttattaaaccctctttgatgtatgcgataataggcttagttctagcaaggtttttatgttttattttggcttttataatttgtcacgataaagtgcttaaagctaaactaacaatcgatataccaacaattaaaagattgtttatgttcggtggttggattacagtaagtaatatcatcagccctgtgctatcatattttgataggtttattgtttcaaatcaacttggggctgctaatgttgctttttatactgcaccatcagaaattatttctcggcttagtataattccaggtgcgttttcaagagccttatttccaagattagctaatgcaaataattccgctgaaagatataaaacgaaaagattaattacaatttcacttttaataatcatcacccctattttttgtattggcgtgttattttcagagaagataatggttttatggatgggggcatcattttttggtgagcctggtttggtattatcaatattactgattggctttatttttaatggattggcacaagtaccatttgccagtattcaatcccgaggtcatgctaagataactgcatttgttcatctcttagagttgtttccttatttattacttttattttacctcataaaagcacatggggttgttggcgcgggtattgcgtggtcagtgaggatgatagtagattatatagcattaagtcttttggacggtaagtatattaataaataaaattcaaaatgcaagttaataactcatggctttatttgggtaggtgacaatttataatgatatatatattaactttaactcttcttctagttatagccataatgttttctcttctcggcacaaaaagtaggatcacatctccattacctttgcattttttaccatggttactaactttaattgtcgggataagtaattacgatcaattttacgagtttaatgaaagaagcttttactctttgttgatttggtttacagttatttttatattttatttcataggggaactggttaattataaacgtgaaaatataaatgtttattatggtctttcacatattaaatatgaatgtaaaaaatattggatcattgtcatcccaatttcattatataccattttcgaaatatatatggttggtatggggggagcagatggattctttctcaatttacgtcttgcaaatacattggagggctatacgggtaaaaaatttatcttaatgcctgctgtatatcctctaatgatggctatgttcgcaattgtttgtctaacaaaaacttccaaattaaataaatactccatttatttctggatgtttttgtattgtattggcacaatgggaaaattttcaatattaacgccaatattgacatatttaattatttatgacttcaaacatagattaaaagtaaaaaaaacaataaagtttacattgttgataattatattagctttaactttgcattttacacgtatggctgagaatgaccactcaacatttttatctattttagggctctatatttattcaccaataattgctttaggccagttgaatgaagtaaatagtagtcattttggtgagtatacgtttagattcatatatgctataactaataaaattggccttattaaagaattgccagtaaatactattcttgactattcatacgttcctgtaccaacaaatgtatatactgcacttcaaccattttaccaggattttggttatactggcatcatatttggagcagtattatacggactaatatatgtgagtttatacacggccggtgttcgtggaaataatacacaggcattactgatttacgcattgttttcagttagcagtgcaacggctttcttcgctgaaacgctagtaacgaatttagctggaaatgtgatgttagtattatgtaccatcttactatggcgatttacagtaatatgcaaaccagtacagtaaccattctaatggccacctacaatggcgaggccttcatcaaaaatcagattttgtcactacaacaacaaacattttctaactggcggttatttattcaggatgatgggtctacagacaatactatatctataataaaaaacttccaaaaatctgactccagaattcggctagttgatgataatttgaaaggtcaaggtgcaggaaaaaattttttatcgctgataaagtacagcgagacagattatacaatttattgtgaccaagatgatatttggttagaaaacaaaatatttgaattagtaaagtatgcaaatgaaattaaattgaatgtatcagatgcgccttcgctagtttatgctgatggctatgcttatatggatggtgagggtacaatcgatttttctgggatatctaacaatcatgctgatcaattaaaggattttcttttttttaatggtggataccaaggatgttctattatgttcaatcgtgcaatgaccaaatttcttctgaattatcgaggatttgtatatctacatgacgatatcacaacattagctgcatacgctcttggtaaagtttattttctcccgaaataccttatgttatatagacagcacacgaatgcggtaactggtatcaaaacattccgcaatggattgacttctaaatttaaatcaccagtaaactatcttttatcacgaaaacattatcaggtaaaaaaatctttttttgaatgtaacagctctatcttatcagagacgaataaaaaagtttttttggattttatttcattttgtgaatcaaataataaatttacagatttttttaagttatggcgaggtgggtttagattaaataacagtagaactaaattattattaaaattcttaatacggagaaaatttagcgaatgatttcaatacttacacctacttttaatcggcaacatactttatcaaggctattcaattctcttatattacaaactgataaagattttgagtggataataattgatgatggtagtatagatgcaacagcggtacttgtagaagattttagaaaaaaatgtgattttgacttgatttattgctatcaggaaaataatggtaagcccatggctttaaacgctggtgttaaagcttgtagaggcgattatatctttattgttgacagtgatgatgcactaactcccgatgccataaaattaattaaagaatcaatacatgattgcttatctgagaaggaaagtttcagcggagtcggttttagaaaagcatatataaaaggggggattattggtaatgatttaaataattcttcagaacatatatactatttaaatgcgactgagattagcaatttaataaatggtgatgttgcatattgttttaaaaaagaaagtttggtaaaaaatccattcccccgtatagaagatgaaaaatttgttccagaattatatatttggaataaaataactgacaaggcgaagattcgatttaacataagcaaagttatatatctttgtgagtatcttgatgatggtctttctaaaaatttccataaccagcttaaaaaatacccaaaggggtttaagatttattacaaagatcaaagaaaacgagagaaaacttatataaaaaaaacaaagatgctaattagatatttgcaatgttgttattatgagaaaataaaatgaaaatactatttgtcattacaggtttaggccttggaggtgctgagaagcaggtttgtcttttagctgataaattaagtttaagcgggcaccatgtaaagattatttcacttggacatatgtctaataataaagtctttcctagcgaaaataatgttaatgtcattaatgtaaatatgtcaaaaaacatttctggagttataaaaggttgtgtcagaattagagatgttatagctaatttcaaaccagacattgtacacagtcatatgtttcatgcaaacattatcactagattgtctgtaattggaatcaaaaacagacctggtattatatcaactgcacataataaaaatgaaggtgggtatttcagaatgctcacatatagaataaccgattgtttaagtgattgttgtacaaatgttagcaaagaagcagtggatgagtttttacggataaaagcctttaatcccgctaaagcaattactatgtataatgggatagataccaataaatttaaatttgatttattggcaaggagggaaattcgagacggtattaatataaaaaatgatgatatattattacttgctgcaggtcgtttaacgttagctaaagattatcctaatttattgaatgcaatgactctgcttcctgaacactttaaacttattattattggtgatggtgaattgcgtgacgaaattaatatgcttataaaaaaattgcaattatctaatagggtgtccttgttgggagttaaaaaaaatattgctccctatttttctgcatgtgatatttttgttctctcttctcgttgggaaggatttggattagtcgtggcagaagctatgtcatgtgagcgaattgttgttggcacggattcagggggagtaagagaagttattggtgacgatgattttcttgtacccatatctgattcaacacaacttgcaagcaaaattgaaaaattgtctttgagccagatacgtgatcacattggttttcggaatcgtgagcgtattttaaaaaatttctcaatagatactattattatgcagtggcaagaactctatggaactataatttgctcaaaacatgaaaggtagatttatatttggaacgtgtcttttgtttgaatttaattcaatctcaattgagatttttgtatttcaaaaataccatcatagctaacgatgattggtatttattttaagatgctttctataaatatattgacgtttttaatgcgccgaaacgattgggctgggaacagagaagtaaaactgttttgagaatgaagagtttttgagatgtttatggatattaaaaattgatccagtgaattaattatttataataaatcaagatttaatgttaataaatgataatcttttctgacactcatattaattatgagtggtacgtttggtaaacggtaaactattatatgacagctagaacaactaaagttttgcacttacaattactcccactcttaagtggcgttcaaagggtaacattaaacgaaattagtgcgttatatactgattatgattatacactagtttgctcaaaaaaaggtccactaacaaaagcattgctggaatatgatgtcgattgtcattgtatccccgaacttacgagagaaattaccgtaaagaatgattttaaagcattgttcaagctttataagttcataaaaaaagaaaaatttgacattgtgcatacacattcttcaaaaacaggtattttggggcgagttgctgccaaattagcacgtgttggaaaggtgatccacactgtacatggtttttcttttccagccgcatctagtaaaaaaagttattacctttattttttcatggaatggatagcaaagttctttacggataagttaatcgtcttgaatgtagatgatgaatatatagcaataaacaaattaaaattcaagcgggataaagtttttttaattcctaatggagtagacactgataagttttctcctttagaaaataaaatttatagtagcaccttgaatctagtaatggttggtagattatccaagcaaaaagatcctgagacattattgcttgctgttgaaaaactgctgaatgaaaatgttaatgttaagctgacacttgtaggagatggtgaactaaaagaacagttagaaagcaggttcaaacggcaagatggacgtataatttttcatggatggtcagataacattgttaatattttaaaagttaatgatctttttatattaccttctctttgggagggtatgccattagcaattttagaagcattgagctgtggacttccatgtatagtcactaatattccaggtaataatagcttaatagaagatggctataatggttgtttgtttgaaattagagattgtcagttattatctcaaaaaatcatgtcatatgttggtaagccagaactgattgcacagcaatctaccaatgcacgatcatttattctgaaaaattatggattagttaaaagaaataataaggtcagacagctatatgataattaagagctcggtacccgggcctagggtgtaggctggagctgcttcgaagttcctatactttctagagaataggaacttcggaataggaactaaggaggatattcatatccgtcgacggcggccgccctgcaggcatgcaagcttgatccatatggatcgctagcttaattaaataaagccgtaagcatataagcatggataagctatttatactttaataagtactttgtatacttatttgcgaacattccaggccgcgagcattcagcgcggtgatcacacctgacaggagtatgtaatgtccaagcaacagatcggcgtagtcggtatggcagtgatgggacgcaaccttgcgctcaacatcgaaagccgtggttataccgtctctattttcaaccgttcccgtgagaagacggaagaagtgattgccgaaaatccaggcaagaaactggttccttactatacggtgaaagagtttgtcgaatctctggaaacgcctcgtcgcatcctgttaatggtgaaagcaggtgcaggcacggatgctgctattgattccctcaaaccatatctcgataaaggagacatcatcattgatggtggtaacaccttcttccaggacactattcgtcgtaatcgtgagctttcagcagagggctttaacttcatcggtaccggtgtttctggcggtgaagagggggcgctgaaaggtccttctattatgcctggtggccagaaagaagcctatgaattggtagcaccgatcctgaccaaaatcgccgccgtagctgaagacggtgaaccatgcgttacctatattggtgccgatggcgcaggtcactatgtgaagatggttcacaacggtattgaatacggcgatatgcagctgattgctgaagcctattctctgcttaaaggtggcctgaacctcaccaacgaagaactggcgcagacctttaccgagtggaataacggtgaactgagcagttacctgatcgacatcaccaaagatatcttcaccaaaaaagatgaagacggtaactacctggttgatgtgatcctggatgaagcggctaacaaaggtacgggtaaatggaccagccagagcgcgctggatctcggcgaaccgctgtcgctgattaccgagtctgtgtttgcacgttatatctcttctctgaaagatcagcgtgttgccgcatctaaagttctctctggtccgcaagcacagccagcaggcgacaaggctgagttcatcgaaaaagttcgtcgtgcgctgtatctgggcaaaatcgtttcttacgcccagggcttctctcagctgcgtgctgcgtctgaagagtacaactgggatctgaactacggcgaaatcgcgaagattttccgtgctggctgcatcatccgtgcgcagttcctgcaaaaaatcaccgatgcttatgccgaaaatccacagatcgctaacctgttgctggctccgtacttcaagcaaattgccgatgactaccagcaggcgctgcgtgatgtcgttgcttatgcagtacagaacggtattccggttccgaccttctccgcagcggttgcctattacgacagctaccgtgctgctgttctgcctgcgaacctgatccaggcacagcgtgactattttggtgcgcatacttataagcgtattgataaagaaggtgtgttccataccgaatggctggattaa

SEQ ID NO: 18 - DNA, 13554 bp, Artificial Sequence
  example O25B rfb locus nucleotide sequence - O25B-EPA production strain stGVXN4459
atgacgaatttaaaagcagttattcctgtagcgggtctcgggatgcatatgttgcctgccactaaggcgatacccaaagagatgctaccaatcgtcgacaagccaatgattcagtacattgttgacgagattgtggctgcagggatcaaagaaatcctcctggtaactcacgcgtccaagaacgcggtcgaaaaccacttcgacacctcttatgagttagaatcactccttgagcagcgcgtgaagcgtcaactgctggcggaagtacagtccatctgtccgccgggcgtgaccattatgaacgtgcgtcagggcgaacctttaggtttaggccactccattttgtgtgcgcgacctgccattggtgacaacccatttgtcgtggtactgccagacgttgtgatcgacgatgccagcgccgacccgctacgttacaaccttgctgccatgattgcacgtttcaacgaaacgggccgcagccaggtgctggcaaaacgtatgccgggtgacctctctgaatactccgtcatccagactaaagagccgctggaccgtgagggtaaagtcagccgcattgttgaatttatcgaaaaaccggatcagccgcagacgctggactcagacatcatggccgtaggtcgctatgtgctttctgccgatatttggccggaactggaacgtactcagcctggtgcatggggacgtattcagctgactgatgctattgccgagctggcgaaaaaacaatccgttgatgcaatgctgatgaccggcgacagttacgactgcggcaaaaaaatgggctatatgcaggcgtttgtgaagtatggcctacgcaacctgaaagaaggggcgaagttccgtaaaggtattgagaagctgttaagcgaataatgaaaatctgaccggatgtaacggttgataagaaaattataacggcagtgaaaattcgcagcaaaagtaatttgttgcgaatcttcctgccgttgttttatataaaccatcagaataacaacgagttagcagtagggttttattcaaagttttccaggattttccttgtttccagagcggattggtaagacaattagcgtttgaatttttcgggtttagcgcgagtgggtaacgctcgtcacatcataggcatgcatgcagtgctctggtagctgtaaagccaggggcggtagcgtgcattaatacctctattaatcaaactgagagccgcttatttcacagcatgctctgaagtaatatggaataaattaagctagcagtgaagatacttgttactggtggcgcaggatttattggttctgctgttgttcgtcacataataaataatacgcaagatagtgttgttaatgtcgataaattaacatacgccggaaacctggaatcacttgcagatgtttctgattctgaacgctatttctttgaacatgcggatatttgtgatgcagctgcaatggcacggatttttgctcagcatcagccggatgcagtgatgcacctggcagctgaaagccatgttgaccgttcaattacaggccctgcggcatttattgaaaccaatattgtgggtacttatgtccttttagaagcggctcggaattattggtctggtctggatgatgaaaagaaaaaaaacttccgttttcatcatatttctactgatgaggtgtatggtgacttaccccatccggatgaagtaaatagcaatgaaacgttgccgctatttacggaaacgacagcatacgcgccaagtagtccatattctgcttctaaagcttccagcgatcatttggttcgcgcatggaaacgtacttatggtttaccgaccattgtgactaattgctcgaacaactatggtccttatcatttcccggaaaagcttattccactggttattcttaattcactggaaggtaaggcattacctatttatggcaaaggagatcagatccgcgactggttgtatgtagaggatcatgctcgagcgttatataccgtcgtaaccgaaggtaaagcgggcgaaacttataacattggtggacacaacgaaaagaaaaacatcgacgtagtgttcactatttgtgatttgttggatgagatagtcccgaaagagaaatcttaccgcgagcaaattacttatgttaccgatcgtccgggacacgatcgccgttatgcgattgatgctgagaagattggtcgcgaattgggatggaaaccacaggaaacgtttgagagtgggattcgtaaaacggtggaatggtacctgtccaatacaaaatgggttgataatgtgaaaagtggtgcctatcaatcgtggattgaacagaactatgagggccgccagtaatgaatatcctcctttttggcaaaacagggcaggtaggttgggaactacagcgtgctctggcacctctgggtaatttgattgctcttgatgttcactccactgattactgtggtgattttagtaatcctgaaggtgtagctgaaaccgtaagaagcattcggcctgatattattgtcaacgcagccgctcacaccgcagtagacaaagcagaatcagaaccgaagtttgcacaattactgaacgcgacgagtgtcgaagcgatcgcgaaagcagccaatgaagtcggcgcctgggttattcactactctactgactacgtatttccggggaccggtgaaataccatggcaggaggaggatgcaaccgcaccgctaaatgtttacggtgaaaccaagttagcgggagaaaaagcattacaagagcattgtgcgaagcaccttattttccggaccagctgggtctatgcaggtaaaggaaataacttcgccaaaacaatgttgcgtctggcaaaagagcgtgaagaattagccgttattaatgatcagtttggtgcgccaactggcgcagagttactggctgattgtacggcacatgctattcgtgtggcactgaataaaccggaagtcgcaggcttgtaccatctggtagctagtggtaccacaacgtggcacgattatgctgcgctggtttttgaagaggcgcgcaaagcaggcattccccttgcactcaacaagctcaacgcagtaccaacaacagcctatcctacaccagctcgtcgtccacataactctcgccttaatacagaaaaatttcagcagaactttgcgcttgtcttgcctgactggcaggttggcgtgaaacgaatgcttaacgaattatttacgactacagcaatttaatagtttttgcatcttgttcgtaatggtggagcaagatgtattaaaaggaatgatgaaatgaaaacgcgtaaaggtattattttggcgggtggttctggtactcgtctttatcctgtgacgatggccgtcagtaaacagctgttaccgatttatgataaaccgatgatctattacccgctctctacactgatgttagcgggtattcgcgatattctgattatcagtacaccacaggatactcctcgttttcaacaactgctgggtgacgggagccagtggggcctgaatcttcagtacaaagtgcaaccgagtccggatggtcttgcgcaggcgtttattatcggtgaagagtttattggtggtgatgattgtgctttggtacttggtgataatatcttctacggccacgacctgccgaagttaatggacgtagctgttaacaaagaaagtggtgcaacggtatttgcctatcacgttaatgatcctgaacgttatggtgtcgtggagtttgataataacggtactgcaattagcctggaagaaaaaccgctggaaccaaaaagtaactatgcggttactgggctttatttctatgacaatgacgttgtggaaatggcgaaaaaccttaagccttctgcccgaggtgaactggaaattaccgatattaaccgtatttatatggaacaaggacgtttgtctgtcgctatgatggggcgtggctatgcatggctggatacagggacgcatcaaagtcttattgaagcaagcaacttcattgccaccattgaagagcgccagggactaaaggtttcctgtccggaagaaattgcttatcgtaaagggtttattgatgctgagcaggtaaaagtattagccgaaccgttgaagaaaaatgcttatggtcagtatctgctcaaaatgattaaaggttattaataagatgaacgtaattaaaactgaaattcctgatgtgctgatttttgaaccaaaagtttttggggatgaacgtggcttcttttttgagagttttaatcagaggatttttgaagaagcagtaggtcgtaaggttgagtttgttcaggataaccattctaagtccagtaaaggtgttttacgtggtcttcattatcagttagaaccttatgctcaaggaaaactggtgcgctgtgttgttggcgaggtttttgatgttgcggttgatattcgtaaatcgtcacctacatttgggaaatgggttggggtgaatttgtctgctgagaataagcgtcagttgtggattcctgagggatttgcacatggttttttggtgctgagtgatttagcagaagttttatataaaacgaatcaatattatgctccatcacatgaaaaaaatattatatggaatgacctcttgcttaatattaaatggccgagcacagcactgatcactctgtctgataaggatgcaaatggggaaagatttgaactaagtgagttttgaaatgtctctcttaaaacatagtatatggaatgttgcgggctactttataccaacattaattgcaattcccgcctttggattaattgcgaggaaaattggtgtagaactatttggtttgtatacgttagcaatgatttttatagggtatgcaagtatatttgatgctgggttaacaagagctgttgtgcgtgaaatagcattactaaaaaacagagtggacgattgtaatacgataatagtaacttctattatcgctgtgatatttttagggtttatcggaggcgggggagtgtttctgcttaaaggcgatattattgaactgttaaatatctcaccaatatattacgccgattcgataaagtctctagtattattatcatctctgatacctgtattcttagtcacgcaaatactattagcagagcttgagggtcgggaatattttgggattctaaatatacaaaaaagtgtagggaattctttaattgcagggttacctgcattatttgttttaattaatcaaacgcttttttctgcaattattggtgtagcgattgcaagagttatatgcttgtggttaagctacattatgagcagggaaagaataactatcgatatctcatttttttcaataactgttttaaagcggttatttagatatggcgggtgggtaactataagtaacataatatctcctatattagcgagtatggatagatttattctatcccatatccagggagcatcaaaaatatcattctatacagtccctaatgagctggtaactaggcttggaatagttccaggctctcttgggaaagctgtttttccaaaattaagtcatgcaaggaattttacagcgtcatatgcagagcaaaaaaaagcttatatattaatgactgtcattgtaatgcctttggttttatttgtatattattacgcaaagtttattttaacattgtggatgggggctgagtatgcagggatttcggtcgaaatattacggattatgcttatagggtatatttttaactgttattcacaaatctcttttgccaacatacaggcctttggaaaagcaaaatacactgcatacatccatatgatggaatttattccttatttgataatgttatatataatttcaaaggaatatggggttattggtgttgcgtggttatggacaattcgagtaataattgattttttgatgcttttatatatgagttatcgttgtaataatcttatgaaaaaagggtagcctgatgatatatattgtggtattaaattggaatggggctatagataccattaattgtgttaaaagtttaatggatttaaatgttagcgattataaaattatcattgttgataactgttctatggataactcatatgatactataaaagaaaatcttaattcattatatattgctgataaaagtatcattgaggtgaagtatgaggatagaaataaatataaaaccttagaaaacgataaaatcatattaatacaatctccgcaaaataatgggtacgcaagtggtaataatattggcatagagttcgctcttaatcaggagaatatgaaatacgtctgggttctgaataatgatactgaagtggataaagaggctttaactcatttaattagtaaatgtgattcagataaaagtatagggatttgcggttctcgtttagtctattttgccgacagagagatgcagcaaggactaggtggggtgcataacaaatggttatgcactacaaaaaattatgaaatgggaagattagtttccaaaaaatatgatgatgaagtcattagtaatgatatagattatataattggcgcatcgatgtttttctctagagaatgtttggaaacagttggattgatgaatgaagaatattttttatactatgaagagttagatatttgcctcagagcaaaagcaaagaactttaaattaggtatttgctcagaaagtttggtttatcataaaataggtgcaagtactgatgggggaaagagcatgatggctgatctttgctcaataaaaaataggctggtcattacagaaaggttttatccccaatattattggacggtatggttgtcactttttgttgtagcatttaaccgtgctagaagaggtgagtttaataagatgaaaagatgtttgaatgttatgtttaacttcaaacgaaacaaaggtagcaaatgccattagaatatgcacttaatcatggtgttaataaatctatagtttgatatgttattaaagggtatttaatgaaagtggcttttttatctgcttatgatccactatctacatccagttggtctggcacaccttattatatgctaaaggcattatcgaagagaaatatttccattgaaatattaggaccggtaaatagctatatgatatacatgttaaaagtatataaattaatattaaggtgtttcggaaaagaatatgattatagtcattcgaagttgctttccaggtattacggtagaatattcggtaggaaattaaaaaaaattgatggtttggattttattatcgcacctgcaggttcctcacaaattgcttttttaaaaacaaccataccaataatatatctatcggatacaacatatgatcaattaaaaagctattatccgaatttaaataaaaaaacaattataaatgatgaggatgcaagtttaatcgaacgcaaggctattgaaaaagcaacagtagtatctttcccatctaaatgggcaatggatttttgcaggaattattacagattagattttgataaattagttgaaataccatggggggctaatttatttgatgatattcactttgctaataaaaatataattcaaaagaatagttatacttgtcttttcttgggagttgattgggaaagaaaaggtgggaaaacagccttgaaagcaattgaatatgtaaggcagttatatgggatcgatgttagactaaaaatttgtggatgtactccgaatcaaaagattttacctacttgggttgaattaattgataaagtagataaaaataacgttgacgaatatcagaaattcatcgatgtgttatctaacgctgatatacttcttttaccaaccattgctgaatgttatggaatggtattttgtgaagctgctgcttttggattgcctgttgtcgctacagatacaggtggagtcagttctatagttatcaacgaaaggacggggatattaattaaagacccgttagactataagcactttggaaatgcaattcataaaataattagttccgtagagacttatcaaaactactcccaaaacgcaagaattagatataataatatattgcattgggacaattgggctaaaaagataattgagattatgtatgagcataagaatagaagaatcaaatagcacaaaaagaattatatgtttatttatactttttcttgttttccctgattttttgttttatacattaggggttgataattttagcatttcaacgataatctcaattacattgctttttgtttttttaagagctaaaaatatttgcaaagataattttctaataatagtagcgttattcatattgttgtgttttaactgtttgttaagtatgctatttaatattgaacaggctttaacatttaaagttgtactttcaatatatagcatcttaataatggcatacgtctcctcttgttatgcacagacgttgtggttatgttctgaagaaatacttaagagatccgtcttttatttgttcgcatttctttgccttattggcattataagtattcttttacagaagactgagattatacatgataaaagtatgattctttttcctgaaccatcagcatttgcattggtttttatacctatcttttcattttgtttatactatacaagagggggggggctactattgctctatatattatctttgggtattgcgttaggtatccagaatttaacaatgttggtaggcattgtgattagtgtttttgtgatgaaaaaaataactataaggcaaactattgttatacttttgggggcatggattttttccatgatattaagtgatttagacatttcttactatacatcgcggcttgattttaaaaatactacgaacctatcagtgcttgtatatctttcaggaattgaaagagctttcttgaattttattacaagttatggtcttggtattggttttcaacaaatgggagtgaatggggagataggaatatatcaacaaattttagctgaacttgatgcccctatgttaaatatatacgatggctcatttatttcttctaagttaatatctgagtttggggttattggtgcattaatgtgtattttctattttttttatttttcccgattttatctgcgtttcaaaaaaagtaagagatattcaccgcagtatattttagcatatagcttctacatgtgtttcttcatccctctttttatacgtggtgctggttatataaacccctatgtgtttatgttattttcatcaatatttttgtgcaaatatcacgctaaaaatatcttgatgaaatctaatgtccagatagctatataatagtagattatattatcattatcacgtaaattacatattaatagcatatatgataactaggacataaataatgtgcattaaaaaaaaacttaagttaattaaacgatatggcctttatggtggtcttaggcttcttaaagatatattcttaacaaaatttttattttgttcaaatgttaggattattagatttccatgttatattagaaaagatggaagtgttagttttggaaaaggttttacatcaggtgtaggattacgagttgatgcatttatggatgccgtagtttccattggagaaaatgttcaaattaatgactatgttcacatcgcggctattaataatgtcattattggtagagatacattaatagcaagtaaagtatttattagtgatcataatcatggtattttttctaaatccgatatccatagttcaccaactattattccttcgtctaggccccttgaatctgcacctgtgtatattggagagcgtgtgtggattggcgaaaatgtgacaatattaccaggtgcgtgtataggtaatggtgtagttattggcgcaaacagtgttgttcgtggtgagattcctaataatgtgatcattgctggtgttccagctaaaattgttaaaaaatataactatgagcgtatgcaatgggaaagaatatagttgtaatatcggctgttaattttacaaccggaggcccctttaccgtactaaaaaatgtgcttacagcaactaaagatagagccgaatgtaaatttattgcactggttcatagctctgctgaactaatggaattatttccgtgggttgaatttatagagtatccagaagtcaagtcttcgtgggttaaaagattatatttcgaatatataacttgcaatagattatctaaggtgattaaggcaactcattgggtatgcttacatgatattacagcaaatgttagtgtaccctatagatttgtttattgccacaatcctgcaccgttctataaatatttaagctatcgagatattataggagaacctaaattttatcttttttatcttttttatgggcttttatacaatatcaatataaaaaagaacacagcagtttttgttcagcagcagtggctaaaaaaagaattcgaaaaaaaatataagttaaagaatgttgttgttagtcgccctgaagatatttgcccttttgaaagtgatggtttggtaagaaataataataaaaaggatgtgaggatattttacccagcagtgccccgtatatttaaaaactttgaagttatcatacgtgctgcacaaatattacaagataaaaatattcatttttatcttacttttgatggtactgaaaataagtatgcaaaaagaatatataaattagcttccgaactgaaaaatgtacatttcctcggttaccttaatgcaaccgagatggttaacttttatcaagattcagatattatttgtttcccatcgaaactagaaacgtggggattaccattatcagaagctaaaacatacaaaaaatggatatttgcggcagacttaccttatgctcatgaagttttatataactattcaaaaactagatattttccatttgacgatgagaaaatacttgttcgctacatattagagtacacaagtaaaaatatgcatgaagatataaaaaatagtagggtgaattttaataatgatgcattgactggttttgaacagtttattgaatatatcctcaaggggaactgacgtggtttatattataatcgtttcacatggccatgatgactatatagaaaatcttttattaaatttaaagttgccctctggaagatttaaaataatagttcgtgataacaaaagttcaatggttttaaaaaaaacatgcgaaaaaaattgcgtaacctatttgcatggagggcaatatggatttggacataataataacatagcagtgtcatatataattaataacttcatgattatgaataatgattattttctctttcttaaccccgatgtattcataaccagtgaaagtttgattaattatgttgattatataattagtaatgattataagtttagcacattatgtctttatcgagattttactaaaagcaaacatgattattcaatacggagttttccaactttatatgattttctttgttcttttttattgggggtgaataaaagtaaaattaagaaggaaaatatactttctgatactgtagttgattggtgtgctggctcatttatgcttattcatgctttaagtttcttaaatgtgaatggttttgatcaaaaatattttatgtattgtgaagatattgacctttgtatgcgtttaaaattaagtggagtagatctttactatactccccattttgatgctattcattatgcgcagcatgaaaatagaagaatatttactaaagcatttcgatggcatataaggagtattacgcgctacatattacggaaaccaattctttcttataaaaactatagaaaaattacatccgaactggtaaagtgattaaggatccgtgtaggctggagctgcttcgaagttcctatactttctagagaataggaacttcggaataggaactaaggaggatattcatatggataaagccgtaagcatataagcatggataagctatttatactttaataagtactttgtatacttatttgcgaacattccaggccgcgagcattcagcgcggtgatcacacctgacaggagtatgtaatgtccaagcaacagatcggcgtagtcggtatggcagtgatgggacgcaaccttgcgctcaacatcgaaagccgtggttataccgtctctattttcaaccgttcccgtgagaagacggaagaagtgattgccgaaaatccaggcaagaaactggttccttactatacggtgaaagagtttgtcgaatctctggaaacgcctcgtcgcatcctgttaatggtgaaagcaggtgcaggcacggatgctgctattgattccctcaaaccatatctcgataaaggagacatcatcattgatggtggtaacaccttcttccaggacactattcgtcgtaatcgtgagctttcagcagagggctttaacttcatcggtaccggtgtttctggcggtgaagagggggcgctgaaaggtccttctattatgcctggtggccagaaagaagcctatgaattggtagcaccgatcctgaccaaaatcgccgccgtagctgaagacggtgaaccatgcgttacctatattggtgccgatggcgcaggtcactatgtgaagatggttcacaacggtattgaatacggcgatatgcagctgattgctgaagcctattctctgcttaaaggtggcctgaacctcaccaacgaagaactggcgcagacctttaccgagtggaataacggtgaactgagcagttacctgatcgacatcaccaaagatatcttcaccaaaaaagatgaagacggtaactacctggttgatgtgatcctggatgaagcggctaacaaaggtaccggtaaatggaccagccagagcgcgctggatctcggcgaaccgctgtcgctgattaccgagtctgtgtttgcacgttatatctcttctctgaaagatcagcgtgttgccgcatctaaagttctctctggtccgcaagcacagccagcaggcgacaaggctgagttcatcgaaaaagttcgtcgtgcgctgtatctgggcaaaatcgtttcttacgcccagggcttctctcagctgcgtgctgcgtctgaagagtacaactgggatctgaactacggcgaaatcgcgaagattttccgtgctggctgcatcatccgtgcgcagttcctgcagaaaatcaccgatgcttatgccgaaaatccacagatcgctaacctgttgctggctccgtacttcaagcaaattgccgatgactaccagcaggcgctgcgtgatgtcgttgcttatgcagtacagaacggtattccggttccgaccttctccgcagcggttgcctattacgacagctaccgtgctgctgttctgcctgcgaacctgatccaggcacagcgtgactattttggtgcgcatacttataagcgtattgataaagaaggtgtgttccataccgaatggctggattaa

SEQ ID NO: 19 - DNA, 15197 bp, Artificial Sequence
  example O75 rfb locus nucleotide sequence - O75-EPA production strain stLMTB11737
atgacgaatttaaaagcagttattcctgtagcgggtctcgggatgcatatgttgcctgccactaaggcgatacccaaagagatgctaccaatcgtcgacaagccaatgattcagtacattgttgacgagattgtggctgcagggatcaaagaaatcctcctggtaactcacgcgtccaagaacgcggtcgaaaaccacttcgacacctcttatgagttagaatcactccttgagcagcgcgtgaagcgtcaactgctggcggaagtacagtccatctgtccgccgggcgtgaccattatgaacgtgcgtcagggcgaacctttaggtttaggccactccattttgtgtgcgcgacctgccattggtgacaacccatttgtcgtggtactgccagacgttgtgatcgacgatgccagcgccgacccgctacgttacaaccttgctgccatgattgcacgtttcaacgaaacgggccgcagccaggtgctggcaaaacgtatgccgggtgacctctctgaatactccgtcatccagactaaagagccgctggaccgtgagggtaaagtcagccgcattgttgaatttatcgaaaaaccggatcagccgcagacgctggactcagacatcatggccgtaggtcgctatgtgctttctgccgatatttggccggaactggaacgtactcagcctggtgcatggggacgtattcagctgactgatgctattgccgagctggcgaaaaaacaatccgttgatgcaatgctgatgaccggcgacagttacgactgcggcaaaaaaatgggctatatgcaggcgtttgtgaagtatggcctacgcaacctgaaagaaggggcgaagttccgtaaaggtattgagaagctgttaagcgaataatgaaaatctgaccggatgtaacggttgataagaaaattataacggcagtgaaaattcgcagcaaaagtaatttgttgcgaatcttcctgccgttgttttatataaaccatcagaataacaacgagttagcagtagggttttattcaaagttttccaggattttccttgtttccagagcggattggtaagacaattagcgtttgaatttttcgggtttagcgcgagtgggtaacgctcgtcacatcataggcatgcatgcagtgctctggtagctgtaaagccaggggcggtagcgtgcattaatacctctattaatcaaactgagagccgcttatttcacagcatgctctgaagtaatatggaataaattaagctagcagtgaagatacttgttactggtggcgcaggatttattggttctgctgttgttcgtcacataataaataatacgcaagatagtgttgttaatgtcgataaattaacatacgccggaaacctggaatcgctcgctgaaatttctgattctgaacgttattcatttgagcatgcagatatctgcgatgccgaagcgatggctcgtattttcgcacagcaccagccagacgcggtgatgcacctggcagcagagagccacgttgaccgctcaataactggccctgcggcatttattgaaaccaatattgtgggtacttatgttcttttagaagcggcgcgcaattattggtctggtctggatgatgaaaagaaaaaaaacttccgctttcatcatatttctactgatgaggtgtatggtgacttaccccatccggatgaagtaaatagcaatgaaacgttgccgctatttacggaaatgacagcatacgcgccaagtagtccatattctgcttctaaagcttccagcgatcatttggttcgcgcatggaaacgtacttatggtttaccgaccattgtgactaattgctcgaacaactatggtccttatcatttcccggaaaagcttattccactggttattcttaatgcactggaaggtaaggcattacctatttatggcaaaggagatcagatccgcgactggttgtatgtagaggatcatgctcgagcgttatataccgtcgtaaccgaaggtaaagcgggcgaaacttataacattggtggacacaacgaaaagaaaaacatcgacgtagtgttcactatttgtgatttgttggatgagatagtcccgaaagagaaatcttatcgtgagcaaattacctatgttgctgatcgcccagggcatgatcgccgttatgcaattgatgccgataaaattagccgcgaattgggctggaaaccacaggaaacgtttgagagcgggattcgtaaaactgtggaatggtatctgtccaatacaaaatgggttgataatgtgaaaagtggtgcctatcaatcgtggattgaacagaactatgggggccgccactaatgaatatcctcctttttggcaaaacagggcaggttggttgggaactacagcgtgctctggcacctctgggtaatttgattgctcttgatgttcactccactgattactgtggtgattttagtaaccctgaaggtgtggctgaaaccgttagaagcattcggcctgatattattgtcaacgcagccgctcacaccgcagtagacaaagcagaatcagaaccggagtttgcacaattactgaacgcgacgagtgtcgaagcgatcgcgaaagcagccaatgaagtcggcgcttgggttattcactactctactgactacgtatttccggggaccggtgaaataccatggcaggaggaggatgcaaccgcaccgctaaatgtttacggtgaaaccaagttagcaggagaaaaagcattacaagagcattgtgcgaagcaccttattttccggaccagctgggtctatgcaggtaaaggaaataacttcgccaaaacgatgttgcgtctggcaaaagagcgtgaagaattagccgttattaatgatcagtttggtgcgccaactggcgcagagttgctggctgattgtacggcacatgccattcgtgtggcactgaataaaccggaagtcgcaggtttgtaccatctggtagccagtggtaccacaacctggcacgattatgctgcgctggtttttgaagaggcgcgcaaagcaggcattccccttgcactcaacaagctcaacgcagtaccaacaacagtctatcctacaccagctcgtcgtccacataactctcgccttaatacagaaaaatttcagcagaactttgcgcttgtcttgcctgactggcaggttggtgtgaaacgcatgctcaacgaattatttacgactacagcaatttaatagtttttgcatcttgttcgtgatggtggaacaagatgaattaaaaggaatgatggaatgaatacgcgtaaaggtattattttagcgggtggttctggtacacgtctttatcctgtgactatggctgtcagtaaacagctgttaccgatttatgataaaccgatgatctattacccgctctctacactgatgttggcgggtattcgcgatattttgattatcagcacgccacaggatactcctcgttttcaacaactgctgggtgatgggagccagtgggggctaaatcttcactacaaagtgcaaccgagtccggatggtcttgcgcaggcatttatcatcggtgaagagtttatcggtggtgatgattgtgctttggtacttggtgataatatcttctacggtcacgacctgcctaagttaatggatgccgctgttaacaaagaaagtggtgcaacggtatttgcctatcacgttaatgatcctgaacgctatggtgtcgttgagtttgataaaaacggtactgcaatcagcctggaagaaaaaccgttacaaccaaaaagtaattatgcggtaaccgggctttatttctatgataactacgttgtggaaatggcgaaaaatcttaagccttctgcccgcggtgaactggaaattaccgatattaaccgtatctatatggaacaggggcatttatctgttgccatgatgggacgtggatatgcctggctggacacggggacacatcaaagtcttattgaagcaagcaacttcattgccaccattgaagagcgccagggcttgaaagtttcctgcccggaagaaattgcttaccgtaaagggtttattgatgctgagcaggtgaaagtattagctaaaccgctgaaaaaaaatgcttatggtcagtatctgctaaaaatgattaaaggttattaataaaatgaatgttattaaaacagaaattccagatgtactgatttttgaaccgaaagtttttggtgatgagcgtggtttctttatggaaagctttaatcagaaagttttcgaagaggctgtagggcggaaggttgaatttgttcaggataatcattctaaatcgtgtaaaggtgtacttagaggtttacactttcagcttcctccctttgagcaggcaaaattagtaaggtgtatagttggcgaggtatttgatgttgcagtagacattagacctaattctgaaacatttggttcatgggttggagtaactctttcgtcagaaaataaaaggcagctatggattccagaaggattcgcccatggttttttaactttaagtgatattgcagagtttgtttataaaactaacaactattattctttaaatcatgaaaggggagtcatttggaacgatgaggaaattaacattgcctggccctctcaatcagagaagattctgtcacagaaagatattaatttaccatcatttagatttgttcaaatgtttagcaagtagtgttatctttacactgcacatagtcatcattttttatgctttaagtaaattatattgcacatctataacacaaagcgcaataatatttcgacctgatgaaggtttgtggttatttatctttctaggcgttttttatgactaaaatagttgtggtttctacagctccaatattcccgacaaataatgggtacaaaagttctgtattaggaagaattgatgagttattaaatgaggataatgaggtcgttttgattgaaataaaccttgaaaatgttacggaaaagaaagatgaattaataccaacaagatttaataatattcaaagatatgaagtaaaaaaaatatctagatcatttattgccgagttacaaatattatttgatatcagaactcggtatgaacaattattttcttctgctgacattagagataacataaaaaagataattgatttagaaaaaccttctattattattgctgagtctatatgggcgttgcaagcattgcctattgaaattagtgcgagaatacactgtgttattcatgatgtggcaactgatttctttaaagaaatgtttgtatctcataatgaggttgtacgaaaaattttgttttttaatgattacctaaagttgaaaattactgaagaaaatattatcaaacgtttgagagttgagcaatttatctttctgacagaagaagataaatgttggtataaaacaagatacaatattgatgagggttgttgttccttagcgagcaatcatctttatgtagaaaagattaagagaactatcaatttccaaacccctttcctgcttattcccggtagcattgaattttcacaaaatttttacggcttaaattggtttataaaaaatatatatcctggattaaataggaaaataagaatagttgtaacaggaaaggcatcagataaaaaaataaagatgttaaactgtggagaggaaattacctttacgggagagcttgacttttccacatataataaacttagctcaacatgcttgtgtgttattgcaccgattacaacgggcactggaattaaaataaaaatattagaagctgtacaaaaaggtattcctgtacttacaacaaaatttgcttcaaaaggaatatgttccgatttatgtttttattgcgaggaggatactgacacaaactttgtcaatttaattaacagttttcttgaaacgacattaagagtccaagaatgaatttattgcttttttcagtccttgcgtttggtttaatattggctttggcccataataataaaagtggagatattaacgcatacttaatgttttttctcgtggtcctaatggtattaatatcagggctgcgtatgaatgatagtgattatatcgaatacaggaaaatgtataatgaagtgcctattttatgtgactttagtctcgcatctataagagatatacatggggaggtaggctatctattcttatcatcaatctttaaaactttatgcttgccatttcaattatttcttttttttattgcttttttatcactcctgcttacatatttttcattcagaaaaataagtttaataccgatactatcgttagttttttatttaagccatgcttttatagttagagatttgattcaaattagggcaggattagctgttagcatatcattatattcaataattaaatttaaaggaaataaaagtataattacaggagttttatttgcttctttgattcattctggggcgcttattattgctctttgttatccttttttcaaaaaaaaatacataacattaaaaatgatgttgtttttatttttagtgtcaattattttttcttatttgaatgggcttaatttatcgatacaactcttatctcaatatagtttgcttccaactgcaatttcgaattatgttggttgggaagaatatgattatcgggtgagtatatttactaatccggtttttattaaaggtgtttttttaattgtcttaatgcacaaatatgtactttcagatattaaaaatgagaaaattatagtgctttataacttatatgttttaggtgtattagctatggttgcattgagtgggatggctattctttcaggccgtctttcatcctttctgacactaggtgaaagcattttaattgtatatgctctgttctacaaaagaaatacacctctggcgtttctaattttttcttttttaacaattgtgcaattaggatatgatctatttatttctaatgtgcatcctgagcttactctgattatatttgggtgaatctaagtgaaaaataataaaataggcatacttatctctaaaatacaaaatcttggacctgtgaatgtagtacgaggattgataaaagaaaataaaaaatatgcttttactgttttttgtttaacaaatagcgtagataaaaatatatatgatgagttatgctgtttaggagccaaggttatattaataccagatggtacttggttcagcaaaattttatttgtgagaagttttttaaaggaacatccacataatatcttacattcacatgggatcacggccgatatgttttcttactttctgaatggcgtgaaaatatctactattcacaatagactagatgaggattatatcccattatttggcgcggttaaagggaatgctatatattatcttcatcgttttatattacgaagatttaatcatatcgttgcttgctcagcagcggtccaatcaaaactgaaacaatcgaaagtaaaaactaaaataaccaccatccagaatgggattgatataactaggtttaagacacttgagtctgataaaaaaaaattattgagggaaaaacacggatttgatagtgaaaaaagaatatttatatattgtggctcgttatcattaaggaaaaatattgcttacctcttggaacacttagccatcgaagaaaatgatatatttttaattctaggtgatggtgaactttttagatattgtaaggataaatattctaaagatttacggtatatatttatggggaaagttgaatgccctcttgaatattatcaattatcagatatttttgtttccgcttctttatcggaagggctccccttggcactattagaagctgcctctactgggtgctatttatatgttagcgatatagagccccatagagaaattgcatctctattaggagaggaaaatatttctatgtttaaaattaaggatggatcatataattatttgcaacctaaaataaaaaaagctgactataacgctctttctgacgataaactttacaatatatccgataaaaaaatgtcaaatctttatgacaaactttttgtttctttattagagcagaggcactaatataatgatttatgtttcggtaatttctcatggtcatttcaaaactcttaaggaattaggagcagtatcaaaattaaataatcacagcagaattaaagttatcatcaaagataatttaggagagagcgagcttttggatttttgtcaggaaaacaaaataacttatttaaggtctaaagagaaaaaaggatttggagagaataataatgaagttttttcctctatatcctccttaattactaaggaagatttttttgtggttatgaatcctgatatatatattgagtgctctgatctattagatgtcgtagatgagtgtggttcagcgaatgttaatctagcaacgataaatttatacagggattttgataaaaaaacatatgataactcagtaaggaaatttccctcggcaattgatttttttatgtcatttttatttaagaaaaatgactgtgtagtaaataagaacaaaataacgaaaccaacatatgttgattgggctgcaggttcttttctaatatttaatgccttcttttattcaaaactcaacggattcaacgaaaagtattttatgtattgcgaagatattgatatatgttggcgagctaaaaaacacttcaatacttcagttttatactatccatgctatgcagcaattcatttggcacaatttaacaatcgtaggatttttagtagacatttcatttggcatataaaaagtattatcctttttttattatataaaaatggtatgctgcgttctagtaagttgctttaatgctaatattcttttaagaggtgagaatgatacctgttattttggctggtggttcgggaagtcgcttgtggccactttcacgagaaaagttccccaagcagtttttaaagttgactggcagtttgacaatgttgcagtcaacattgtcacgtcttaataatttaaatgctgatgattcaatagttatatgcaacgaagagcatagatttattgttgcagaacaattaagagagttaggcaaactttcaaataacattattcttgaacccaaaggtcgtaatacagcccctgctataacactcgcagcattagcagcaaaaagaaaattcgctgatgaagatccattgattcttattttagctgcagatcacaacatccaagacgaacatgttttctgtgaggcaattaataaggcgtcatctttagctagttatggaaaactagtgacttttggtatcgttccattcaaacctgaaactgggtatggctatattcgtcgcggtgatgaagtgcctgtagatgagcagcatgcggtggcctttgaagtggcgcagtttgtcgaaaaaccgaatctggaaaccgcgcaggcctatgtggcaagcggcgaatattactggaacagcggtatgttcctgttccgtgccggacgctatctcgaagaactgaaaaagtatcgtccggatattctcgatgcctgtgaaaaagcgatgagcgccgtcgatccggatctcgattttattcgtgtggatgaagaggcgtttctcgcttgtccggaagagtcggtggattacgcggtcatggaatgcacggcagatgccgttgtggtgccgatggatgcgggctggagcgatgtcggttcctggtcttcattatgggagatcagcgcccacaccgccgagggcaacgtttgccacggcgatgtgattaatcacaaaactgaaaacagctatgtgtacgccgaatctggcctggtcaccaccgtcggggtgaaagatttggtggtagtgcagaccaaagatgcagtgctgattgccgaccgtaatgcggtgcaggatgtgaagaaagtggtcgagcagatcaaagctgatggtcgccatgagcatcgggtgcatcgcgaagtgtatcgtccgtggggcaaatatgactctatcgacgcgggcgaccgctaccaggtgaaacgcatcaccgtgaaaccgggcgaaggtttgtcggtacagatgcattatcatcgcgcggaacactgggtggttgtcgcgggaacggcaaaagtcactatcaacggtgatatcaaactgcttggtgaaaacgagtccatttatattccgctgggggcgatgcactgcctggaaaacccggggaaaatagatttagaattaattgaagttcgctctggtgcatatcttgaagaagatgatgttattagatgttatgatcgctatggacgaaagtaatatataataattatttcagaattagaaatgataattataagttttcgtctggataaacaatagatagtatgggttggaaaatatgagttctttaacttgttttaaagcttacgacattcgcgggaaattaggtgaagaactgaatgaagatatcgcctggcgcattggtcgcgcctatggcgaatttctcaaaccgaaaaccattgtgttaggcggtgatgtccgtctcaccagcgaaaccttaaaactggcgctggcaaaaggtttacaggatgcgggcgtcgatgtgctggatattggcatgtccggcaccgaagagatttatttcgccacgttccatctcggcgtggatggcggcattgaagttaccgccagccataatccgatggattacaacggcatgaagctggtgcgcgaaggggctcgcccgatcagcggtgataccggactgcgcgacgtccagcgtctggcagaagctaacgactttcctcccgtcgatgaaaccaaacgcggtcgctatcagcaaatcaatctgcgtgacgcttacgttgatcacctgttcggttatatcaatgtcaaaaaccttacgccgctcaagctggtgatcaactccgggaatggcgcagcgggtccggtggtggacgctatcgaagcccgctttaaagccctcggcgcaccggtggagttaatcaaagtgcataacacgccggacggcaatttccccaacggtattcctaacccgttgctgccggaatgtcgcgacgacacccgcaatgcggtcatcaaacacggcgcggatatgggcattgcctttgatggcgattttgaccgctgtttcctgtttgacgaaaaagggcagtttattgagggctactacattgtcggcctgctggcagaagcgttcctcgaaaaaaatcccggcgcgaagatcatccacgatccacgtctctcctggaacaccattgatgtggtgacggccgcgggcggcacgccggtgatgtcgaaaacaggacacgcctttattaaagaacgtatgcgcaaggaagacgccatctacggtggcgaaatgagcgctcaccattacttccgcgatttcgcttactgtgacagcggcatgatcccgtggctgctggtcgccgaactggtgtgcctgaaaggaaaaacgctgggcgaactggtgcgcgaccggatggcggcgtttccggcaagcggtgagatcaacagaaaactggcgcaccctgttgaggcgattaaccgcgtggaacagcattttagccgtgaggtgctggcggtggatcgcaccgatggcatcagcatgacctttgccgactggcgctttaacctgcgctcttccaacaccgaaccggtggtgcgcctgaatgtggaatctcgcggtgatgttcaggttatggtaatccatactcaagaaatattatcaattttgacgtcataaagaataagccctgacaagttagggcttaattaatatatattttttttgaattggggatttgtggtaagatttttaatatgttatttaatgtggttgaattaatgttgactggaaaataataatgagaacgaaaaaagcattacacaactttaaagttgatttattaattacttttttattggttttgctagggttttatattcgaactgtttttgtttcaaaaatgggaagtgatattactggagtgatgttactattcacacagttgacagcatatctcaatttggcagaattaggtattggaattgcagctgccagcgtattatataaaccgctcagcgagaatgaatacaataaaataacttacataatatctttgctctcagtcatatacaaatatatatttgtgtttgttttgattcttggcgttgttataggtatctgtatttattactttattgattctgtaaaggttgtaaatggcgtttttttatattgggctttgttcgtttttaatacatcgttgacatatagttatgctaaatactccacattattaactgctaatcagcggtactcagcagtaagaaaaattcaaggtggcggaaaagttataataattgtatttcagatattaattttgtgctttacgcaaagtttcatactttatttgttagttgagactttaggtattttttctcaatatttgatttttaaaaaaataattgggaacggaaatcaatatctcagtaatgaggttttacttattgaaagcgataaacttttgataaaaaaagaattaaaaataagaataaaaaatatgttcttccataaaataggtgctgtgcttgtccttaatacagactacctgcttgtatcaaagtttctgacattaagttatgtgacaatttttggcagctatatgatggtatttcagatagtaactgttttgatgtcaagttttgttaatgctattactgcaggaatgggtaattacttaattaataaaagtaatttagaaattaaggaaattacacgtcaattttatgtgatatttatcgcctttgcaacattcatatcactaaatatgttttttcttgttaatgattttatcgcaaaatggataggtgttaattatacattaagtaacaccctagttgcattaatgattgttaacgtattcattagtgttgtcagggtaccttctgatatattaaaaaacgcaagtggacattttggtgatatttattatccattattagaaggtgtgctgaatattacgatatccatcattttggctatcattattggattacctggcattattatagggacaatagtatctaacttaatagtaataatgcttgcgaaaccattatatctttactctaagttatttaatcttagaaatccgacgagggtttattttgaatttatttctcggcctatgttatattcattatgtgtgattggggtgagctatttattgcgcgatgaaatatattcatttaaagtaagtacatggttggattttattaacaagctactcttagtctctactcctagcatattggtaatatgtgctattttctctacggatagtgactttagattatttttcagaaaaattatatatgtgattatgaagaaataaaaatttcgaaaatgtattaatcgaaattatgcaacgagctttatttttataaatgatatgtgatcttttcgcgaataggagtaaggatccgtgtaggctggagctgcttcgaagttcctatactttctagagaataggaacttcggaataggaactaaggaggatattcatatggataaagccgtaagcatataagcatggataagctatttatactttaataagtactttgtatacttatttgcgaacattccaggccgcgagcattcagcgcggtgatcacacctgacaggagtatgtaatgtccaagcaacagatcggcgtagtcggtatggcagtgatgggacgcaaccttgcgctcaacatcgaaagccgtggttataccgtctctattttcaaccgttcccgtgagaagacggaagaagtgattgccgaaaatccaggcaagaaactggttccttactatacggtgaaagagtttgtcgaatctctggaaacgcctcgtcgcatcctgttaatggtgaaagcaggtgcaggcacggatgctgctattgattccctcaaaccatatctcgataaaggagacatcatcattgatggtggtaacaccttcttccaggacactattcgtcgtaatcgtgagctttcagcagagggctttaacttcatcggtaccggtgtttctggcggtgaagagggggcgctgaaaggtccttctattatgcctggtggccagaaagaagcctatgaattggtagcaccgatcctgaccaaaatcgccgccgtagctgaagacggtgaaccatgcgttacctatattggtgccgatggcgcaggtcactatgtgaagatggttcacaacggtattgaatacggcgatatgcagctgattgctgaagcctattctctgcttaaaggtggcctgaacctcaccaacgaagaactggcgcagacctttaccgagtggaataacggtgaactgagcagttacctgatcgacatcaccaaagatatcttcaccaaaaaagatgaagacggtaactacctggttgatgtgatcctggatgaagcggctaacaaaggtaccggtaaatggaccagccagagcgcgctggatctcggcgaaccgctgtcgctgattaccgagtctgtgtttgcacgttatatctcttctctgaaagatcagcgtgttgccgcatctaaagttctctctggtccgcaagcacagccagcaggcgacaaggctgagttcatcgaaaaagttcgtcgtgcgctgtatctgggcaaaatcgtttcttacgcccagggcttctctcagctgcgtgctgcgtctgaagagtacaactgggatctgaactacggcgaaatcgcgaagattttccgtgctggctgcatcatccgtgcgcagttcctgcagaaaatcaccgatgcttatgccgaaaatccacagatcgctaacctgttgctggctccgtacttcaagcaaattgccgatgactaccagcaggcgctgcgtgatgtcgttgcttatgcagtacagaacggtattccggttccgaccttctccgcagcggttgcctattacgacagctaccgtgctgctgttctgcctgcgaacctgatccaggcacagcgtgactattttggtgcgcatacttataagcgtattgataaagaaggtgtgttccataccgaatggctggattaa